European Patent Application EP 4 606 897 A1, published August 27, 2025. Title: Nucelic acid molecule coding CAR, CAR, immunocyte comprising CAR, pharmaceutical composition comrising immunocyte and method for producing imunnocyte comprising CAR. Applicant: MIE UNIVERSITY. Application WO. The sequence listing filed with the application follows.

SEQUENCE LISTING (271 sequences)

SEQ ID NO: 1 - protein, 10 aa, Homo sapiens
GVYDGREHTV

SEQ ID NO: 2 - protein, 9 aa, Homo sapiens
LYVDSLFFL

SEQ ID NO: 3 - DNA, 1707 bp, synthetic construct
  source 1..1707: mol_type = other DNA
atgaaacacctgtggttcttcctcctgctggtggcagctcccagatgggtcctgtcccaggtgcagctgcaggtccagctggtacagtctggggctgaggtgaagaagcctgggtcctcggtgaaggtctcctgcaaggcttctggaggcaccttcagcagctatgctatcagctgggtgcgacaggcccctggacaagggcttgagtggatgggagggatcatccctatctttggtacagcaaactacgcacagaagttccagggcagagtcacgattaccgcggacaaatccacgagcacagcctacatggagctgagcagcctgagatctgaggacacggccgtgtattactgtgcgagatccccccggcgggcatatcatgatgcttttgatatctggggccaagggacaatggtcaccgtctcttcaggtggaggcggttcaggcggaggtggcagcggcggtggcgggagttcctatgagctgactcagccaccctcgatgtcagtggccccaggaaagacggccagcattacctgtggcggagaccatattggaagtaaaagtgttcactggtaccagcagaagccaggccaggcccctgtactggtcgtctatgatgatagcgaccggccctcagggatccctgagcgattctctggctccaactctgggaacacagccactctgaccatcagcgggacccaggctatggatgaggctgactattactgtctggcgtgggacagcagcactgcgatcttcggcggaggcacccagctgaccgtcctcgtgggtcagcccaaggccaaccccactgtcactctgtttccgccctcctctgaggagctccaagccaacaaggccacactagtgtgtctgatcagtgacttctacccgggagctgtgacagtggcctggaaggcagatggcagccccgtcaaggcgggagtggagaccaccaaaccctccaaacagagcaacaacaagtacgcggccagcagctacctgagcctgacgcccgagcagtggaagtcccacagaagctacagctgccaggtcacgcatgaagggagcaccgtggagaagactgtggcccctacagaatgttcggcgcgccagactagattttgggtgctggtggtggttggtggagtcctggcttgctatagcttgctagtaacagtggcctttattattttctgggtgaggctgagagtgaagttcagcaggagcgcagacgcccccgcgtaccagcagggccagaaccagctctataacgagctcaatctaggacgaagagaggagtacgatgttttggacaagagacgtggccgggaccctgagatggggggaaagccgcagagaaggaagaaccctcaggaaggcctgtacaatgaactgcagaaagataagatggcggaggcctacagtgagattgggatgaaaggcgagcgccggaggggcaaggggcacgatggcctttaccagggtctcagtacagccaccaaggacacctacgacgcccttcacatgcaggccctgccccctcgcaggagtcagtgcatgtggccccgagagacccagctgctgctggaggtgccgccgtcgaccgaagacgccagaagctgccagttccccgaggaagagcggggcgagcgatcggcagaggagaaggggcggctgggagacctgtgggtgtaa

SEQ ID NO: 4 - protein, 568 aa, synthetic construct
MKHLWFFLLLVAAPRWVLSQVQLQVQLVQSGAEVKKPGSSVKVSCKASGGTFSSYAISWVRQAPGQGLEWMGGIIPIFGTANYAQKFQGRVTITADKSTSTAYMELSSLRSEDTAVYYCARSPRRAYHDAFDIWGQGTMVTVSSGGGGSGGGGSGGGGSSYELTQPPSMSVAPGKTASITCGGDHIGSKSVHWYQQKPGQAPVLVVYDDSDRPSGIPERFSGSNSGNTATLTISGTQAMDEADYYCLAWDSSTAIFGGGTQLTVLVGQPKANPTVTLFPPSSEELQANKATLVCLISDFYPGAVTVAWKADGSPVKAGVETTKPSKQSNNKYAASSYLSLTPEQWKSHRSYSCQVTHEGSTVEKTVAPTECSARQTRFWVLVVVGGVLACYSLLVTVAFIIFWVRLRVKFSRSADAPAYQQGQNQLYNELNLGRREEYDVLDKRRGRDPEMGGKPQRRKNPQEGLYNELQKDKMAEAYSEIGMKGERRRGKGHDGLYQGLSTATKDTYDALHMQALPPRRSQCMWPRETQLLLEVPPSTEDARSCQFPEEERGERSAEEKGRLGDLWV

SEQ ID NO: 5 - DNA, 1707 bp, synthetic construct
  source 1..1707: mol_type = other DNA
atgaaacacctgtggttcttcctcctgctggtggcagctcccagatgggtcctgtcccaggtgcagctgcaggtccagctggtacagtctggggctgaggtgaagaagcctgggtcctcggtgaaggtctcctgcaaggcttctggaggcaccttcagcagctatgctatcagctgggtgcgacaggcccctggacaagggcttgagtggatgggagggatcatccctatctttggtacagcaaactacgcacagaagttccagggcagagtcacgattaccgcggacaaatccacgagcacagcctacatggagctgagcagcctgagatctgaggacacggccgtgtattactgtgcgagatccccccggcgggcatatcatgatgcttttgatatctggggccaagggacaatggtcaccgtctcttcaggtggaggcggttcaggcggaggtggcagcggcggtggcgggagttcctatgagctgactcagccaccctcgatgtcagtggccccaggaaagacggccagcattacctgtggcggagaccatattggaagtaaaagtgttcactggtaccagcagaagccaggccaggcccctgtactggtcgtctatgatgatagcgaccggccctcagggatccctgagcgattccgaggccgaaaccgagggaaccgagccactctgaccatcagcgggacccaggctatggatgaggctgactattactgtctggcgtgggacagcagcactgcgatcttcggcggaggcacccagctgaccgtcctcgtgggtcagcccaaggccaaccccactgtcactctgtttccgccctcctctgaggagctccaagccaacaaggccacactagtgtgtctgatcagtgacttctacccgggagctgtgacagtggcctggaaggcagatggcagccccgtcaaggcgggagtggagaccaccaaaccctccaaacagagcaacaacaagtacgcggccagcagctacctgagcctgacgcccgagcagtggaagtcccacagaagctacagctgccaggtcacgcatgaagggagcaccgtggagaagactgtggcccctacagaatgttcggcgcgccagactagattttgggtgctggtggtggttggtggagtcctggcttgctatagcttgctagtaacagtggcctttattattttctgggtgaggctgagagtgaagttcagcaggagcgcagacgcccccgcgtaccagcagggccagaaccagctctataacgagctcaatctaggacgaagagaggagtacgatgttttggacaagagacgtggccgggaccctgagatggggggaaagccgcagagaaggaagaaccctcaggaaggcctgtacaatgaactgcagaaagataagatggcggaggcctacagtgagattgggatgaaaggcgagcgccggaggggcaaggggcacgatggcctttaccagggtctcagtacagccaccaaggacacctacgacgcccttcacatgcaggccctgccccctcgcaggagtcagtgcatgtggccccgagagacccagctgctgctggaggtgccgccgtcgaccgaagacgccagaagctgccagttccccgaggaagagcggggcgagcgatcggcagaggagaaggggcggctgggagacctgtgggtgtaa

SEQ ID NO: 6 - protein, 568 aa, synthetic construct
MKHLWFFLLLVAAPRWVLSQVQLQVQLVQSGAEVKKPGSSVKVSCKASGGTFSSYAISWVRQAPGQGLEWMGGIIPIFGTANYAQKFQGRVTITADKSTSTAYMELSSLRSEDTAVYYCARSPRRAYHDAFDIWGQGTMVTVSSGGGGSGGGGSGGGGSSYELTQPPSMSVAPGKTASITCGGDHIGSKSVHWYQQKPGQAPVLVVYDDSDRPSGIPERFRGRNRGNRATLTISGTQAMDEADYYCLAWDSSTAIFGGGTQLTVLVGQPKANPTVTLFPPSSEELQANKATLVCLISDFYPGAVTVAWKADGSPVKAGVETTKPSKQSNNKYAASSYLSLTPEQWKSHRSYSCQVTHEGSTVEKTVAPTECSARQTRFWVLVVVGGVLACYSLLVTVAFIIFWVRLRVKFSRSADAPAYQQGQNQLYNELNLGRREEYDVLDKRRGRDPEMGGKPQRRKNPQEGLYNELQKDKMAEAYSEIGMKGERRRGKGHDGLYQGLSTATKDTYDALHMQALPPRRSQCMWPRETQLLLEVPPSTEDARSCQFPEEERGERSAEEKGRLGDLWV

SEQ ID NO: 7 - DNA, 1707 bp, synthetic construct
  source 1..1707: mol_type = other DNA
atgaaacacctgtggttcttcctcctgctggtggcagctcccagatgggtcctgtcccaggtgcagctgcaggtccagctggtacagtctggggctgaggtgaagaagcctgggtcctcggtgaaggtctcctgcaaggcttctggaggcaccttcagcagctatgctatcagctgggtgcgacaggcccctggacaagggcttgagtggatgggagggatcatccctatctttggtacagcaaactacgcacagaagttccagggcagagtcacgattaccgcggacaaatccacgagcacagcctacatggagctgagcagcctgagatctgaggacacggccgtgtattactgtgcgagatccccccggcgggcatatcatgatgcttttgatatctggggccaagggacaatggtcaccgtctcttcaggtggaggcggttcaggcggaggtggcagcggcggtggcgggagttcctatgagctgactcagccaccctcgatgtcagtggccccaggaaagacggccagcattacctgtggcggagaccatattggaagtaaaagtgttcactggtaccagcagaagccaggccaggcccctgtactggtcgtctatgatgatagcgaccggccctcagggatccctgagcgattccgaggccgaaaccgagggaacacagcccgactgaccatcagcgggacccaggctatggatgaggctgactattactgtctggcgtgggacagcagcactgcgatcttcggcggaggcacccagctgaccgtcctcgtgggtcagcccaaggccaaccccactgtcactctgtttccgccctcctctgaggagctccaagccaacaaggccacactagtgtgtctgatcagtgacttctacccgggagctgtgacagtggcctggaaggcagatggcagccccgtcaaggcgggagtggagaccaccaaaccctccaaacagagcaacaacaagtacgcggccagcagctacctgagcctgacgcccgagcagtggaagtcccacagaagctacagctgccaggtcacgcatgaagggagcaccgtggagaagactgtggcccctacagaatgttcggcgcgccagactagattttgggtgctggtggtggttggtggagtcctggcttgctatagcttgctagtaacagtggcctttattattttctgggtgaggctgagagtgaagttcagcaggagcgcagacgcccccgcgtaccagcagggccagaaccagctctataacgagctcaatctaggacgaagagaggagtacgatgttttggacaagagacgtggccgggaccctgagatggggggaaagccgcagagaaggaagaaccctcaggaaggcctgtacaatgaactgcagaaagataagatggcggaggcctacagtgagattgggatgaaaggcgagcgccggaggggcaaggggcacgatggcctttaccagggtctcagtacagccaccaaggacacctacgacgcccttcacatgcaggccctgccccctcgcaggagtcagtgcatgtggccccgagagacccagctgctgctggaggtgccgccgtcgaccgaagacgccagaagctgccagttccccgaggaagagcggggcgagcgatcggcagaggagaaggggcggctgggagacctgtgggtgtaa

SEQ ID NO: 8 - protein, 568 aa, synthetic construct
MKHLWFFLLLVAAPRWVLSQVQLQVQLVQSGAEVKKPGSSVKVSCKASGGTFSSYAISWVRQAPGQGLEWMGGIIPIFGTANYAQKFQGRVTITADKSTSTAYMELSSLRSEDTAVYYCARSPRRAYHDAFDIWGQGTMVTVSSGGGGSGGGGSGGGGSSYELTQPPSMSVAPGKTASITCGGDHIGSKSVHWYQQKPGQAPVLVVYDDSDRPSGIPERFRGRNRGNTARLTISGTQAMDEADYYCLAWDSSTAIFGGGTQLTVLVGQPKANPTVTLFPPSSEELQANKATLVCLISDFYPGAVTVAWKADGSPVKAGVETTKPSKQSNNKYAASSYLSLTPEQWKSHRSYSCQVTHEGSTVEKTVAPTECSARQTRFWVLVVVGGVLACYSLLVTVAFIIFWVRLRVKFSRSADAPAYQQGQNQLYNELNLGRREEYDVLDKRRGRDPEMGGKPQRRKNPQEGLYNELQKDKMAEAYSEIGMKGERRRGKGHDGLYQGLSTATKDTYDALHMQALPPRRSQCMWPRETQLLLEVPPSTEDARSCQFPEEERGERSAEEKGRLGDLWV

SEQ ID NO: 9 - DNA, 1800 bp, synthetic construct
  source 1..1800: mol_type = other DNA
atgaaacacctgtggttcttcctcctgctggtggcagctcccagatgggtcctgtcccaggtgcagctgcaggtccagctggtacagtctggggctgaggtgaagaagcctgggtcctcggtgaaggtctcctgcaaggcttctggaggcaccttcagcagctatgctatcagctgggtgcgacaggcccctggacaagggcttgagtggatgggagggatcatccctatctttggtacagcaaactacgcacagaagttccagggcagagtcacgattaccgcggacaaatccacgagcacagcctacatggagctgagcagcctgagatctgaggacacggccgtgtattactgtgcgagatccccccggcgggcatatcatgatgcttttgatatctggggccaagggacaatggtcaccgtctcttcaggtggaggcggttcaggcggaggtggcagcggcggtggcgggagttcctatgagctgactcagccaccctcgatgtcagtggccccaggaaagacggccagcattacctgtggcggagaccatattggaagtaaaagtgttcactggtaccagcagaagccaggccaggcccctgtactggtcgtctatgatgatagcgaccggccctcagggatccctgagcgattctctggctccaactctgggaacacagccactctgaccatcagcgggacccaggctatggatgaggctgactattactgtctggcgtgggacagcagcactgcgatcttcggcggaggcacccagctgaccgtcctcgtgggtcagcccaaggccaaccccactgtcactctgtttccgccctcctctgaggagctccaagccaacaaggccacactagtgtgtctgatcagtgacttctacccgggagctgtgacagtggcctggaaggcagatggcagccccgtcaaggcgggagtggagaccaccaaaccctccaaacagagcaacaacaagtacgcggccagcagctacctgagcctgacgcccgagcagtggaagtcccacagaagctacagctgccaggtcacgcatgaagggagcaccgtggagaagactgtggcccctacagaatgttcggcgcgccagactagattttgggtgctggtggtggttggtggagtcctggcttgctatagcttgctagtaacagtggcctttattattttctgggtgaggctgagagtgaagttcagcaggagcgcagacgcccccgcgtaccagcagggccagaaccagctctataacgagctcaatctaggacgaagagaggagtacgatgttttggacaagagacgtggccgggaccctgagatggggggaaagccgcagagaaggaagaaccctcaggaaggcctgtacaatgaactgcagaaagataagatggcggaggcctacagtgagattgggatgaaaggcgagcgccggaggggcaaggggcacgatggcctttaccagggtctcagtacagccaccaaggacacctacgacgcccttcacatgcaggccctgccccctcgcaggagtcagtgcatgtggccccgagagacccagctgctgctggaggtgccgccgtcgaccgaagacgccagaagctgccagttccccgaggaagagcggggcgagcgatcggcagaggagaaggggcggctgggagaccttgggtgtaatcgattctcgagcgataaaataaaagatttatttagtctccagaaaaaggggggaatgaaagaccccaccccacctgtaggtttggcaagctag

SEQ ID NO: 10 - protein, 599 aa, synthetic construct
MKHLWFFLLLVAAPRWVLSQVQLQVQLVQSGAEVKKPGSSVKVSCKASGGTFSSYAISWVRQAPGQGLEWMGGIIPIFGTANYAQKFQGRVTITADKSTSTAYMELSSLRSEDTAVYYCARSPRRAYHDAFDIWGQGTMVTVSSGGGGSGGGGSGGGGSSYELTQPPSMSVAPGKTASITCGGDHIGSKSVHWYQQKPGQAPVLVVYDDSDRPSGIPERFSGSNSGNTATLTISGTQAMDEADYYCLAWDSSTAIFGGGTQLTVLVGQPKANPTVTLFPPSSEELQANKATLVCLISDFYPGAVTVAWKADGSPVKAGVETTKPSKQSNNKYAASSYLSLTPEQWKSHRSYSCQVTHEGSTVEKTVAPTECSARQTRFWVLVVVGGVLACYSLLVTVAFIIFWVRLRVKFSRSADAPAYQQGQNQLYNELNLGRREEYDVLDKRRGRDPEMGGKPQRRKNPQEGLYNELQKDKMAEAYSEIGMKGERRRGKGHDGLYQGLSTATKDTYDALHMQALPPRRSQCMWPRETQLLLEVPPSTEDARSCQFPEEERGERSAEEKGRLGDLGCNRFSSDKIKDLFSLQKKGGMKDPTPPVGLAS

SEQ ID NO: 11 - DNA, 1800 bp, synthetic construct
  source 1..1800: mol_type = other DNA
atgaaacacctgtggttcttcctcctgctggtggcagctcccagatgggtcctgtcccaggtgcagctgcaggtccagctggtacagtctggggctgaggtgaagaagcctgggtcctcggtgaaggtctcctgcaaggcttctggaggcaccttcagcagctatgctatcagctgggtgcgacaggcccctggacaagggcttgagtggatgggagggatcatccctatctttggtacagcaaactacgcacagaagttccagggcagagtcacgattaccgcggacaaatccacgagcacagcctacatggagctgagcagcctgagatctgaggacacggccgtgtattactgtgcgagatccccccggcgggcatatcatgatgcttttgatatctggggccaagggacaatggtcaccgtctcttcaggtggaggcggttcaggcggaggtggcagcggcggtggcgggagttcctatgagctgactcagccaccctcgatgtcagtggccccaggaaagacggccagcattacctgtggcggagaccatattggaagtaaaagtgttcactggtaccagcagaagccaggccaggcccctgtactggtcgtctatgatgatagcgaccggccctcagggatccctgagcgattccgaggccgaaaccgagggaaccgagccactctgaccatcagcgggacccaggctatggatgaggctgactattactgtctggcgtgggacagcagcactgcgatcttcggcggaggcacccagctgaccgtcctcgtgggtcagcccaaggccaaccccactgtcactctgtttccgccctcctctgaggagctccaagccaacaaggccacactagtgtgtctgatcagtgacttctacccgggagctgtgacagtggcctggaaggcagatggcagccccgtcaaggcgggagtggagaccaccaaaccctccaaacagagcaacaacaagtacgcggccagcagctacctgagcctgacgcccgagcagtggaagtcccacagaagctacagctgccaggtcacgcatgaagggagcaccgtggagaagactgtggcccctacagaatgttcggcgcgccagactagattttgggtgctggtggtggttggtggagtcctggcttgctatagcttgctagtaacagtggcctttattattttctgggtgaggctgagagtgaagttcagcaggagcgcagacgcccccgcgtaccagcagggccagaaccagctctataacgagctcaatctaggacgaagagaggagtacgatgttttggacaagagacgtggccgggaccctgagatggggggaaagccgcagagaaggaagaaccctcaggaaggcctgtacaatgaactgcagaaagataagatggcggaggcctacagtgagattgggatgaaaggcgagcgccggaggggcaaggggcacgatggcctttaccagggtctcagtacagccaccaaggacacctacgacgcccttcacatgcaggccctgccccctcgcaggagtcagtgcatgtggccccgagagacccagctgctgctggaggtgccgccgtcgaccgaagacgccagaagctgccagttccccgaggaagagcggggcgagcgatcggcagaggagaaggggcggctgggagaccttgggtgtaatcgattctcgagcgataaaataaaagatttatttagtctccagaaaaaggggggaatgaaagaccccaccccacctgtaggtttggcaagctag

SEQ ID NO: 12 - protein, 599 aa, synthetic construct
MKHLWFFLLLVAAPRWVLSQVQLQVQLVQSGAEVKKPGSSVKVSCKASGGTFSSYAISWVRQAPGQGLEWMGGIIPIFGTANYAQKFQGRVTITADKSTSTAYMELSSLRSEDTAVYYCARSPRRAYHDAFDIWGQGTMVTVSSGGGGSGGGGSGGGGSSYELTQPPSMSVAPGKTASITCGGDHIGSKSVHWYQQKPGQAPVLVVYDDSDRPSGIPERFRGRNRGNRATLTISGTQAMDEADYYCLAWDSSTAIFGGGTQLTVLVGQPKANPTVTLFPPSSEELQANKATLVCLISDFYPGAVTVAWKADGSPVKAGVETTKPSKQSNNKYAASSYLSLTPEQWKSHRSYSCQVTHEGSTVEKTVAPTECSARQTRFWVLVVVGGVLACYSLLVTVAFIIFWVRLRVKFSRSADAPAYQQGQNQLYNELNLGRREEYDVLDKRRGRDPEMGGKPQRRKNPQEGLYNELQKDKMAEAYSEIGMKGERRRGKGHDGLYQGLSTATKDTYDALHMQALPPRRSQCMWPRETQLLLEVPPSTEDARSCQFPEEERGERSAEEKGRLGDLGCNRFSSDKIKDLFSLQKKGGMKDPTPPVGLAS

SEQ ID NO: 13 - DNA, 1707 bp, synthetic construct
  source 1..1707: mol_type = other DNA
atgaaacacctgtggttcttcctcctgctggtggcagctcccagatgggtcctgtcccaggtgcagctgcaggtccagctggtacagtctggggctgaggtgaagaagcctgggtcctcggtgaaggtctcctgcaaggcttctggaggcaccttcagcagctatgctatcagctgggtgcgacaggcccctggacaagggcttgagtggatgggagggatcatccctatctttggtacagcaaactacgcacagaagttccagggcagagtcacgattaccgcggacaaatccacgagcacagcctacatggagctgagcagcctgagatctgaggacacggccgtgtattactgtgcgagatccccccggcgggcatatcatgatgcttttgatatctggggccaagggacaatggtcaccgtctcttcaggtggaggcggttcaggcggaggtggcagcggcggtggcgggagttcctatgagctgactcagccaccctcgatgtcagtggccccaggaaagacggccagcattacctgtggcggagaccatattggaagtaaaagtgttcactggtaccagcagaagccaggccaggcccctgtactggtcgtctatgatgatagcgaccggccctcagggatccctgagcgattcagaggcaggaactctgggaacacagccaggctgaccatcagcgggacccaggctatggatgaggctgactattactgtctggcgtgggacagcagcactgcgatcttcggcggaggcacccagctgaccgtcctcgtgggtcagcccaaggccaaccccactgtcactctgtttccgccctcctctgaggagctccaagccaacaaggccacactagtgtgtctgatcagtgacttctacccgggagctgtgacagtggcctggaaggcagatggcagccccgtcaaggcgggagtggagaccaccaaaccctccaaacagagcaacaacaagtacgcggccagcagctacctgagcctgacgcccgagcagtggaagtcccacagaagctacagctgccaggtcacgcatgaagggagcaccgtggagaagactgtggcccctacagaatgttcggcgcgccagactagattttgggtgctggtggtggttggtggagtcctggcttgctatagcttgctagtaacagtggcctttattattttctgggtgaggctgagagtgaagttcagcaggagcgcagacgcccccgcgtaccagcagggccagaaccagctctataacgagctcaatctaggacgaagagaggagtacgatgttttggacaagagacgtggccgggaccctgagatggggggaaagccgcagagaaggaagaaccctcaggaaggcctgtacaatgaactgcagaaagataagatggcggaggcctacagtgagattgggatgaaaggcgagcgccggaggggcaaggggcacgatggcctttaccagggtctcagtacagccaccaaggacacctacgacgcccttcacatgcaggccctgccccctcgcaggagtcagtgcatgtggccccgagagacccagctgctgctggaggtgccgccgtcgaccgaagacgccagaagctgccagttccccgaggaagagcggggcgagcgatcggcagaggagaaggggcggctgggagacctgtgggtgtaa

SEQ ID NO: 14 - protein, 568 aa, synthetic construct
MKHLWFFLLLVAAPRWVLSQVQLQVQLVQSGAEVKKPGSSVKVSCKASGGTFSSYAISWVRQAPGQGLEWMGGIIPIFGTANYAQKFQGRVTITADKSTSTAYMELSSLRSEDTAVYYCARSPRRAYHDAFDIWGQGTMVTVSSGGGGSGGGGSGGGGSSYELTQPPSMSVAPGKTASITCGGDHIGSKSVHWYQQKPGQAPVLVVYDDSDRPSGIPERFRGRNSGNTARLTISGTQAMDEADYYCLAWDSSTAIFGGGTQLTVLVGQPKANPTVTLFPPSSEELQANKATLVCLISDFYPGAVTVAWKADGSPVKAGVETTKPSKQSNNKYAASSYLSLTPEQWKSHRSYSCQVTHEGSTVEKTVAPTECSARQTRFWVLVVVGGVLACYSLLVTVAFIIFWVRLRVKFSRSADAPAYQQGQNQLYNELNLGRREEYDVLDKRRGRDPEMGGKPQRRKNPQEGLYNELQKDKMAEAYSEIGMKGERRRGKGHDGLYQGLSTATKDTYDALHMQALPPRRSQCMWPRETQLLLEVPPSTEDARSCQFPEEERGERSAEEKGRLGDLWV

SEQ ID NO: 15 - DNA, 1707 bp, synthetic construct
  source 1..1707: mol_type = other DNA
atgaaacacctgtggttcttcctcctgctggtggcagctcccagatgggtcctgtcccaggtgcagctgcaggtccagctggtacagtctggggctgaggtgaagaagcctgggtcctcggtgaaggtctcctgcaaggcttctggaggcaccttcagcagctatgctatcagctgggtgcgacaggcccctggacaagggcttgagtggatgggagggatcatccctatctttggtacagcaaactacgcacagaagttccagggcagagtcacgattaccgcggacaaatccacgagcacagcctacatggagctgagcagcctgagatctgaggacacggccgtgtattactgtgcgagatccccccggcgggcatatcatgatgcttttgatatctggggccaagggacaatggtcaccgtctcttcaggtggaggcggttcaggcggaggtggcagcggcggtggcgggagttcctatgagctgactcagccaccctcgatgtcagtggccccaggaaagacggccagcattacctgtggcggagaccatattggaagtaaaagtgttcactggtaccagcagaagccaggccaggcccctgtactggtcgtctatgatgatagcgaccggccctcagggatccctgagcgattcaagggctccaacaaggggaacaaagccactctgaccatcagcgggacccaggctatggatgaggctgactattactgtctggcgtgggacagcagcactgcgatcttcggcggaggcacccagctgaccgtcctcgtgggtcagcccaaggccaaccccactgtcactctgtttccgccctcctctgaggagctccaagccaacaaggccacactagtgtgtctgatcagtgacttctacccgggagctgtgacagtggcctggaaggcagatggcagccccgtcaaggcgggagtggagaccaccaaaccctccaaacagagcaacaacaagtacgcggccagcagctacctgagcctgacgcccgagcagtggaagtcccacagaagctacagctgccaggtcacgcatgaagggagcaccgtggagaagactgtggcccctacagaatgttcggcgcgccagactagattttgggtgctggtggtggttggtggagtcctggcttgctatagcttgctagtaacagtggcctttattattttctgggtgaggctgagagtgaagttcagcaggagcgcagacgcccccgcgtaccagcagggccagaaccagctctataacgagctcaatctaggacgaagagaggagtacgatgttttggacaagagacgtggccgggaccctgagatggggggaaagccgcagagaaggaagaaccctcaggaaggcctgtacaatgaactgcagaaagataagatggcggaggcctacagtgagattgggatgaaaggcgagcgccggaggggcaaggggcacgatggcctttaccagggtctcagtacagccaccaaggacacctacgacgcccttcacatgcaggccctgccccctcgcaggagtcagtgcatgtggccccgagagacccagctgctgctggaggtgccgccgtcgaccgaagacgccagaagctgccagttccccgaggaagagcggggcgagcgatcggcagaggagaaggggcggctgggagacctgtgggtgtaa

SEQ ID NO: 16 - protein, 568 aa, synthetic construct
MKHLWFFLLLVAAPRWVLSQVQLQVQLVQSGAEVKKPGSSVKVSCKASGGTFSSYAISWVRQAPGQGLEWMGGIIPIFGTANYAQKFQGRVTITADKSTSTAYMELSSLRSEDTAVYYCARSPRRAYHDAFDIWGQGTMVTVSSGGGGSGGGGSGGGGSSYELTQPPSMSVAPGKTASITCGGDHIGSKSVHWYQQKPGQAPVLVVYDDSDRPSGIPERFKGSNKGNKATLTISGTQAMDEADYYCLAWDSSTAIFGGGTQLTVLVGQPKANPTVTLFPPSSEELQANKATLVCLISDFYPGAVTVAWKADGSPVKAGVETTKPSKQSNNKYAASSYLSLTPEQWKSHRSYSCQVTHEGSTVEKTVAPTECSARQTRFWVLVVVGGVLACYSLLVTVAFIIFWVRLRVKFSRSADAPAYQQGQNQLYNELNLGRREEYDVLDKRRGRDPEMGGKPQRRKNPQEGLYNELQKDKMAEAYSEIGMKGERRRGKGHDGLYQGLSTATKDTYDALHMQALPPRRSQCMWPRETQLLLEVPPSTEDARSCQFPEEERGERSAEEKGRLGDLWV

SEQ ID NO: 17 - DNA, 1707 bp, synthetic construct
  source 1..1707: mol_type = other DNA
atgaaacacctgtggttcttcctcctgctggtggcagctcccagatgggtcctgtcccaggtgcagctgcaggtccagctggtacagtctggggctgaggtgaagaagcctgggtcctcggtgaaggtctcctgcaaggcttctggaggcaccttcagcagctatgctatcagctgggtgcgacaggcccctggacaagggcttgagtggatgggagggatcatccctatctttggtacagcaaactacgcacagaagttccagggcagagtcacgattaccgcggacaaatccacgagcacagcctacatggagctgagcagcctgagatctgaggacacggccgtgtattactgtgcgagatccccccggcgggcatatcatgatgcttttgatatctggggccaagggacaatggtcaccgtctcttcaggtggaggcggttcaggcggaggtggcagcggcggtggcgggagttcctatgagctgactcagccaccctcgatgtcagtggccccaggaaagacggccagcattacctgtggcggagaccatattggaagtaaaagtgttcactggtaccagcagaagccaggccaggcccctgtactggtcgtctatgatgatagcgaccggccctcagggatccctgagcgattcagaggctccaactctgggaacagagccaggctgaccatcagcgggacccaggctatggatgaggctgactattactgtctggcgtgggacagcagcactgcgatcttcggcggaggcacccagctgaccgtcctcgtgggtcagcccaaggccaaccccactgtcactctgtttccgccctcctctgaggagctccaagccaacaaggccacactagtgtgtctgatcagtgacttctacccgggagctgtgacagtggcctggaaggcagatggcagccccgtcaaggcgggagtggagaccaccaaaccctccaaacagagcaacaacaagtacgcggccagcagctacctgagcctgacgcccgagcagtggaagtcccacagaagctacagctgccaggtcacgcatgaagggagcaccgtggagaagactgtggcccctacagaatgttcggcgcgccagactagattttgggtgctggtggtggttggtggagtcctggcttgctatagcttgctagtaacagtggcctttattattttctgggtgaggctgagagtgaagttcagcaggagcgcagacgcccccgcgtaccagcagggccagaaccagctctataacgagctcaatctaggacgaagagaggagtacgatgttttggacaagagacgtggccgggaccctgagatggggggaaagccgcagagaaggaagaaccctcaggaaggcctgtacaatgaactgcagaaagataagatggcggaggcctacagtgagattgggatgaaaggcgagcgccggaggggcaaggggcacgatggcctttaccagggtctcagtacagccaccaaggacacctacgacgcccttcacatgcaggccctgccccctcgcaggagtcagtgcatgtggccccgagagacccagctgctgctggaggtgccgccgtcgaccgaagacgccagaagctgccagttccccgaggaagagcggggcgagcgatcggcagaggagaaggggcggctgggagacctgtgggtgtaa

SEQ ID NO: 18 - protein, 568 aa, synthetic construct
MKHLWFFLLLVAAPRWVLSQVQLQVQLVQSGAEVKKPGSSVKVSCKASGGTFSSYAISWVRQAPGQGLEWMGGIIPIFGTANYAQKFQGRVTITADKSTSTAYMELSSLRSEDTAVYYCARSPRRAYHDAFDIWGQGTMVTVSSGGGGSGGGGSGGGGSSYELTQPPSMSVAPGKTASITCGGDHIGSKSVHWYQQKPGQAPVLVVYDDSDRPSGIPERFRGSNSGNRARLTISGTQAMDEADYYCLAWDSSTAIFGGGTQLTVLVGQPKANPTVTLFPPSSEELQANKATLVCLISDFYPGAVTVAWKADGSPVKAGVETTKPSKQSNNKYAASSYLSLTPEQWKSHRSYSCQVTHEGSTVEKTVAPTECSARQTRFWVLVVVGGVLACYSLLVTVAFIIFWVRLRVKFSRSADAPAYQQGQNQLYNELNLGRREEYDVLDKRRGRDPEMGGKPQRRKNPQEGLYNELQKDKMAEAYSEIGMKGERRRGKGHDGLYQGLSTATKDTYDALHMQALPPRRSQCMWPRETQLLLEVPPSTEDARSCQFPEEERGERSAEEKGRLGDLWV

SEQ ID NO: 19 - DNA, 1707 bp, synthetic construct
  source 1..1707: mol_type = other DNA
atgaaacacctgtggttcttcctcctgctggtggcagctcccagatgggtcctgtcccaggtgcagctgcaggtccagctggtacagtctggggctgaggtgaagaagcctgggtcctcggtgaaggtctcctgcaaggcttctggaggcaccttcagcagctatgctatcagctgggtgcgacaggcccctggacaagggcttgagtggatgggagggatcatccctatctttggtacagcaaactacgcacagaagttccagggcagagtcacgattaccgcggacaaatccacgagcacagcctacatggagctgagcagcctgagatctgaggacacggccgtgtattactgtgcgagatccccccggcgggcatatcatgatgcttttgatatctggggccaagggacaatggtcaccgtctcttcaggtggaggcggttcaggcggaggtggcagcggcggtggcgggagttcctatgagctgactcagccaccctcgatgtcagtggccccaggaaagacggccagcattacctgtggcggagaccatattggaagtaaaagtgttcactggtaccagcagaagccaggccaggcccctgtactggtcgtctatgatgatagcgaccggccctcagggatccctgagcgattctctggcaagaacaaggggaacaaagccactctgaccatcagcgggacccaggctatggatgaggctgactattactgtctggcgtgggacagcagcactgcgatcttcggcggaggcacccagctgaccgtcctcgtgggtcagcccaaggccaaccccactgtcactctgtttccgccctcctctgaggagctccaagccaacaaggccacactagtgtgtctgatcagtgacttctacccgggagctgtgacagtggcctggaaggcagatggcagccccgtcaaggcgggagtggagaccaccaaaccctccaaacagagcaacaacaagtacgcggccagcagctacctgagcctgacgcccgagcagtggaagtcccacagaagctacagctgccaggtcacgcatgaagggagcaccgtggagaagactgtggcccctacagaatgttcggcgcgccagactagattttgggtgctggtggtggttggtggagtcctggcttgctatagcttgctagtaacagtggcctttattattttctgggtgaggctgagagtgaagttcagcaggagcgcagacgcccccgcgtaccagcagggccagaaccagctctataacgagctcaatctaggacgaagagaggagtacgatgttttggacaagagacgtggccgggaccctgagatggggggaaagccgcagagaaggaagaaccctcaggaaggcctgtacaatgaactgcagaaagataagatggcggaggcctacagtgagattgggatgaaaggcgagcgccggaggggcaaggggcacgatggcctttaccagggtctcagtacagccaccaaggacacctacgacgcccttcacatgcaggccctgccccctcgcaggagtcagtgcatgtggccccgagagacccagctgctgctggaggtgccgccgtcgaccgaagacgccagaagctgccagttccccgaggaagagcggggcgagcgatcggcagaggagaaggggcggctgggagacctgtgggtgtaa

SEQ ID NO: 20 - protein, 568 aa, synthetic construct
MKHLWFFLLLVAAPRWVLSQVQLQVQLVQSGAEVKKPGSSVKVSCKASGGTFSSYAISWVRQAPGQGLEWMGGIIPIFGTANYAQKFQGRVTITADKSTSTAYMELSSLRSEDTAVYYCARSPRRAYHDAFDIWGQGTMVTVSSGGGGSGGGGSGGGGSSYELTQPPSMSVAPGKTASITCGGDHIGSKSVHWYQQKPGQAPVLVVYDDSDRPSGIPERFSGKNKGNKATLTISGTQAMDEADYYCLAWDSSTAIFGGGTQLTVLVGQPKANPTVTLFPPSSEELQANKATLVCLISDFYPGAVTVAWKADGSPVKAGVETTKPSKQSNNKYAASSYLSLTPEQWKSHRSYSCQVTHEGSTVEKTVAPTECSARQTRFWVLVVVGGVLACYSLLVTVAFIIFWVRLRVKFSRSADAPAYQQGQNQLYNELNLGRREEYDVLDKRRGRDPEMGGKPQRRKNPQEGLYNELQKDKMAEAYSEIGMKGERRRGKGHDGLYQGLSTATKDTYDALHMQALPPRRSQCMWPRETQLLLEVPPSTEDARSCQFPEEERGERSAEEKGRLGDLWV

SEQ ID NO: 21 - DNA, 1707 bp, synthetic construct
  source 1..1707: mol_type = other DNA
atgaaacacctgtggttcttcctcctgctggtggcagctcccagatgggtcctgtcccaggtgcagctgcaggtccagctggtacagtctggggctgaggtgaagaagcctgggtcctcggtgaaggtctcctgcaaggcttctggaggcaccttcagcagctatgctatcagctgggtgcgacaggcccctggacaagggcttgagtggatgggagggatcatccctatctttggtacagcaaactacgcacagaagttccagggcagagtcacgattaccgcggacaaatccacgagcacagcctacatggagctgagcagcctgagatctgaggacacggccgtgtattactgtgcgagatccccccggcgggcatatcatgatgcttttgatatctggggccaagggacaatggtcaccgtctcttcaggtggaggcggttcaggcggaggtggcagcggcggtggcgggagttcctatgagctgactcagccaccctcgatgtcagtggccccaggaaagacggccagcattacctgtggcggagaccatattggaagtaaaagtgttcactggtaccagcagaagccaggccaggcccctgtactggtcgtctatgatgatagcgaccggccctcagggatccctgagcgattctctggcaggaactctgggaacagagccaggctgaccatcagcgggacccaggctatggatgaggctgactattactgtctggcgtgggacagcagcactgcgatcttcggcggaggcacccagctgaccgtcctcgtgggtcagcccaaggccaaccccactgtcactctgtttccgccctcctctgaggagctccaagccaacaaggccacactagtgtgtctgatcagtgacttctacccgggagctgtgacagtggcctggaaggcagatggcagccccgtcaaggcgggagtggagaccaccaaaccctccaaacagagcaacaacaagtacgcggccagcagctacctgagcctgacgcccgagcagtggaagtcccacagaagctacagctgccaggtcacgcatgaagggagcaccgtggagaagactgtggcccctacagaatgttcggcgcgccagactagattttgggtgctggtggtggttggtggagtcctggcttgctatagcttgctagtaacagtggcctttattattttctgggtgaggctgagagtgaagttcagcaggagcgcagacgcccccgcgtaccagcagggccagaaccagctctataacgagctcaatctaggacgaagagaggagtacgatgttttggacaagagacgtggccgggaccctgagatggggggaaagccgcagagaaggaagaaccctcaggaaggcctgtacaatgaactgcagaaagataagatggcggaggcctacagtgagattgggatgaaaggcgagcgccggaggggcaaggggcacgatggcctttaccagggtctcagtacagccaccaaggacacctacgacgcccttcacatgcaggccctgccccctcgcaggagtcagtgcatgtggccccgagagacccagctgctgctggaggtgccgccgtcgaccgaagacgccagaagctgccagttccccgaggaagagcggggcgagcgatcggcagaggagaaggggcggctgggagacctgtgggtgtaa

SEQ ID NO: 22 - protein, 568 aa, synthetic construct
MKHLWFFLLLVAAPRWVLSQVQLQVQLVQSGAEVKKPGSSVKVSCKASGGTFSSYAISWVRQAPGQGLEWMGGIIPIFGTANYAQKFQGRVTITADKSTSTAYMELSSLRSEDTAVYYCARSPRRAYHDAFDIWGQGTMVTVSSGGGGSGGGGSGGGGSSYELTQPPSMSVAPGKTASITCGGDHIGSKSVHWYQQKPGQAPVLVVYDDSDRPSGIPERFSGRNSGNRARLTISGTQAMDEADYYCLAWDSSTAIFGGGTQLTVLVGQPKANPTVTLFPPSSEELQANKATLVCLISDFYPGAVTVAWKADGSPVKAGVETTKPSKQSNNKYAASSYLSLTPEQWKSHRSYSCQVTHEGSTVEKTVAPTECSARQTRFWVLVVVGGVLACYSLLVTVAFIIFWVRLRVKFSRSADAPAYQQGQNQLYNELNLGRREEYDVLDKRRGRDPEMGGKPQRRKNPQEGLYNELQKDKMAEAYSEIGMKGERRRGKGHDGLYQGLSTATKDTYDALHMQALPPRRSQCMWPRETQLLLEVPPSTEDARSCQFPEEERGERSAEEKGRLGDLWV

SEQ ID NO: 23 - DNA, 1707 bp, synthetic construct
  source 1..1707: mol_type = other DNA
atgaaacacctgtggttcttcctcctgctggtggcagctcccagatgggtcctgtcccaggtgcagctgcaggtccagctggtacagtctggggctgaggtgaagaagcctgggtcctcggtgaaggtctcctgcaaggcttctggaggcaccttcagcagctatgctatcagctgggtgcgacaggcccctggacaagggcttgagtggatgggagggatcatccctatctttggtacagcaaactacgcacagaagttccagggcagagtcacgattaccgcggacaaatccacgagcacagcctacatggagctgagcagcctgagatctgaggacacggccgtgtattactgtgcgagatccccccggcgggcatatcatgatgcttttgatatctggggccaagggacaatggtcaccgtctcttcaggtggaggcggttcaggcggaggtggcagcggcggtggcgggagttcctatgagctgactcagccaccctcgatgtcagtggccccaggaaagacggccagcattacctgtggcggagaccatattggaagtaaaagtgttcactggtaccagcagaagccaggccaggcccctgtactggtcgtctatgatgatagcgaccggccctcagggatccctgagcgattctctggctccaacagagggaacagagccaggctgaccatcagcgggacccaggctatggatgaggctgactattactgtctggcgtgggacagcagcactgcgatcttcggcggaggcacccagctgaccgtcctcgtgggtcagcccaaggccaaccccactgtcactctgtttccgccctcctctgaggagctccaagccaacaaggccacactagtgtgtctgatcagtgacttctacccgggagctgtgacagtggcctggaaggcagatggcagccccgtcaaggcgggagtggagaccaccaaaccctccaaacagagcaacaacaagtacgcggccagcagctacctgagcctgacgcccgagcagtggaagtcccacagaagctacagctgccaggtcacgcatgaagggagcaccgtggagaagactgtggcccctacagaatgttcggcgcgccagactagattttgggtgctggtggtggttggtggagtcctggcttgctatagcttgctagtaacagtggcctttattattttctgggtgaggctgagagtgaagttcagcaggagcgcagacgcccccgcgtaccagcagggccagaaccagctctataacgagctcaatctaggacgaagagaggagtacgatgttttggacaagagacgtggccgggaccctgagatggggggaaagccgcagagaaggaagaaccctcaggaaggcctgtacaatgaactgcagaaagataagatggcggaggcctacagtgagattgggatgaaaggcgagcgccggaggggcaaggggcacgatggcctttaccagggtctcagtacagccaccaaggacacctacgacgcccttcacatgcaggccctgccccctcgcaggagtcagtgcatgtggccccgagagacccagctgctgctggaggtgccgccgtcgaccgaagacgccagaagctgccagttccccgaggaagagcggggcgagcgatcggcagaggagaaggggcggctgggagacctgtgggtgtaa

SEQ ID NO: 24 - protein, 568 aa, synthetic construct
MKHLWFFLLLVAAPRWVLSQVQLQVQLVQSGAEVKKPGSSVKVSCKASGGTFSSYAISWVRQAPGQGLEWMGGIIPIFGTANYAQKFQGRVTITADKSTSTAYMELSSLRSEDTAVYYCARSPRRAYHDAFDIWGQGTMVTVSSGGGGSGGGGSGGGGSSYELTQPPSMSVAPGKTASITCGGDHIGSKSVHWYQQKPGQAPVLVVYDDSDRPSGIPERFSGSNRGNRARLTISGTQAMDEADYYCLAWDSSTAIFGGGTQLTVLVGQPKANPTVTLFPPSSEELQANKATLVCLISDFYPGAVTVAWKADGSPVKAGVETTKPSKQSNNKYAASSYLSLTPEQWKSHRSYSCQVTHEGSTVEKTVAPTECSARQTRFWVLVVVGGVLACYSLLVTVAFIIFWVRLRVKFSRSADAPAYQQGQNQLYNELNLGRREEYDVLDKRRGRDPEMGGKPQRRKNPQEGLYNELQKDKMAEAYSEIGMKGERRRGKGHDGLYQGLSTATKDTYDALHMQALPPRRSQCMWPRETQLLLEVPPSTEDARSCQFPEEERGERSAEEKGRLGDLWV

SEQ ID NO: 25 - DNA, 1707 bp, synthetic construct
  source 1..1707: mol_type = other DNA
atgaaacacctgtggttcttcctcctgctggtggcagctcccagatgggtcctgtcccaggtgcagctgcaggtccagctggtacagtctggggctgaggtgaagaagcctgggtcctcggtgaaggtctcctgcaaggcttctggaggcaccttcagcagctatgctatcagctgggtgcgacaggcccctggacaagggcttgagtggatgggagggatcatccctatctttggtacagcaaactacgcacagaagttccagggcagagtcacgattaccgcggacaaatccacgagcacagcctacatggagctgagcagcctgagatctgaggacacggccgtgtattactgtgcgagatccccccggcgggcatatcatgatgcttttgatatctggggccaagggacaatggtcaccgtctcttcaggtggaggcggttcaggcggaggtggcagcggcggtggcgggagttcctatgagctgactcagccaccctcgatgtcagtggccccaggaaagacggccagcattacctgtggcggagaccatattggaagtaaaagtgttcactggtaccagcagaagccaggccaggcccctgtactggtcgtctatgatgatagcgaccggccctcagggatccctgagcgattcaagggcaagaacaaggggaacaaagccaagctgaccatcagcgggacccaggctatggatgaggctgactattactgtctggcgtgggacagcagcactgcgatcttcggcggaggcacccagctgaccgtcctcgtgggtcagcccaaggccaaccccactgtcactctgtttccgccctcctctgaggagctccaagccaacaaggccacactagtgtgtctgatcagtgacttctacccgggagctgtgacagtggcctggaaggcagatggcagccccgtcaaggcgggagtggagaccaccaaaccctccaaacagagcaacaacaagtacgcggccagcagctacctgagcctgacgcccgagcagtggaagtcccacagaagctacagctgccaggtcacgcatgaagggagcaccgtggagaagactgtggcccctacagaatgttcggcgcgccagactagattttgggtgctggtggtggttggtggagtcctggcttgctatagcttgctagtaacagtggcctttattattttctgggtgaggctgagagtgaagttcagcaggagcgcagacgcccccgcgtaccagcagggccagaaccagctctataacgagctcaatctaggacgaagagaggagtacgatgttttggacaagagacgtggccgggaccctgagatggggggaaagccgcagagaaggaagaaccctcaggaaggcctgtacaatgaactgcagaaagataagatggcggaggcctacagtgagattgggatgaaaggcgagcgccggaggggcaaggggcacgatggcctttaccagggtctcagtacagccaccaaggacacctacgacgcccttcacatgcaggccctgccccctcgcaggagtcagtgcatgtggccccgagagacccagctgctgctggaggtgccgccgtcgaccgaagacgccagaagctgccagttccccgaggaagagcggggcgagcgatcggcagaggagaaggggcggctgggagacctgtgggtgtaa

SEQ ID NO: 26 - protein, 568 aa, synthetic construct
MKHLWFFLLLVAAPRWVLSQVQLQVQLVQSGAEVKKPGSSVKVSCKASGGTFSSYAISWVRQAPGQGLEWMGGIIPIFGTANYAQKFQGRVTITADKSTSTAYMELSSLRSEDTAVYYCARSPRRAYHDAFDIWGQGTMVTVSSGGGGSGGGGSGGGGSSYELTQPPSMSVAPGKTASITCGGDHIGSKSVHWYQQKPGQAPVLVVYDDSDRPSGIPERFKGKNKGNKAKLTISGTQAMDEADYYCLAWDSSTAIFGGGTQLTVLVGQPKANPTVTLFPPSSEELQANKATLVCLISDFYPGAVTVAWKADGSPVKAGVETTKPSKQSNNKYAASSYLSLTPEQWKSHRSYSCQVTHEGSTVEKTVAPTECSARQTRFWVLVVVGGVLACYSLLVTVAFIIFWVRLRVKFSRSADAPAYQQGQNQLYNELNLGRREEYDVLDKRRGRDPEMGGKPQRRKNPQEGLYNELQKDKMAEAYSEIGMKGERRRGKGHDGLYQGLSTATKDTYDALHMQALPPRRSQCMWPRETQLLLEVPPSTEDARSCQFPEEERGERSAEEKGRLGDLWV

SEQ ID NO: 27 - DNA, 1707 bp, synthetic construct
  source 1..1707: mol_type = other DNA
atgaaacacctgtggttcttcctcctgctggtggcagctcccagatgggtcctgtcccaggtgcagctgcaggtccagctggtacagtctggggctgaggtgaagaagcctgggtcctcggtgaaggtctcctgcaaggcttctggaggcaccttcagcagctatgctatcagctgggtgcgacaggcccctggacaagggcttgagtggatgggagggatcatccctatctttggtacagcaaactacgcacagaagttccagggcagagtcacgattaccgcggacaaatccacgagcacagcctacatggagctgagcagcctgagatctgaggacacggccgtgtattactgtgcgagatccccccggcgggcatatcatgatgcttttgatatctggggccaagggacaatggtcaccgtctcttcaggtggaggcggttcaggcggaggtggcagcggcggtggcgggagttcctatgagctgactcagccaccctcgatgtcagtggccccaggaaagacggccagcattacctgtggcggagaccatattggaagtaaaagtgttcactggtaccagcagaagccaggccaggcccctgtactggtcgtctatgatgatagcgaccggccctcagggatccctaggcgattctctggctccaactctgggaacacagccactctgaggatcagggggacccaggctatggatgaggctgactattactgtctggcgtgggacagcagcactgcgatcttcggcggaggcacccagctgaccgtcctcgtgggtcagcccaaggccaaccccactgtcactctgtttccgccctcctctgaggagctccaagccaacaaggccacactagtgtgtctgatcagtgacttctacccgggagctgtgacagtggcctggaaggcagatggcagccccgtcaaggcgggagtggagaccaccaaaccctccaaacagagcaacaacaagtacgcggccagcagctacctgagcctgacgcccgagcagtggaagtcccacagaagctacagctgccaggtcacgcatgaagggagcaccgtggagaagactgtggcccctacagaatgttcggcgcgccagactagattttgggtgctggtggtggttggtggagtcctggcttgctatagcttgctagtaacagtggcctttattattttctgggtgaggctgagagtgaagttcagcaggagcgcagacgcccccgcgtaccagcagggccagaaccagctctataacgagctcaatctaggacgaagagaggagtacgatgttttggacaagagacgtggccgggaccctgagatggggggaaagccgcagagaaggaagaaccctcaggaaggcctgtacaatgaactgcagaaagataagatggcggaggcctacagtgagattgggatgaaaggcgagcgccggaggggcaaggggcacgatggcctttaccagggtctcagtacagccaccaaggacacctacgacgcccttcacatgcaggccctgccccctcgcaggagtcagtgcatgtggccccgagagacccagctgctgctggaggtgccgccgtcgaccgaagacgccagaagctgccagttccccgaggaagagcggggcgagcgatcggcagaggagaaggggcggctgggagacctgtgggtgtaa

SEQ ID NO: 28 - protein, 568 aa, synthetic construct
MKHLWFFLLLVAAPRWVLSQVQLQVQLVQSGAEVKKPGSSVKVSCKASGGTFSSYAISWVRQAPGQGLEWMGGIIPIFGTANYAQKFQGRVTITADKSTSTAYMELSSLRSEDTAVYYCARSPRRAYHDAFDIWGQGTMVTVSSGGGGSGGGGSGGGGSSYELTQPPSMSVAPGKTASITCGGDHIGSKSVHWYQQKPGQAPVLVVYDDSDRPSGIPRRFSGSNSGNTATLRIRGTQAMDEADYYCLAWDSSTAIFGGGTQLTVLVGQPKANPTVTLFPPSSEELQANKATLVCLISDFYPGAVTVAWKADGSPVKAGVETTKPSKQSNNKYAASSYLSLTPEQWKSHRSYSCQVTHEGSTVEKTVAPTECSARQTRFWVLVVVGGVLACYSLLVTVAFIIFWVRLRVKFSRSADAPAYQQGQNQLYNELNLGRREEYDVLDKRRGRDPEMGGKPQRRKNPQEGLYNELQKDKMAEAYSEIGMKGERRRGKGHDGLYQGLSTATKDTYDALHMQALPPRRSQCMWPRETQLLLEVPPSTEDARSCQFPEEERGERSAEEKGRLGDLWV

SEQ ID NO: 29 - DNA, 1707 bp, synthetic construct
  source 1..1707: mol_type = other DNA
atgaaacacctgtggttcttcctcctgctggtggcagctcccagatgggtcctgtcccaggtgcagctgcaggtgcagctggtgcagtctggggctgaggtgaagaagcctgggtcctcggtgaaggtctcctgcaaggcttctggaggcaccttcagcagctatgctatcagctgggtgcgacaggcccctggacaagggcttgagtggatgggagggatcatccctatctttggtacagcaaactacgcacagaagttccagggcagagtcacgattaccgcggacgaatccacgggcacagcctacatggagctgagcagcctgagatctgaggacacggccgtgtattactgtgcgagacaccacagtaactactactactacggtatggacgtctggggccaagggaccacggtcaccgtctcgagaggcggtggcggatcaggtggcggtggaagtggcggtggtgggtccatggcctcctatgagctgactcagccactctcagtgtcagtggccctgggacagacggccaggattacctgtggcggaaacaacattggaagtaaaaatgtgcactggtaccagcagaagccaggccaggcccctgtgctggtcatctatagggatagcaaccggccctctgggatccctgagcgattctctggctccaactcggggaacacggccaccctgaccatcagcagagcccaagccggggatgaggctgactattactgtcaggtgtgggacagcagccatgtcttcggaactgggaccaaggtcaccgtcctaggtcagcccaaggccaaccccactgtcactctgttcccgccctcctctgaggagctccaagccaacaaggccacactagtgtgtctgatcagtgacttctacccgggagctgtgacagtggcctggaaggcagatggcagccccgtcaaggcgggagtggagaccaccaaaccctccaaacagagcaacaacaagtacgcggccagcagctatctgagcctgacgcctgagcagtggaagtcccacagaagctacagctgccaggtcacgcatgaagggagcaccgtggagaagacagtggcccctacagaatgttcggcgcgccagactagattttgggtgctggtggtggttggtggagtcctggcttgctatagcttgctagtaacagtggcctttattattttctgggtgaggctgagagtgaagttcagcaggagcgcagacgcccccgcgtaccagcagggccagaaccagctctataacgagctcaatctaggacgaagagaggagtacgatgttttggacaagagacgtggccgggaccctgagatggggggaaagccgcagagaaggaagaaccctcaggaaggcctgtacaatgaactgcagaaagataagatggcggaggcctacagtgagattgggatgaaaggcgagcgccggaggggcaaggggcacgatggcctttaccagggtctcagtacagccaccaaggacacctacgacgcccttcacatgcaggccctgccccctcgcaggagtcagtgcatgtggccccgagagacccagctgctgctggaggtgccgccgtcgaccgaagacgccagaagctgccagttccccgaggaagagcggggcgagcgatcggcagaggagaaggggcggctgggagacctgtgggtgtaa

SEQ ID NO: 30 - protein, 568 aa, synthetic construct
MKHLWFFLLLVAAPRWVLSQVQLQVQLVQSGAEVKKPGSSVKVSCKASGGTFSSYAISWVRQAPGQGLEWMGGIIPIFGTANYAQKFQGRVTITADESTGTAYMELSSLRSEDTAVYYCARHHSNYYYYGMDVWGQGTTVTVSRGGGGSGGGGSGGGGSMASYELTQPLSVSVALGQTARITCGGNNIGSKNVHWYQQKPGQAPVLVIYRDSNRPSGIPERFSGSNSGNTATLTISRAQAGDEADYYCQVWDSSHVFGTGTKVTVLGQPKANPTVTLFPPSSEELQANKATLVCLISDFYPGAVTVAWKADGSPVKAGVETTKPSKQSNNKYAASSYLSLTPEQWKSHRSYSCQVTHEGSTVEKTVAPTECSARQTRFWVLVVVGGVLACYSLLVTVAFIIFWVRLRVKFSRSADAPAYQQGQNQLYNELNLGRREEYDVLDKRRGRDPEMGGKPQRRKNPQEGLYNELQKDKMAEAYSEIGMKGERRRGKGHDGLYQGLSTATKDTYDALHMQALPPRRSQCMWPRETQLLLEVPPSTEDARSCQFPEEERGERSAEEKGRLGDLWV

SEQ ID NO: 31 - DNA, 1707 bp, synthetic construct
  source 1..1707: mol_type = other DNA
atgaaacacctgtggttcttcctcctgctggtggcagctcccagatgggtcctgtcccaggtgcagctgcaggtgcagctggtgcagtctggggctgaggtgaagaagcctgggtcctcggtgaaggtctcctgcaaggcttctggaggcaccttcagcagctatgctatcagctgggtgcgacaggcccctggacaagggcttgagtggatgggagggatcatccctatctttggtacagcaaactacgcacagaagttccagggcagagtcacgattaccgcggacgaatccacgggcacagcctacatggagctgagcagcctgagatctgaggacacggccgtgtattactgtgcgagacaccacagtaactactactactacggtatggacgtctggggccaagggaccacggtcaccgtctcgagaggcggtggcggatcaggtggcggtggaagtggcggtggtgggtccatggcctcctatgagctgactcagccactctcagtgtcagtggccctgggacagacggccaggattacctgtggcggaaacaacattggaagtaaaaatgtgcactggtaccagcagaagccaggccaggcccctgtgctggtcatctatagggatagcaaccggccctctgggatccctgagcgattccgaggccgaaactcggggaacacggcccgactgaccatcagcagagcccaagccggggatgaggctgactattactgtcaggtgtgggacagcagccatgtcttcggaactgggaccaaggtcaccgtcctaggtcagcccaaggccaaccccactgtcactctgttcccgccctcctctgaggagctccaagccaacaaggccacactagtgtgtctgatcagtgacttctacccgggagctgtgacagtggcctggaaggcagatggcagccccgtcaaggcgggagtggagaccaccaaaccctccaaacagagcaacaacaagtacgcggccagcagctatctgagcctgacgcctgagcagtggaagtcccacagaagctacagctgccaggtcacgcatgaagggagcaccgtggagaagacagtggcccctacagaatgttcggcgcgccagactagattttgggtgctggtggtggttggtggagtcctggcttgctatagcttgctagtaacagtggcctttattattttctgggtgaggctgagagtgaagttcagcaggagcgcagacgcccccgcgtaccagcagggccagaaccagctctataacgagctcaatctaggacgaagagaggagtacgatgttttggacaagagacgtggccgggaccctgagatggggggaaagccgcagagaaggaagaaccctcaggaaggcctgtacaatgaactgcagaaagataagatggcggaggcctacagtgagattgggatgaaaggcgagcgccggaggggcaaggggcacgatggcctttaccagggtctcagtacagccaccaaggacacctacgacgcccttcacatgcaggccctgccccctcgcaggagtcagtgcatgtggccccgagagacccagctgctgctggaggtgccgccgtcgaccgaagacgccagaagctgccagttccccgaggaagagcggggcgagcgatcggcagaggagaaggggcggctgggagacctgtgggtgtaa

SEQ ID NO: 32 - protein, 568 aa, synthetic construct
MKHLWFFLLLVAAPRWVLSQVQLQVQLVQSGAEVKKPGSSVKVSCKASGGTFSSYAISWVRQAPGQGLEWMGGIIPIFGTANYAQKFQGRVTITADESTGTAYMELSSLRSEDTAVYYCARHHSNYYYYGMDVWGQGTTVTVSRGGGGSGGGGSGGGGSMASYELTQPLSVSVALGQTARITCGGNNIGSKNVHWYQQKPGQAPVLVIYRDSNRPSGIPERFRGRNSGNTARLTISRAQAGDEADYYCQVWDSSHVFGTGTKVTVLGQPKANPTVTLFPPSSEELQANKATLVCLISDFYPGAVTVAWKADGSPVKAGVETTKPSKQSNNKYAASSYLSLTPEQWKSHRSYSCQVTHEGSTVEKTVAPTECSARQTRFWVLVVVGGVLACYSLLVTVAFIIFWVRLRVKFSRSADAPAYQQGQNQLYNELNLGRREEYDVLDKRRGRDPEMGGKPQRRKNPQEGLYNELQKDKMAEAYSEIGMKGERRRGKGHDGLYQGLSTATKDTYDALHMQALPPRRSQCMWPRETQLLLEVPPSTEDARSCQFPEEERGERSAEEKGRLGDLWV

SEQ ID NO: 33 - DNA, 1707 bp, synthetic construct
  source 1..1707: mol_type = other DNA
atgaaacacctgtggttcttcctcctgctggtggcagctcccagatgggtcctgtcccaggtgcagctgcaggtgcagctggtgcagtctggggctgaggtgaagaagcctgggtcctcggtgaaggtctcctgcaaggcttctggaggcaccttcagcagctatgctatcagctgggtgcgacaggcccctggacaagggcttgagtggatgggagggatcatccctatctttggtacagcaaactacgcacagaagttccagggcagagtcacgattaccgcggacgaatccacgggcacagcctacatggagctgagcagcctgagatctgaggacacggccgtgtattactgtgcgagacaccacagtaactactactactacggtatggacgtctggggccaagggaccacggtcaccgtctcgagaggcggtggcggatcaggtggcggtggaagtggcggtggtgggtccatggcctcctatgagctgactcagccactctcagtgtcagtggccctgggacagacggccaggattacctgtggcggaaacaacattggaagtaaaaatgtgcactggtaccagcagaagccaggccaggcccctgtgctggtcatctatagggatagcaaccggccctctgggatccctgagcgattccgaggctccaactcggggaaccgagcccgactgaccatcagcagagcccaagccggggatgaggctgactattactgtcaggtgtgggacagcagccatgtcttcggaactgggaccaaggtcaccgtcctaggtcagcccaaggccaaccccactgtcactctgttcccgccctcctctgaggagctccaagccaacaaggccacactagtgtgtctgatcagtgacttctacccgggagctgtgacagtggcctggaaggcagatggcagccccgtcaaggcgggagtggagaccaccaaaccctccaaacagagcaacaacaagtacgcggccagcagctatctgagcctgacgcctgagcagtggaagtcccacagaagctacagctgccaggtcacgcatgaagggagcaccgtggagaagacagtggcccctacagaatgttcggcgcgccagactagattttgggtgctggtggtggttggtggagtcctggcttgctatagcttgctagtaacagtggcctttattattttctgggtgaggctgagagtgaagttcagcaggagcgcagacgcccccgcgtaccagcagggccagaaccagctctataacgagctcaatctaggacgaagagaggagtacgatgttttggacaagagacgtggccgggaccctgagatggggggaaagccgcagagaaggaagaaccctcaggaaggcctgtacaatgaactgcagaaagataagatggcggaggcctacagtgagattgggatgaaaggcgagcgccggaggggcaaggggcacgatggcctttaccagggtctcagtacagccaccaaggacacctacgacgcccttcacatgcaggccctgccccctcgcaggagtcagtgcatgtggccccgagagacccagctgctgctggaggtgccgccgtcgaccgaagacgccagaagctgccagttccccgaggaagagcggggcgagcgatcggcagaggagaaggggcggctgggagacctgtgggtgtaa

SEQ ID NO: 34 - protein, 568 aa, synthetic construct
MKHLWFFLLLVAAPRWVLSQVQLQVQLVQSGAEVKKPGSSVKVSCKASGGTFSSYAISWVRQAPGQGLEWMGGIIPIFGTANYAQKFQGRVTITADESTGTAYMELSSLRSEDTAVYYCARHHSNYYYYGMDVWGQGTTVTVSRGGGGSGGGGSGGGGSMASYELTQPLSVSVALGQTARITCGGNNIGSKNVHWYQQKPGQAPVLVIYRDSNRPSGIPERFRGSNSGNRARLTISRAQAGDEADYYCQVWDSSHVFGTGTKVTVLGQPKANPTVTLFPPSSEELQANKATLVCLISDFYPGAVTVAWKADGSPVKAGVETTKPSKQSNNKYAASSYLSLTPEQWKSHRSYSCQVTHEGSTVEKTVAPTECSARQTRFWVLVVVGGVLACYSLLVTVAFIIFWVRLRVKFSRSADAPAYQQGQNQLYNELNLGRREEYDVLDKRRGRDPEMGGKPQRRKNPQEGLYNELQKDKMAEAYSEIGMKGERRRGKGHDGLYQGLSTATKDTYDALHMQALPPRRSQCMWPRETQLLLEVPPSTEDARSCQFPEEERGERSAEEKGRLGDLWV

SEQ ID NO: 35 - DNA, 1707 bp, synthetic construct
  source 1..1707: mol_type = other DNA
atgaaacacctgtggttcttcctcctgctggtggcagctcccagatgggtcctgtcccaggtgcagctgcaggtgcagctggtgcagtctggggctgaggtgaagaagcctgggtcctcggtgaaggtctcctgcaaggcttctggaggcaccttcagcagctatgctatcagctgggtgcgacaggcccctggacaagggcttgagtggatgggagggatcatccctatctttggtacagcaaactacgcacagaagttccagggcagagtcacgattaccgcggacgaatccacgggcacagcctacatggagctgagcagcctgagatctgaggacacggccgtgtattactgtgcgagacaccacagtaactactactactacggtatggacgtctggggccaagggaccacggtcaccgtctcgagaggcggtggcggatcaggtggcggtggaagtggcggtggtgggtccatggcctcctatgagctgactcagccactctcagtgtcagtggccctgggacagacggccaggattacctgtggcggaaacaacattggaagtaaaaatgtgcactggtaccagcagaagccaggccaggcccctgtgctggtcatctatagggatagcaaccggccctctgggatccctgagcgattctctggcaagaactcggggaacaaggccaagctgaccatcagcagagcccaagccggggatgaggctgactattactgtcaggtgtgggacagcagccatgtcttcggaactgggaccaaggtcaccgtcctaggtcagcccaaggccaaccccactgtcactctgttcccgccctcctctgaggagctccaagccaacaaggccacactagtgtgtctgatcagtgacttctacccgggagctgtgacagtggcctggaaggcagatggcagccccgtcaaggcgggagtggagaccaccaaaccctccaaacagagcaacaacaagtacgcggccagcagctatctgagcctgacgcctgagcagtggaagtcccacagaagctacagctgccaggtcacgcatgaagggagcaccgtggagaagacagtggcccctacagaatgttcggcgcgccagactagattttgggtgctggtggtggttggtggagtcctggcttgctatagcttgctagtaacagtggcctttattattttctgggtgaggctgagagtgaagttcagcaggagcgcagacgcccccgcgtaccagcagggccagaaccagctctataacgagctcaatctaggacgaagagaggagtacgatgttttggacaagagacgtggccgggaccctgagatggggggaaagccgcagagaaggaagaaccctcaggaaggcctgtacaatgaactgcagaaagataagatggcggaggcctacagtgagattgggatgaaaggcgagcgccggaggggcaaggggcacgatggcctttaccagggtctcagtacagccaccaaggacacctacgacgcccttcacatgcaggccctgccccctcgcaggagtcagtgcatgtggccccgagagacccagctgctgctggaggtgccgccgtcgaccgaagacgccagaagctgccagttccccgaggaagagcggggcgagcgatcggcagaggagaaggggcggctgggagacctgtgggtgtaa

SEQ ID NO: 36 - protein, 568 aa, synthetic construct
MKHLWFFLLLVAAPRWVLSQVQLQVQLVQSGAEVKKPGSSVKVSCKASGGTFSSYAISWVRQAPGQGLEWMGGIIPIFGTANYAQKFQGRVTITADESTGTAYMELSSLRSEDTAVYYCARHHSNYYYYGMDVWGQGTTVTVSRGGGGSGGGGSGGGGSMASYELTQPLSVSVALGQTARITCGGNNIGSKNVHWYQQKPGQAPVLVIYRDSNRPSGIPERFSGKNSGNKAKLTISRAQAGDEADYYCQVWDSSHVFGTGTKVTVLGQPKANPTVTLFPPSSEELQANKATLVCLISDFYPGAVTVAWKADGSPVKAGVETTKPSKQSNNKYAASSYLSLTPEQWKSHRSYSCQVTHEGSTVEKTVAPTECSARQTRFWVLVVVGGVLACYSLLVTVAFIIFWVRLRVKFSRSADAPAYQQGQNQLYNELNLGRREEYDVLDKRRGRDPEMGGKPQRRKNPQEGLYNELQKDKMAEAYSEIGMKGERRRGKGHDGLYQGLSTATKDTYDALHMQALPPRRSQCMWPRETQLLLEVPPSTEDARSCQFPEEERGERSAEEKGRLGDLWV

SEQ ID NO: 37 - DNA, 1449 bp, synthetic construct
  source 1..1449: mol_type = other DNA
atgaaacacctgtggttcttcctcctgctggtggcagctcccagatgggtcctgtccgacatccaaatgacgcagactacaagcagcttgtcagcctcactgggagatcgagtcaccattagctgcagagctagccaggatataagcaaatacctgaactggtatcagcagaaacccgatggcaccgtgaagctgctgatctatcacacatctcggctgcatagtggagttccttctcgattttcaggctctggctctgggacagattatagtctgacaatctccaacttggaacaggaggatatagccacctatttctgccagcaagggaataccctcccgtatacatttggaggcggcactaagctggagattacgggtggaggcggttcaggcggaggtggcagcggcggtggcgggagtgaagtgaaactgcaggagtcaggcccaggccttgtcgcaccctcccaatccctgagtgtcacatgcacagtaagcggggtttccctccccgactacggtgtttcatggatcagacagcctccaaggaaaggacttgagtggctcggggtgatttggggtagcgaaaccacctactacaatagcgcgttgaagtccaggctcaccatcatcaaggataacagtaaatcccaggttttcctgaaaatgaatagcctgcagacagatgatactgccatatactactgcgccaaacactattactacggcggatcttatgcgatggactattggggtcaaggtacatctgtaaccgtgagttccatcgaagtgatgtaccctcctccttacctggacaacgagaagtccaacggcaccatcatccacgtgaagggcaagcacctgtgtccttctccactgttccccggacctagcaagcctttttgggtgctggtggtggttggtggagtcctggcttgctatagcttgctagtaacagtggcctttattattttctgggtgaggagtaagaggagcaggctcctgcacagtgactacatgaacatgactccccgccgccccgggcccacccgcaagcattaccagccctatgccccaccacgcgacttcgcagcctatcgctccctgagagtgaagttcagcaggagcgcagacgcccccgcgtaccagcagggccagaaccagctctataacgagctcaatctaggacgaagagaggagtacgatgttttggacaagagacgtggccgggaccctgagatggggggaaagccgcagagaaggaagaaccctcaggaaggcctgtacaatgaactgcagaaagataagatggcggaggcctacagtgagattgggatgaaaggcgagcgccggaggggcaaggggcacgatggcctttaccagggtctcagtacagccaccaaggacacctacgacgcccttcacatgcaggccctgccccctcgctaa

SEQ ID NO: 38 - protein, 482 aa, synthetic construct
MKHLWFFLLLVAAPRWVLSDIQMTQTTSSLSASLGDRVTISCRASQDISKYLNWYQQKPDGTVKLLIYHTSRLHSGVPSRFSGSGSGTDYSLTISNLEQEDIATYFCQQGNTLPYTFGGGTKLEITGGGGSGGGGSGGGGSEVKLQESGPGLVAPSQSLSVTCTVSGVSLPDYGVSWIRQPPRKGLEWLGVIWGSETTYYNSALKSRLTIIKDNSKSQVFLKMNSLQTDDTAIYYCAKHYYYGGSYAMDYWGQGTSVTVSSIEVMYPPPYLDNEKSNGTIIHVKGKHLCPSPLFPGPSKPFWVLVVVGGVLACYSLLVTVAFIIFWVRSKRSRLLHSDYMNMTPRRPGPTRKHYQPYAPPRDFAAYRSLRVKFSRSADAPAYQQGQNQLYNELNLGRREEYDVLDKRRGRDPEMGGKPQRRKNPQEGLYNELQKDKMAEAYSEIGMKGERRRGKGHDGLYQGLSTATKDTYDALHMQALPPR

SEQ ID NO: 39 - DNA, 1449 bp, synthetic construct
  source 1..1449: mol_type = other DNA
atgaaacacctgtggttcttcctcctgctggtggcagctcccagatgggtcctgtccgacatccaaatgacgcagactacaagcagcttgtcagcctcactgggagatcgagtcaccattagctgcagagctagccaggatataagcaaatacctgaactggtatcagcagaaacccgatggcaccgtgaagctgctgatctatcacacatctcggctgcatagtggagttccttctcgatttcgaggccgaggccgagggacacgatatagtctgacaatctccaacttggaacaggaggatatagccacctatttctgccagcaagggaataccctcccgtatacatttggaggcggcactaagctggagattacgggtggaggcggttcaggcggaggtggcagcggcggtggcgggagtgaagtgaaactgcaggagtcaggcccaggccttgtcgcaccctcccaatccctgagtgtcacatgcacagtaagcggggtttccctccccgactacggtgtttcatggatcagacagcctccaaggaaaggacttgagtggctcggggtgatttggggtagcgaaaccacctactacaatagcgcgttgaagtccaggctcaccatcatcaaggataacagtaaatcccaggttttcctgaaaatgaatagcctgcagacagatgatactgccatatactactgcgccaaacactattactacggcggatcttatgcgatggactattggggtcaaggtacatctgtaaccgtgagttccatcgaagtgatgtaccctcctccttacctggacaacgagaagtccaacggcaccatcatccacgtgaagggcaagcacctgtgtccttctccactgttccccggacctagcaagcctttttgggtgctggtggtggttggtggagtcctggcttgctatagcttgctagtaacagtggcctttattattttctgggtgaggagtaagaggagcaggctcctgcacagtgactacatgaacatgactccccgccgccccgggcccacccgcaagcattaccagccctatgccccaccacgcgacttcgcagcctatcgctccctgagagtgaagttcagcaggagcgcagacgcccccgcgtaccagcagggccagaaccagctctataacgagctcaatctaggacgaagagaggagtacgatgttttggacaagagacgtggccgggaccctgagatggggggaaagccgcagagaaggaagaaccctcaggaaggcctgtacaatgaactgcagaaagataagatggcggaggcctacagtgagattgggatgaaaggcgagcgccggaggggcaaggggcacgatggcctttaccagggtctcagtacagccaccaaggacacctacgacgcccttcacatgcaggccctgccccctcgctaa

SEQ ID NO: 40 - protein, 482 aa, synthetic construct
MKHLWFFLLLVAAPRWVLSDIQMTQTTSSLSASLGDRVTISCRASQDISKYLNWYQQKPDGTVKLLIYHTSRLHSGVPSRFRGRGRGTRYSLTISNLEQEDIATYFCQQGNTLPYTFGGGTKLEITGGGGSGGGGSGGGGSEVKLQESGPGLVAPSQSLSVTCTVSGVSLPDYGVSWIRQPPRKGLEWLGVIWGSETTYYNSALKSRLTIIKDNSKSQVFLKMNSLQTDDTAIYYCAKHYYYGGSYAMDYWGQGTSVTVSSIEVMYPPPYLDNEKSNGTIIHVKGKHLCPSPLFPGPSKPFWVLVVVGGVLACYSLLVTVAFIIFWVRSKRSRLLHSDYMNMTPRRPGPTRKHYQPYAPPRDFAAYRSLRVKFSRSADAPAYQQGQNQLYNELNLGRREEYDVLDKRRGRDPEMGGKPQRRKNPQEGLYNELQKDKMAEAYSEIGMKGERRRGKGHDGLYQGLSTATKDTYDALHMQALPPR

SEQ ID NO: 41 - DNA, 1449 bp, synthetic construct
  source 1..1449: mol_type = other DNA
atgaaacacctgtggttcttcctcctgctggtggcagctcccagatgggtcctgtccgacatccaaatgacgcagactacaagcagcttgtcagcctcactgggagatcgagtcaccattagctgcagagctagccaggatataagcaaatacctgaactggtatcagcagaaacccgatggcaccgtgaagctgctgatctatcacacatctcggctgcatagtggagttccttctcgatttcgaggccgaggccgagggacagattatcgactgacaatctccaacttggaacaggaggatatagccacctatttctgccagcaagggaataccctcccgtatacatttggaggcggcactaagctggagattacgggtggaggcggttcaggcggaggtggcagcggcggtggcgggagtgaagtgaaactgcaggagtcaggcccaggccttgtcgcaccctcccaatccctgagtgtcacatgcacagtaagcggggtttccctccccgactacggtgtttcatggatcagacagcctccaaggaaaggacttgagtggctcggggtgatttggggtagcgaaaccacctactacaatagcgcgttgaagtccaggctcaccatcatcaaggataacagtaaatcccaggttttcctgaaaatgaatagcctgcagacagatgatactgccatatactactgcgccaaacactattactacggcggatcttatgcgatggactattggggtcaaggtacatctgtaaccgtgagttccatcgaagtgatgtaccctcctccttacctggacaacgagaagtccaacggcaccatcatccacgtgaagggcaagcacctgtgtccttctccactgttccccggacctagcaagcctttttgggtgctggtggtggttggtggagtcctggcttgctatagcttgctagtaacagtggcctttattattttctgggtgaggagtaagaggagcaggctcctgcacagtgactacatgaacatgactccccgccgccccgggcccacccgcaagcattaccagccctatgccccaccacgcgacttcgcagcctatcgctccctgagagtgaagttcagcaggagcgcagacgcccccgcgtaccagcagggccagaaccagctctataacgagctcaatctaggacgaagagaggagtacgatgttttggacaagagacgtggccgggaccctgagatggggggaaagccgcagagaaggaagaaccctcaggaaggcctgtacaatgaactgcagaaagataagatggcggaggcctacagtgagattgggatgaaaggcgagcgccggaggggcaaggggcacgatggcctttaccagggtctcagtacagccaccaaggacacctacgacgcccttcacatgcaggccctgccccctcgctaa

SEQ ID NO: 42 - protein, 482 aa, synthetic construct
MKHLWFFLLLVAAPRWVLSDIQMTQTTSSLSASLGDRVTISCRASQDISKYLNWYQQKPDGTVKLLIYHTSRLHSGVPSRFRGRGRGTDYRLTISNLEQEDIATYFCQQGNTLPYTFGGGTKLEITGGGGSGGGGSGGGGSEVKLQESGPGLVAPSQSLSVTCTVSGVSLPDYGVSWIRQPPRKGLEWLGVIWGSETTYYNSALKSRLTIIKDNSKSQVFLKMNSLQTDDTAIYYCAKHYYYGGSYAMDYWGQGTSVTVSSIEVMYPPPYLDNEKSNGTIIHVKGKHLCPSPLFPGPSKPFWVLVVVGGVLACYSLLVTVAFIIFWVRSKRSRLLHSDYMNMTPRRPGPTRKHYQPYAPPRDFAAYRSLRVKFSRSADAPAYQQGQNQLYNELNLGRREEYDVLDKRRGRDPEMGGKPQRRKNPQEGLYNELQKDKMAEAYSEIGMKGERRRGKGHDGLYQGLSTATKDTYDALHMQALPPR

SEQ ID NO: 43 - DNA, 1449 bp, synthetic construct
  source 1..1449: mol_type = other DNA
atgaaacacctgtggttcttcctcctgctggtggcagctcccagatgggtcctgtccgacatccaaatgacgcagactacaagcagcttgtcagcctcactgggagatcgagtcaccattagctgcagagctagccaggatataagcaaatacctgaactggtatcagcagaaacccgatggcaccgtgaagctgctgatctatcacacatctcggctgcatagtggagttccttctcgatttcgaggccgaggctctgggacacgatatcgactgacaatctccaacttggaacaggaggatatagccacctatttctgccagcaagggaataccctcccgtatacatttggaggcggcactaagctggagattacgggtggaggcggttcaggcggaggtggcagcggcggtggcgggagtgaagtgaaactgcaggagtcaggcccaggccttgtcgcaccctcccaatccctgagtgtcacatgcacagtaagcggggtttccctccccgactacggtgtttcatggatcagacagcctccaaggaaaggacttgagtggctcggggtgatttggggtagcgaaaccacctactacaatagcgcgttgaagtccaggctcaccatcatcaaggataacagtaaatcccaggttttcctgaaaatgaatagcctgcagacagatgatactgccatatactactgcgccaaacactattactacggcggatcttatgcgatggactattggggtcaaggtacatctgtaaccgtgagttccatcgaagtgatgtaccctcctccttacctggacaacgagaagtccaacggcaccatcatccacgtgaagggcaagcacctgtgtccttctccactgttccccggacctagcaagcctttttgggtgctggtggtggttggtggagtcctggcttgctatagcttgctagtaacagtggcctttattattttctgggtgaggagtaagaggagcaggctcctgcacagtgactacatgaacatgactccccgccgccccgggcccacccgcaagcattaccagccctatgccccaccacgcgacttcgcagcctatcgctccctgagagtgaagttcagcaggagcgcagacgcccccgcgtaccagcagggccagaaccagctctataacgagctcaatctaggacgaagagaggagtacgatgttttggacaagagacgtggccgggaccctgagatggggggaaagccgcagagaaggaagaaccctcaggaaggcctgtacaatgaactgcagaaagataagatggcggaggcctacagtgagattgggatgaaaggcgagcgccggaggggcaaggggcacgatggcctttaccagggtctcagtacagccaccaaggacacctacgacgcccttcacatgcaggccctgccccctcgctaa

SEQ ID NO: 44 - protein, 482 aa, synthetic construct
MKHLWFFLLLVAAPRWVLSDIQMTQTTSSLSASLGDRVTISCRASQDISKYLNWYQQKPDGTVKLLIYHTSRLHSGVPSRFRGRGSGTRYRLTISNLEQEDIATYFCQQGNTLPYTFGGGTKLEITGGGGSGGGGSGGGGSEVKLQESGPGLVAPSQSLSVTCTVSGVSLPDYGVSWIRQPPRKGLEWLGVIWGSETTYYNSALKSRLTIIKDNSKSQVFLKMNSLQTDDTAIYYCAKHYYYGGSYAMDYWGQGTSVTVSSIEVMYPPPYLDNEKSNGTIIHVKGKHLCPSPLFPGPSKPFWVLVVVGGVLACYSLLVTVAFIIFWVRSKRSRLLHSDYMNMTPRRPGPTRKHYQPYAPPRDFAAYRSLRVKFSRSADAPAYQQGQNQLYNELNLGRREEYDVLDKRRGRDPEMGGKPQRRKNPQEGLYNELQKDKMAEAYSEIGMKGERRRGKGHDGLYQGLSTATKDTYDALHMQALPPR

SEQ ID NO: 45 - DNA, 1449 bp, synthetic construct
  source 1..1449: mol_type = other DNA
atgaaacacctgtggttcttcctcctgctggtggcagctcccagatgggtcctgtccgacatccaaatgacgcagactacaagcagcttgtcagcctcactgggagatcgagtcaccattagctgcagagctagccaggatataagcaaatacctgaactggtatcagcagaaacccgatggcaccgtgaagctgctgatctatcacacatctcggctgcatagtggagttccttctcgattttcaggcaggggcagagggacaagatataggctgacaatctccaacttggaacaggaggatatagccacctatttctgccagcaagggaataccctcccgtatacatttggaggcggcactaagctggagattacgggtggaggcggttcaggcggaggtggcagcggcggtggcgggagtgaagtgaaactgcaggagtcaggcccaggccttgtcgcaccctcccaatccctgagtgtcacatgcacagtaagcggggtttccctccccgactacggtgtttcatggatcagacagcctccaaggaaaggacttgagtggctcggggtgatttggggtagcgaaaccacctactacaatagcgcgttgaagtccaggctcaccatcatcaaggataacagtaaatcccaggttttcctgaaaatgaatagcctgcagacagatgatactgccatatactactgcgccaaacactattactacggcggatcttatgcgatggactattggggtcaaggtacatctgtaaccgtgagttccatcgaagtgatgtaccctcctccttacctggacaacgagaagtccaacggcaccatcatccacgtgaagggcaagcacctgtgtccttctccactgttccccggacctagcaagcctttttgggtgctggtggtggttggtggagtcctggcttgctatagcttgctagtaacagtggcctttattattttctgggtgaggagtaagaggagcaggctcctgcacagtgactacatgaacatgactccccgccgccccgggcccacccgcaagcattaccagccctatgccccaccacgcgacttcgcagcctatcgctccctgagagtgaagttcagcaggagcgcagacgcccccgcgtaccagcagggccagaaccagctctataacgagctcaatctaggacgaagagaggagtacgatgttttggacaagagacgtggccgggaccctgagatggggggaaagccgcagagaaggaagaaccctcaggaaggcctgtacaatgaactgcagaaagataagatggcggaggcctacagtgagattgggatgaaaggcgagcgccggaggggcaaggggcacgatggcctttaccagggtctcagtacagccaccaaggacacctacgacgcccttcacatgcaggccctgccccctcgctaa

SEQ ID NO: 46 - protein, 482 aa, synthetic construct
MKHLWFFLLLVAAPRWVLSDIQMTQTTSSLSASLGDRVTISCRASQDISKYLNWYQQKPDGTVKLLIYHTSRLHSGVPSRFSGRGRGTRYRLTISNLEQEDIATYFCQQGNTLPYTFGGGTKLEITGGGGSGGGGSGGGGSEVKLQESGPGLVAPSQSLSVTCTVSGVSLPDYGVSWIRQPPRKGLEWLGVIWGSETTYYNSALKSRLTIIKDNSKSQVFLKMNSLQTDDTAIYYCAKHYYYGGSYAMDYWGQGTSVTVSSIEVMYPPPYLDNEKSNGTIIHVKGKHLCPSPLFPGPSKPFWVLVVVGGVLACYSLLVTVAFIIFWVRSKRSRLLHSDYMNMTPRRPGPTRKHYQPYAPPRDFAAYRSLRVKFSRSADAPAYQQGQNQLYNELNLGRREEYDVLDKRRGRDPEMGGKPQRRKNPQEGLYNELQKDKMAEAYSEIGMKGERRRGKGHDGLYQGLSTATKDTYDALHMQALPPR

SEQ ID NO: 47 - DNA, 1449 bp, synthetic construct
  source 1..1449: mol_type = other DNA
atgaaacacctgtggttcttcctcctgctggtggcagctcccagatgggtcctgtccgacatccaaatgacgcagactacaagcagcttgtcagcctcactgggagatcgagtcaccattagctgcagagctagccaggatataagcaaatacctgaactggtatcagcagaaacccgatggcaccgtgaagctgctgatctatcacacatctcggctgcatagtggagttcctagacgatttagaggcagaggctctgggacagattatagtctgacaatctccaacttggaacaggaggatatagccacctatttctgccagcaagggaataccctcccgtatacatttggaggcggcactaagctggagattacgggtggaggcggttcaggcggaggtggcagcggcggtggcgggagtgaagtgaaactgcaggagtcaggcccaggccttgtcgcaccctcccaatccctgagtgtcacatgcacagtaagcggggtttccctccccgactacggtgtttcatggatcagacagcctccaaggaaaggacttgagtggctcggggtgatttggggtagcgaaaccacctactacaatagcgcgttgaagtccaggctcaccatcatcaaggataacagtaaatcccaggttttcctgaaaatgaatagcctgcagacagatgatactgccatatactactgcgccaaacactattactacggcggatcttatgcgatggactattggggtcaaggtacatctgtaaccgtgagttccatcgaagtgatgtaccctcctccttacctggacaacgagaagtccaacggcaccatcatccacgtgaagggcaagcacctgtgtccttctccactgttccccggacctagcaagcctttttgggtgctggtggtggttggtggagtcctggcttgctatagcttgctagtaacagtggcctttattattttctgggtgaggagtaagaggagcaggctcctgcacagtgactacatgaacatgactccccgccgccccgggcccacccgcaagcattaccagccctatgccccaccacgcgacttcgcagcctatcgctccctgagagtgaagttcagcaggagcgcagacgcccccgcgtaccagcagggccagaaccagctctataacgagctcaatctaggacgaagagaggagtacgatgttttggacaagagacgtggccgggaccctgagatggggggaaagccgcagagaaggaagaaccctcaggaaggcctgtacaatgaactgcagaaagataagatggcggaggcctacagtgagattgggatgaaaggcgagcgccggaggggcaaggggcacgatggcctttaccagggtctcagtacagccaccaaggacacctacgacgcccttcacatgcaggccctgccccctcgctaa

SEQ ID NO: 48 - protein, 482 aa, synthetic construct
MKHLWFFLLLVAAPRWVLSDIQMTQTTSSLSASLGDRVTISCRASQDISKYLNWYQQKPDGTVKLLIYHTSRLHSGVPRRFRGRGSGTDYSLTISNLEQEDIATYFCQQGNTLPYTFGGGTKLEITGGGGSGGGGSGGGGSEVKLQESGPGLVAPSQSLSVTCTVSGVSLPDYGVSWIRQPPRKGLEWLGVIWGSETTYYNSALKSRLTIIKDNSKSQVFLKMNSLQTDDTAIYYCAKHYYYGGSYAMDYWGQGTSVTVSSIEVMYPPPYLDNEKSNGTIIHVKGKHLCPSPLFPGPSKPFWVLVVVGGVLACYSLLVTVAFIIFWVRSKRSRLLHSDYMNMTPRRPGPTRKHYQPYAPPRDFAAYRSLRVKFSRSADAPAYQQGQNQLYNELNLGRREEYDVLDKRRGRDPEMGGKPQRRKNPQEGLYNELQKDKMAEAYSEIGMKGERRRGKGHDGLYQGLSTATKDTYDALHMQALPPR

SEQ ID NO: 49 - DNA, 1449 bp, synthetic construct
  source 1..1449: mol_type = other DNA
atgaaacacctgtggttcttcctcctgctggtggcagctcccagatgggtcctgtccgacatccaaatgacgcagactacaagcagcttgtcagcctcactgggagatcgagtcaccattagctgcagagctagccaggatataagcaaatacctgaactggtatcagcagaaacccgatggcaccgtgaagctgctgatctatcacacatctcggctgcatagtggagttccttctcgatttaagggcaagggctctgggacaaaatatagtctgacaatctccaacttggaacaggaggatatagccacctatttctgccagcaagggaataccctcccgtatacatttggaggcggcactaagctggagattacgggtggaggcggttcaggcggaggtggcagcggcggtggcgggagtgaagtgaaactgcaggagtcaggcccaggccttgtcgcaccctcccaatccctgagtgtcacatgcacagtaagcggggtttccctccccgactacggtgtttcatggatcagacagcctccaaggaaaggacttgagtggctcggggtgatttggggtagcgaaaccacctactacaatagcgcgttgaagtccaggctcaccatcatcaaggataacagtaaatcccaggttttcctgaaaatgaatagcctgcagacagatgatactgccatatactactgcgccaaacactattactacggcggatcttatgcgatggactattggggtcaaggtacatctgtaaccgtgagttccatcgaagtgatgtaccctcctccttacctggacaacgagaagtccaacggcaccatcatccacgtgaagggcaagcacctgtgtccttctccactgttccccggacctagcaagcctttttgggtgctggtggtggttggtggagtcctggcttgctatagcttgctagtaacagtggcctttattattttctgggtgaggagtaagaggagcaggctcctgcacagtgactacatgaacatgactccccgccgccccgggcccacccgcaagcattaccagccctatgccccaccacgcgacttcgcagcctatcgctccctgagagtgaagttcagcaggagcgcagacgcccccgcgtaccagcagggccagaaccagctctataacgagctcaatctaggacgaagagaggagtacgatgttttggacaagagacgtggccgggaccctgagatggggggaaagccgcagagaaggaagaaccctcaggaaggcctgtacaatgaactgcagaaagataagatggcggaggcctacagtgagattgggatgaaaggcgagcgccggaggggcaaggggcacgatggcctttaccagggtctcagtacagccaccaaggacacctacgacgcccttcacatgcaggccctgccccctcgctaa

SEQ ID NO: 50 - protein, 482 aa, synthetic construct
MKHLWFFLLLVAAPRWVLSDIQMTQTTSSLSASLGDRVTISCRASQDISKYLNWYQQKPDGTVKLLIYHTSRLHSGVPSRFKGKGSGTKYSLTISNLEQEDIATYFCQQGNTLPYTFGGGTKLEITGGGGSGGGGSGGGGSEVKLQESGPGLVAPSQSLSVTCTVSGVSLPDYGVSWIRQPPRKGLEWLGVIWGSETTYYNSALKSRLTIIKDNSKSQVFLKMNSLQTDDTAIYYCAKHYYYGGSYAMDYWGQGTSVTVSSIEVMYPPPYLDNEKSNGTIIHVKGKHLCPSPLFPGPSKPFWVLVVVGGVLACYSLLVTVAFIIFWVRSKRSRLLHSDYMNMTPRRPGPTRKHYQPYAPPRDFAAYRSLRVKFSRSADAPAYQQGQNQLYNELNLGRREEYDVLDKRRGRDPEMGGKPQRRKNPQEGLYNELQKDKMAEAYSEIGMKGERRRGKGHDGLYQGLSTATKDTYDALHMQALPPR

SEQ ID NO: 51 - DNA, 1449 bp, synthetic construct
  source 1..1449: mol_type = other DNA
atgaaacacctgtggttcttcctcctgctggtggcagctcccagatgggtcctgtccgacatccaaatgacgcagactacaagcagcttgtcagcctcactgggagatcgagtcaccattagctgcagagctagccaggatataagcaaatacctgaactggtatcagcagaaacccgatggcaccgtgaagctgctgatctatcacacatctcggctgcatagtggagttccttctcgatttagaggcaggggctctgggacagattataggctgacaatctccaacttggaacaggaggatatagccacctatttctgccagcaagggaataccctcccgtatacatttggaggcggcactaagctggagattacgggtggaggcggttcaggcggaggtggcagcggcggtggcgggagtgaagtgaaactgcaggagtcaggcccaggccttgtcgcaccctcccaatccctgagtgtcacatgcacagtaagcggggtttccctccccgactacggtgtttcatggatcagacagcctccaaggaaaggacttgagtggctcggggtgatttggggtagcgaaaccacctactacaatagcgcgttgaagtccaggctcaccatcatcaaggataacagtaaatcccaggttttcctgaaaatgaatagcctgcagacagatgatactgccatatactactgcgccaaacactattactacggcggatcttatgcgatggactattggggtcaaggtacatctgtaaccgtgagttccatcgaagtgatgtaccctcctccttacctggacaacgagaagtccaacggcaccatcatccacgtgaagggcaagcacctgtgtccttctccactgttccccggacctagcaagcctttttgggtgctggtggtggttggtggagtcctggcttgctatagcttgctagtaacagtggcctttattattttctgggtgaggagtaagaggagcaggctcctgcacagtgactacatgaacatgactccccgccgccccgggcccacccgcaagcattaccagccctatgccccaccacgcgacttcgcagcctatcgctccctgagagtgaagttcagcaggagcgcagacgcccccgcgtaccagcagggccagaaccagctctataacgagctcaatctaggacgaagagaggagtacgatgttttggacaagagacgtggccgggaccctgagatggggggaaagccgcagagaaggaagaaccctcaggaaggcctgtacaatgaactgcagaaagataagatggcggaggcctacagtgagattgggatgaaaggcgagcgccggaggggcaaggggcacgatggcctttaccagggtctcagtacagccaccaaggacacctacgacgcccttcacatgcaggccctgccccctcgctaa

SEQ ID NO: 52 - protein, 482 aa, synthetic construct
MKHLWFFLLLVAAPRWVLSDIQMTQTTSSLSASLGDRVTISCRASQDISKYLNWYQQKPDGTVKLLIYHTSRLHSGVPSRFRGRGSGTDYRLTISNLEQEDIATYFCQQGNTLPYTFGGGTKLEITGGGGSGGGGSGGGGSEVKLQESGPGLVAPSQSLSVTCTVSGVSLPDYGVSWIRQPPRKGLEWLGVIWGSETTYYNSALKSRLTIIKDNSKSQVFLKMNSLQTDDTAIYYCAKHYYYGGSYAMDYWGQGTSVTVSSIEVMYPPPYLDNEKSNGTIIHVKGKHLCPSPLFPGPSKPFWVLVVVGGVLACYSLLVTVAFIIFWVRSKRSRLLHSDYMNMTPRRPGPTRKHYQPYAPPRDFAAYRSLRVKFSRSADAPAYQQGQNQLYNELNLGRREEYDVLDKRRGRDPEMGGKPQRRKNPQEGLYNELQKDKMAEAYSEIGMKGERRRGKGHDGLYQGLSTATKDTYDALHMQALPPR

SEQ ID NO: 53 - DNA, 1449 bp, synthetic construct
  source 1..1449: mol_type = other DNA
atgaaacacctgtggttcttcctcctgctggtggcagctcccagatgggtcctgtccgacatccaaatgacgcagactacaagcagcttgtcagcctcactgggagatcgagtcaccattagctgcagagctagccaggatataagcaaatacctgaactggtatcagcagaaacccgatggcaccgtgaagctgctgatctatcacacatctcggctgcatagtggagttccttctcgatttagaggctctggcagagggacaagatatagtctgacaatctccaacttggaacaggaggatatagccacctatttctgccagcaagggaataccctcccgtatacatttggaggcggcactaagctggagattacgggtggaggcggttcaggcggaggtggcagcggcggtggcgggagtgaagtgaaactgcaggagtcaggcccaggccttgtcgcaccctcccaatccctgagtgtcacatgcacagtaagcggggtttccctccccgactacggtgtttcatggatcagacagcctccaaggaaaggacttgagtggctcggggtgatttggggtagcgaaaccacctactacaatagcgcgttgaagtccaggctcaccatcatcaaggataacagtaaatcccaggttttcctgaaaatgaatagcctgcagacagatgatactgccatatactactgcgccaaacactattactacggcggatcttatgcgatggactattggggtcaaggtacatctgtaaccgtgagttccatcgaagtgatgtaccctcctccttacctggacaacgagaagtccaacggcaccatcatccacgtgaagggcaagcacctgtgtccttctccactgttccccggacctagcaagcctttttgggtgctggtggtggttggtggagtcctggcttgctatagcttgctagtaacagtggcctttattattttctgggtgaggagtaagaggagcaggctcctgcacagtgactacatgaacatgactccccgccgccccgggcccacccgcaagcattaccagccctatgccccaccacgcgacttcgcagcctatcgctccctgagagtgaagttcagcaggagcgcagacgcccccgcgtaccagcagggccagaaccagctctataacgagctcaatctaggacgaagagaggagtacgatgttttggacaagagacgtggccgggaccctgagatggggggaaagccgcagagaaggaagaaccctcaggaaggcctgtacaatgaactgcagaaagataagatggcggaggcctacagtgagattgggatgaaaggcgagcgccggaggggcaaggggcacgatggcctttaccagggtctcagtacagccaccaaggacacctacgacgcccttcacatgcaggccctgccccctcgctaa

SEQ ID NO: 54 - skipped

SEQ ID NO: 55 - DNA, 1449 bp, synthetic construct
  source 1..1449: mol_type = other DNA
atgaaacacctgtggttcttcctcctgctggtggcagctcccagatgggtcctgtccgacatccaaatgacgcagactacaagcagcttgtcagcctcactgggagatcgagtcaccattagctgcagagctagccaggatataagcaaatacctgaactggtatcagcagaaacccgatggcaccgtgaagctgctgatctatcacacatctcggctgcatagtggagttccttctcgatttagaggctctggctctgggacaagatataggctgacaatctccaacttggaacaggaggatatagccacctatttctgccagcaagggaataccctcccgtatacatttggaggcggcactaagctggagattacgggtggaggcggttcaggcggaggtggcagcggcggtggcgggagtgaagtgaaactgcaggagtcaggcccaggccttgtcgcaccctcccaatccctgagtgtcacatgcacagtaagcggggtttccctccccgactacggtgtttcatggatcagacagcctccaaggaaaggacttgagtggctcggggtgatttggggtagcgaaaccacctactacaatagcgcgttgaagtccaggctcaccatcatcaaggataacagtaaatcccaggttttcctgaaaatgaatagcctgcagacagatgatactgccatatactactgcgccaaacactattactacggcggatcttatgcgatggactattggggtcaaggtacatctgtaaccgtgagttccatcgaagtgatgtaccctcctccttacctggacaacgagaagtccaacggcaccatcatccacgtgaagggcaagcacctgtgtccttctccactgttccccggacctagcaagcctttttgggtgctggtggtggttggtggagtcctggcttgctatagcttgctagtaacagtggcctttattattttctgggtgaggagtaagaggagcaggctcctgcacagtgactacatgaacatgactccccgccgccccgggcccacccgcaagcattaccagccctatgccccaccacgcgacttcgcagcctatcgctccctgagagtgaagttcagcaggagcgcagacgcccccgcgtaccagcagggccagaaccagctctataacgagctcaatctaggacgaagagaggagtacgatgttttggacaagagacgtggccgggaccctgagatggggggaaagccgcagagaaggaagaaccctcaggaaggcctgtacaatgaactgcagaaagataagatggcggaggcctacagtgagattgggatgaaaggcgagcgccggaggggcaaggggcacgatggcctttaccagggtctcagtacagccaccaaggacacctacgacgcccttcacatgcaggccctgccccctcgctaa

SEQ ID NO: 56 - protein, 482 aa, synthetic construct
MKHLWFFLLLVAAPRWVLSDIQMTQTTSSLSASLGDRVTISCRASQDISKYLNWYQQKPDGTVKLLIYHTSRLHSGVPSRFRGSGSGTRYRLTISNLEQEDIATYFCQQGNTLPYTFGGGTKLEITGGGGSGGGGSGGGGSEVKLQESGPGLVAPSQSLSVTCTVSGVSLPDYGVSWIRQPPRKGLEWLGVIWGSETTYYNSALKSRLTIIKDNSKSQVFLKMNSLQTDDTAIYYCAKHYYYGGSYAMDYWGQGTSVTVSSIEVMYPPPYLDNEKSNGTIIHVKGKHLCPSPLFPGPSKPFWVLVVVGGVLACYSLLVTVAFIIFWVRSKRSRLLHSDYMNMTPRRPGPTRKHYQPYAPPRDFAAYRSLRVKFSRSADAPAYQQGQNQLYNELNLGRREEYDVLDKRRGRDPEMGGKPQRRKNPQEGLYNELQKDKMAEAYSEIGMKGERRRGKGHDGLYQGLSTATKDTYDALHMQALPPR

SEQ ID NO: 57 - DNA, 1449 bp, synthetic construct
  source 1..1449: mol_type = other DNA
atgaaacacctgtggttcttcctcctgctggtggcagctcccagatgggtcctgtccgacatccaaatgacgcagactacaagcagcttgtcagcctcactgggagatcgagtcaccattagctgcagagctagccaggatataagcaaatacctgaactggtatcagcagaaacccgatggcaccgtgaagctgctgatctatcacacatctcggctgcatagtggagttccttctcgattttcaggcaggggcagagggacaagatatagtctgacaatctccaacttggaacaggaggatatagccacctatttctgccagcaagggaataccctcccgtatacatttggaggcggcactaagctggagattacgggtggaggcggttcaggcggaggtggcagcggcggtggcgggagtgaagtgaaactgcaggagtcaggcccaggccttgtcgcaccctcccaatccctgagtgtcacatgcacagtaagcggggtttccctccccgactacggtgtttcatggatcagacagcctccaaggaaaggacttgagtggctcggggtgatttggggtagcgaaaccacctactacaatagcgcgttgaagtccaggctcaccatcatcaaggataacagtaaatcccaggttttcctgaaaatgaatagcctgcagacagatgatactgccatatactactgcgccaaacactattactacggcggatcttatgcgatggactattggggtcaaggtacatctgtaaccgtgagttccatcgaagtgatgtaccctcctccttacctggacaacgagaagtccaacggcaccatcatccacgtgaagggcaagcacctgtgtccttctccactgttccccggacctagcaagcctttttgggtgctggtggtggttggtggagtcctggcttgctatagcttgctagtaacagtggcctttattattttctgggtgaggagtaagaggagcaggctcctgcacagtgactacatgaacatgactccccgccgccccgggcccacccgcaagcattaccagccctatgccccaccacgcgacttcgcagcctatcgctccctgagagtgaagttcagcaggagcgcagacgcccccgcgtaccagcagggccagaaccagctctataacgagctcaatctaggacgaagagaggagtacgatgttttggacaagagacgtggccgggaccctgagatggggggaaagccgcagagaaggaagaaccctcaggaaggcctgtacaatgaactgcagaaagataagatggcggaggcctacagtgagattgggatgaaaggcgagcgccggaggggcaaggggcacgatggcctttaccagggtctcagtacagccaccaaggacacctacgacgcccttcacatgcaggccctgccccctcgctaa

SEQ ID NO: 58 - protein, 482 aa, synthetic construct
MKHLWFFLLLVAAPRWVLSDIQMTQTTSSLSASLGDRVTISCRASQDISKYLNWYQQKPDGTVKLLIYHTSRLHSGVPSRFSGRGRGTRYSLTISNLEQEDIATYFCQQGNTLPYTFGGGTKLEITGGGGSGGGGSGGGGSEVKLQESGPGLVAPSQSLSVTCTVSGVSLPDYGVSWIRQPPRKGLEWLGVIWGSETTYYNSALKSRLTIIKDNSKSQVFLKMNSLQTDDTAIYYCAKHYYYGGSYAMDYWGQGTSVTVSSIEVMYPPPYLDNEKSNGTIIHVKGKHLCPSPLFPGPSKPFWVLVVVGGVLACYSLLVTVAFIIFWVRSKRSRLLHSDYMNMTPRRPGPTRKHYQPYAPPRDFAAYRSLRVKFSRSADAPAYQQGQNQLYNELNLGRREEYDVLDKRRGRDPEMGGKPQRRKNPQEGLYNELQKDKMAEAYSEIGMKGERRRGKGHDGLYQGLSTATKDTYDALHMQALPPR

SEQ ID NO: 59 - DNA, 1449 bp, synthetic construct
  source 1..1449: mol_type = other DNA
atgaaacacctgtggttcttcctcctgctggtggcagctcccagatgggtcctgtccgacatccaaatgacgcagactacaagcagcttgtcagcctcactgggagatcgagtcaccattagctgcagagctagccaggatataagcaaatacctgaactggtatcagcagaaacccgatggcaccgtgaagctgctgatctatcacacatctcggctgcatagtggagttccttctcgattttcaggcaggggcagagggacagattataggctgacaatctccaacttggaacaggaggatatagccacctatttctgccagcaagggaataccctcccgtatacatttggaggcggcactaagctggagattacgggtggaggcggttcaggcggaggtggcagcggcggtggcgggagtgaagtgaaactgcaggagtcaggcccaggccttgtcgcaccctcccaatccctgagtgtcacatgcacagtaagcggggtttccctccccgactacggtgtttcatggatcagacagcctccaaggaaaggacttgagtggctcggggtgatttggggtagcgaaaccacctactacaatagcgcgttgaagtccaggctcaccatcatcaaggataacagtaaatcccaggttttcctgaaaatgaatagcctgcagacagatgatactgccatatactactgcgccaaacactattactacggcggatcttatgcgatggactattggggtcaaggtacatctgtaaccgtgagttccatcgaagtgatgtaccctcctccttacctggacaacgagaagtccaacggcaccatcatccacgtgaagggcaagcacctgtgtccttctccactgttccccggacctagcaagcctttttgggtgctggtggtggttggtggagtcctggcttgctatagcttgctagtaacagtggcctttattattttctgggtgaggagtaagaggagcaggctcctgcacagtgactacatgaacatgactccccgccgccccgggcccacccgcaagcattaccagccctatgccccaccacgcgacttcgcagcctatcgctccctgagagtgaagttcagcaggagcgcagacgcccccgcgtaccagcagggccagaaccagctctataacgagctcaatctaggacgaagagaggagtacgatgttttggacaagagacgtggccgggaccctgagatggggggaaagccgcagagaaggaagaaccctcaggaaggcctgtacaatgaactgcagaaagataagatggcggaggcctacagtgagattgggatgaaaggcgagcgccggaggggcaaggggcacgatggcctttaccagggtctcagtacagccaccaaggacacctacgacgcccttcacatgcaggccctgccccctcgctaa

SEQ ID NO: 60 - protein, 482 aa, synthetic construct
MKHLWFFLLLVAAPRWVLSDIQMTQTTSSLSASLGDRVTISCRASQDISKYLNWYQQKPDGTVKLLIYHTSRLHSGVPSRFSGRGRGTDYRLTISNLEQEDIATYFCQQGNTLPYTFGGGTKLEITGGGGSGGGGSGGGGSEVKLQESGPGLVAPSQSLSVTCTVSGVSLPDYGVSWIRQPPRKGLEWLGVIWGSETTYYNSALKSRLTIIKDNSKSQVFLKMNSLQTDDTAIYYCAKHYYYGGSYAMDYWGQGTSVTVSSIEVMYPPPYLDNEKSNGTIIHVKGKHLCPSPLFPGPSKPFWVLVVVGGVLACYSLLVTVAFIIFWVRSKRSRLLHSDYMNMTPRRPGPTRKHYQPYAPPRDFAAYRSLRVKFSRSADAPAYQQGQNQLYNELNLGRREEYDVLDKRRGRDPEMGGKPQRRKNPQEGLYNELQKDKMAEAYSEIGMKGERRRGKGHDGLYQGLSTATKDTYDALHMQALPPR

SEQ ID NO: 61 - DNA, 1449 bp, synthetic construct
  source 1..1449: mol_type = other DNA
atgaaacacctgtggttcttcctcctgctggtggcagctcccagatgggtcctgtccgacatccaaatgacgcagactacaagcagcttgtcagcctcactgggagatcgagtcaccattagctgcagagctagccaggatataagcaaatacctgaactggtatcagcagaaacccgatggcaccgtgaagctgctgatctatcacacatctcggctgcatagtggagttccttctcgatttaagggcaagggctctgggacaaaatataagctgacaatctccaacttggaacaggaggatatagccacctatttctgccagcaagggaataccctcccgtatacatttggaggcggcactaagctggagattacgggtggaggcggttcaggcggaggtggcagcggcggtggcgggagtgaagtgaaactgcaggagtcaggcccaggccttgtcgcaccctcccaatccctgagtgtcacatgcacagtaagcggggtttccctccccgactacggtgtttcatggatcagacagcctccaaggaaaggacttgagtggctcggggtgatttggggtagcgaaaccacctactacaatagcgcgttgaagtccaggctcaccatcatcaaggataacagtaaatcccaggttttcctgaaaatgaatagcctgcagacagatgatactgccatatactactgcgccaaacactattactacggcggatcttatgcgatggactattggggtcaaggtacatctgtaaccgtgagttccatcgaagtgatgtaccctcctccttacctggacaacgagaagtccaacggcaccatcatccacgtgaagggcaagcacctgtgtccttctccactgttccccggacctagcaagcctttttgggtgctggtggtggttggtggagtcctggcttgctatagcttgctagtaacagtggcctttattattttctgggtgaggagtaagaggagcaggctcctgcacagtgactacatgaacatgactccccgccgccccgggcccacccgcaagcattaccagccctatgccccaccacgcgacttcgcagcctatcgctccctgagagtgaagttcagcaggagcgcagacgcccccgcgtaccagcagggccagaaccagctctataacgagctcaatctaggacgaagagaggagtacgatgttttggacaagagacgtggccgggaccctgagatggggggaaagccgcagagaaggaagaaccctcaggaaggcctgtacaatgaactgcagaaagataagatggcggaggcctacagtgagattgggatgaaaggcgagcgccggaggggcaaggggcacgatggcctttaccagggtctcagtacagccaccaaggacacctacgacgcccttcacatgcaggccctgccccctcgctaa

SEQ ID NO: 62 - protein, 482 aa, synthetic construct
MKHLWFFLLLVAAPRWVLSDIQMTQTTSSLSASLGDRVTISCRASQDISKYLNWYQQKPDGTVKLLIYHTSRLHSGVPSRFKGKGSGTKYKLTISNLEQEDIATYFCQQGNTLPYTFGGGTKLEITGGGGSGGGGSGGGGSEVKLQESGPGLVAPSQSLSVTCTVSGVSLPDYGVSWIRQPPRKGLEWLGVIWGSETTYYNSALKSRLTIIKDNSKSQVFLKMNSLQTDDTAIYYCAKHYYYGGSYAMDYWGQGTSVTVSSIEVMYPPPYLDNEKSNGTIIHVKGKHLCPSPLFPGPSKPFWVLVVVGGVLACYSLLVTVAFIIFWVRSKRSRLLHSDYMNMTPRRPGPTRKHYQPYAPPRDFAAYRSLRVKFSRSADAPAYQQGQNQLYNELNLGRREEYDVLDKRRGRDPEMGGKPQRRKNPQEGLYNELQKDKMAEAYSEIGMKGERRRGKGHDGLYQGLSTATKDTYDALHMQALPPR

SEQ ID NO: 63 - DNA, 1449 bp, synthetic construct
  source 1..1449: mol_type = other DNA
atgaaacacctgtggttcttcctcctgctggtggcagctcccagatgggtcctgtccgacatccaaatgacgcagactacaagcagcttgtcagcctcactgggagatcgagtcaccattagctgcagagctagccaggatataagcaaatacctgaactggtatcagcagaaacccgatggcaccgtgaagctgctgatctatcacacatctcggctgcatagtggagttccttctcgattttcaggcaagggcaaggggacaaaatataagctgacaatctccaacttggaacaggaggatatagccacctatttctgccagcaagggaataccctcccgtatacatttggaggcggcactaagctggagattacgggtggaggcggttcaggcggaggtggcagcggcggtggcgggagtgaagtgaaactgcaggagtcaggcccaggccttgtcgcaccctcccaatccctgagtgtcacatgcacagtaagcggggtttccctccccgactacggtgtttcatggatcagacagcctccaaggaaaggacttgagtggctcggggtgatttggggtagcgaaaccacctactacaatagcgcgttgaagtccaggctcaccatcatcaaggataacagtaaatcccaggttttcctgaaaatgaatagcctgcagacagatgatactgccatatactactgcgccaaacactattactacggcggatcttatgcgatggactattggggtcaaggtacatctgtaaccgtgagttccatcgaagtgatgtaccctcctccttacctggacaacgagaagtccaacggcaccatcatccacgtgaagggcaagcacctgtgtccttctccactgttccccggacctagcaagcctttttgggtgctggtggtggttggtggagtcctggcttgctatagcttgctagtaacagtggcctttattattttctgggtgaggagtaagaggagcaggctcctgcacagtgactacatgaacatgactccccgccgccccgggcccacccgcaagcattaccagccctatgccccaccacgcgacttcgcagcctatcgctccctgagagtgaagttcagcaggagcgcagacgcccccgcgtaccagcagggccagaaccagctctataacgagctcaatctaggacgaagagaggagtacgatgttttggacaagagacgtggccgggaccctgagatggggggaaagccgcagagaaggaagaaccctcaggaaggcctgtacaatgaactgcagaaagataagatggcggaggcctacagtgagattgggatgaaaggcgagcgccggaggggcaaggggcacgatggcctttaccagggtctcagtacagccaccaaggacacctacgacgcccttcacatgcaggccctgccccctcgctaa

SEQ ID NO: 64 - protein, 482 aa, synthetic construct
MKHLWFFLLLVAAPRWVLSDIQMTQTTSSLSASLGDRVTISCRASQDISKYLNWYQQKPDGTVKLLIYHTSRLHSGVPSRFSGKGKGTKYKLTISNLEQEDIATYFCQQGNTLPYTFGGGTKLEITGGGGSGGGGSGGGGSEVKLQESGPGLVAPSQSLSVTCTVSGVSLPDYGVSWIRQPPRKGLEWLGVIWGSETTYYNSALKSRLTIIKDNSKSQVFLKMNSLQTDDTAIYYCAKHYYYGGSYAMDYWGQGTSVTVSSIEVMYPPPYLDNEKSNGTIIHVKGKHLCPSPLFPGPSKPFWVLVVVGGVLACYSLLVTVAFIIFWVRSKRSRLLHSDYMNMTPRRPGPTRKHYQPYAPPRDFAAYRSLRVKFSRSADAPAYQQGQNQLYNELNLGRREEYDVLDKRRGRDPEMGGKPQRRKNPQEGLYNELQKDKMAEAYSEIGMKGERRRGKGHDGLYQGLSTATKDTYDALHMQALPPR

SEQ ID NO: 65 - DNA, 1449 bp, synthetic construct
  source 1..1449: mol_type = other DNA
atgaaacacctgtggttcttcctcctgctggtggcagctcccagatgggtcctgtccgacatccaaatgacgcagactacaagcagcttgtcagcctcactgggagatcgagtcaccattagctgcagagctagccaggatataagcaaatacctgaactggtatcagcagaaacccgatggcaccgtgaagctgctgatctatcacacatctcggctgcatagtggagttccttctcgatttaagggcaagggcaaggggacaaaatataagctgacaatctccaacttggaacaggaggatatagccacctatttctgccagcaagggaataccctcccgtatacatttggaggcggcactaagctggagattacgggtggaggcggttcaggcggaggtggcagcggcggtggcgggagtgaagtgaaactgcaggagtcaggcccaggccttgtcgcaccctcccaatccctgagtgtcacatgcacagtaagcggggtttccctccccgactacggtgtttcatggatcagacagcctccaaggaaaggacttgagtggctcggggtgatttggggtagcgaaaccacctactacaatagcgcgttgaagtccaggctcaccatcatcaaggataacagtaaatcccaggttttcctgaaaatgaatagcctgcagacagatgatactgccatatactactgcgccaaacactattactacggcggatcttatgcgatggactattggggtcaaggtacatctgtaaccgtgagttccatcgaagtgatgtaccctcctccttacctggacaacgagaagtccaacggcaccatcatccacgtgaagggcaagcacctgtgtccttctccactgttccccggacctagcaagcctttttgggtgctggtggtggttggtggagtcctggcttgctatagcttgctagtaacagtggcctttattattttctgggtgaggagtaagaggagcaggctcctgcacagtgactacatgaacatgactccccgccgccccgggcccacccgcaagcattaccagccctatgccccaccacgcgacttcgcagcctatcgctccctgagagtgaagttcagcaggagcgcagacgcccccgcgtaccagcagggccagaaccagctctataacgagctcaatctaggacgaagagaggagtacgatgttttggacaagagacgtggccgggaccctgagatggggggaaagccgcagagaaggaagaaccctcaggaaggcctgtacaatgaactgcagaaagataagatggcggaggcctacagtgagattgggatgaaaggcgagcgccggaggggcaaggggcacgatggcctttaccagggtctcagtacagccaccaaggacacctacgacgcccttcacatgcaggccctgccccctcgctaa

SEQ ID NO: 66 - protein, 482 aa, synthetic construct
MKHLWFFLLLVAAPRWVLSDIQMTQTTSSLSASLGDRVTISCRASQDISKYLNWYQQKPDGTVKLLIYHTSRLHSGVPSRFKGKGKGTKYKLTISNLEQEDIATYFCQQGNTLPYTFGGGTKLEITGGGGSGGGGSGGGGSEVKLQESGPGLVAPSQSLSVTCTVSGVSLPDYGVSWIRQPPRKGLEWLGVIWGSETTYYNSALKSRLTIIKDNSKSQVFLKMNSLQTDDTAIYYCAKHYYYGGSYAMDYWGQGTSVTVSSIEVMYPPPYLDNEKSNGTIIHVKGKHLCPSPLFPGPSKPFWVLVVVGGVLACYSLLVTVAFIIFWVRSKRSRLLHSDYMNMTPRRPGPTRKHYQPYAPPRDFAAYRSLRVKFSRSADAPAYQQGQNQLYNELNLGRREEYDVLDKRRGRDPEMGGKPQRRKNPQEGLYNELQKDKMAEAYSEIGMKGERRRGKGHDGLYQGLSTATKDTYDALHMQALPPR

SEQ ID NO: 67 - DNA, 1449 bp, synthetic construct
  source 1..1449: mol_type = other DNA
atgaaacacctgtggttcttcctcctgctggtggcagctcccagatgggtcctgtccgacatccaaatgacgcagactacaagcagcttgtcagcctcactgggagatcgagtcaccattagctgcagagctagccaggatataagcaaatacctgaactggtatcagcagaaacccgatggcaccgtgaagctgctgatctatcacacatctcggctgcatagtggagttccttctcgatttagaggcaggggcagagggacaagatataggctgacaatctccaacttggaacaggaggatatagccacctatttctgccagcaagggaataccctcccgtatacatttggaggcggcactaagctggagattacgggtggaggcggttcaggcggaggtggcagcggcggtggcgggagtgaagtgaaactgcaggagtcaggcccaggccttgtcgcaccctcccaatccctgagtgtcacatgcacagtaagcggggtttccctccccgactacggtgtttcatggatcagacagcctccaaggaaaggacttgagtggctcggggtgatttggggtagcgaaaccacctactacaatagcgcgttgaagtccaggctcaccatcatcaaggataacagtaaatcccaggttttcctgaaaatgaatagcctgcagacagatgatactgccatatactactgcgccaaacactattactacggcggatcttatgcgatggactattggggtcaaggtacatctgtaaccgtgagttccatcgaagtgatgtaccctcctccttacctggacaacgagaagtccaacggcaccatcatccacgtgaagggcaagcacctgtgtccttctccactgttccccggacctagcaagcctttttgggtgctggtggtggttggtggagtcctggcttgctatagcttgctagtaacagtggcctttattattttctgggtgaggagtaagaggagcaggctcctgcacagtgactacatgaacatgactccccgccgccccgggcccacccgcaagcattaccagccctatgccccaccacgcgacttcgcagcctatcgctccctgagagtgaagttcagcaggagcgcagacgcccccgcgtaccagcagggccagaaccagctctataacgagctcaatctaggacgaagagaggagtacgatgttttggacaagagacgtggccgggaccctgagatggggggaaagccgcagagaaggaagaaccctcaggaaggcctgtacaatgaactgcagaaagataagatggcggaggcctacagtgagattgggatgaaaggcgagcgccggaggggcaaggggcacgatggcctttaccagggtctcagtacagccaccaaggacacctacgacgcccttcacatgcaggccctgccccctcgctaa

SEQ ID NO: 68 - protein, 482 aa, synthetic construct
MKHLWFFLLLVAAPRWVLSDIQMTQTTSSLSASLGDRVTISCRASQDISKYLNWYQQKPDGTVKLLIYHTSRLHSGVPSRFRGRGRGTRYRLTISNLEQEDIATYFCQQGNTLPYTFGGGTKLEITGGGGSGGGGSGGGGSEVKLQESGPGLVAPSQSLSVTCTVSGVSLPDYGVSWIRQPPRKGLEWLGVIWGSETTYYNSALKSRLTIIKDNSKSQVFLKMNSLQTDDTAIYYCAKHYYYGGSYAMDYWGQGTSVTVSSIEVMYPPPYLDNEKSNGTIIHVKGKHLCPSPLFPGPSKPFWVLVVVGGVLACYSLLVTVAFIIFWVRSKRSRLLHSDYMNMTPRRPGPTRKHYQPYAPPRDFAAYRSLRVKFSRSADAPAYQQGQNQLYNELNLGRREEYDVLDKRRGRDPEMGGKPQRRKNPQEGLYNELQKDKMAEAYSEIGMKGERRRGKGHDGLYQGLSTATKDTYDALHMQALPPR

SEQ ID NO: 69 - DNA, 1449 bp, synthetic construct
  source 1..1449: mol_type = other DNA
atgaaacacctgtggttcttcctcctgctggtggcagctcccagatgggtcctgtccgacatccaaatgacgcagactacaagcagcttgtcagcctcactgggagatcgagtcaccattagctgcagagctagccaggatataagcaaatacctgaactggtatcagcagaaacccgatggcaccgtgaagctgctgatctatcacacatctcggctgcatagtggagttccttctcgattttcaggctctggctctgggacaagatatagactgagaatctccaacttggaacaggaggatatagccacctatttctgccagcaagggaataccctcccgtatacatttggaggcggcactaagctggagattacgggtggaggcggttcaggcggaggtggcagcggcggtggcgggagtgaagtgaaactgcaggagtcaggcccaggccttgtcgcaccctcccaatccctgagtgtcacatgcacagtaagcggggtttccctccccgactacggtgtttcatggatcagacagcctccaaggaaaggacttgagtggctcggggtgatttggggtagcgaaaccacctactacaatagcgcgttgaagtccaggctcaccatcatcaaggataacagtaaatcccaggttttcctgaaaatgaatagcctgcagacagatgatactgccatatactactgcgccaaacactattactacggcggatcttatgcgatggactattggggtcaaggtacatctgtaaccgtgagttccatcgaagtgatgtaccctcctccttacctggacaacgagaagtccaacggcaccatcatccacgtgaagggcaagcacctgtgtccttctccactgttccccggacctagcaagcctttttgggtgctggtggtggttggtggagtcctggcttgctatagcttgctagtaacagtggcctttattattttctgggtgaggagtaagaggagcaggctcctgcacagtgactacatgaacatgactccccgccgccccgggcccacccgcaagcattaccagccctatgccccaccacgcgacttcgcagcctatcgctccctgagagtgaagttcagcaggagcgcagacgcccccgcgtaccagcagggccagaaccagctctataacgagctcaatctaggacgaagagaggagtacgatgttttggacaagagacgtggccgggaccctgagatggggggaaagccgcagagaaggaagaaccctcaggaaggcctgtacaatgaactgcagaaagataagatggcggaggcctacagtgagattgggatgaaaggcgagcgccggaggggcaaggggcacgatggcctttaccagggtctcagtacagccaccaaggacacctacgacgcccttcacatgcaggccctgccccctcgctaa

SEQ ID NO: 70 - protein, 482 aa, synthetic construct
MKHLWFFLLLVAAPRWVLSDIQMTQTTSSLSASLGDRVTISCRASQDISKYLNWYQQKPDGTVKLLIYHTSRLHSGVPSRFSGSGSGTRYRLRISNLEQEDIATYFCQQGNTLPYTFGGGTKLEITGGGGSGGGGSGGGGSEVKLQESGPGLVAPSQSLSVTCTVSGVSLPDYGVSWIRQPPRKGLEWLGVIWGSETTYYNSALKSRLTIIKDNSKSQVFLKMNSLQTDDTAIYYCAKHYYYGGSYAMDYWGQGTSVTVSSIEVMYPPPYLDNEKSNGTIIHVKGKHLCPSPLFPGPSKPFWVLVVVGGVLACYSLLVTVAFIIFWVRSKRSRLLHSDYMNMTPRRPGPTRKHYQPYAPPRDFAAYRSLRVKFSRSADAPAYQQGQNQLYNELNLGRREEYDVLDKRRGRDPEMGGKPQRRKNPQEGLYNELQKDKMAEAYSEIGMKGERRRGKGHDGLYQGLSTATKDTYDALHMQALPPR

SEQ ID NO: 71 - DNA, 1449 bp, synthetic construct
  source 1..1449: mol_type = other DNA
atgaaacacctgtggttcttcctcctgctggtggcagctcccagatgggtcctgtccgacatccaaatgacgcagactacaagcagcttgtcagcctcactgggagatcgagtcaccattagctgcagagctagccaggatataagcaaatacctgaactggtatcagcagaaacccgatggcaccgtgaagctgctgatctatcacacatctcggctgcatagtggagttcctagacgatttagaggctctggctctgggacagattatagtctgacaatcaggaacttggaacaggaggatatagccacctatttctgccagcaagggaataccctcccgtatacatttggaggcggcactaagctggagattacgggtggaggcggttcaggcggaggtggcagcggcggtggcgggagtgaagtgaaactgcaggagtcaggcccaggccttgtcgcaccctcccaatccctgagtgtcacatgcacagtaagcggggtttccctccccgactacggtgtttcatggatcagacagcctccaaggaaaggacttgagtggctcggggtgatttggggtagcgaaaccacctactacaatagcgcgttgaagtccaggctcaccatcatcaaggataacagtaaatcccaggttttcctgaaaatgaatagcctgcagacagatgatactgccatatactactgcgccaaacactattactacggcggatcttatgcgatggactattggggtcaaggtacatctgtaaccgtgagttccatcgaagtgatgtaccctcctccttacctggacaacgagaagtccaacggcaccatcatccacgtgaagggcaagcacctgtgtccttctccactgttccccggacctagcaagcctttttgggtgctggtggtggttggtggagtcctggcttgctatagcttgctagtaacagtggcctttattattttctgggtgaggagtaagaggagcaggctcctgcacagtgactacatgaacatgactccccgccgccccgggcccacccgcaagcattaccagccctatgccccaccacgcgacttcgcagcctatcgctccctgagagtgaagttcagcaggagcgcagacgcccccgcgtaccagcagggccagaaccagctctataacgagctcaatctaggacgaagagaggagtacgatgttttggacaagagacgtggccgggaccctgagatggggggaaagccgcagagaaggaagaaccctcaggaaggcctgtacaatgaactgcagaaagataagatggcggaggcctacagtgagattgggatgaaaggcgagcgccggaggggcaaggggcacgatggcctttaccagggtctcagtacagccaccaaggacacctacgacgcccttcacatgcaggccctgccccctcgctaa

SEQ ID NO: 72 - protein, 482 aa, synthetic construct
MKHLWFFLLLVAAPRWVLSDIQMTQTTSSLSASLGDRVTISCRASQDISKYLNWYQQKPDGTVKLLIYHTSRLHSGVPRRFRGSGSGTDYSLTIRNLEQEDIATYFCQQGNTLPYTFGGGTKLEITGGGGSGGGGSGGGGSEVKLQESGPGLVAPSQSLSVTCTVSGVSLPDYGVSWIRQPPRKGLEWLGVIWGSETTYYNSALKSRLTIIKDNSKSQVFLKMNSLQTDDTAIYYCAKHYYYGGSYAMDYWGQGTSVTVSSIEVMYPPPYLDNEKSNGTIIHVKGKHLCPSPLFPGPSKPFWVLVVVGGVLACYSLLVTVAFIIFWVRSKRSRLLHSDYMNMTPRRPGPTRKHYQPYAPPRDFAAYRSLRVKFSRSADAPAYQQGQNQLYNELNLGRREEYDVLDKRRGRDPEMGGKPQRRKNPQEGLYNELQKDKMAEAYSEIGMKGERRRGKGHDGLYQGLSTATKDTYDALHMQALPPR

SEQ ID NO: 73 - DNA, 1449 bp, synthetic construct
  source 1..1449: mol_type = other DNA
atgaaacacctgtggttcttcctcctgctggtggcagctcccagatgggtcctgtccgacatccaaatgacgcagactacaagcagcttgtcagcctcactgggagatcgagtcaccattagctgcagagctagccaggatataagcaaatacctgaactggtatcagcagaaacccgatggcaccgtgaagctgctgatctatcacacatctcggctgcatagtggagttcctagacgattttcaggctctggctctgggacagattatagtctgagaatcaggaacttggaacaggaggatatagccacctatttctgccagcaagggaataccctcccgtatacatttggaggcggcactaagctggagattacgggtggaggcggttcaggcggaggtggcagcggcggtggcgggagtgaagtgaaactgcaggagtcaggcccaggccttgtcgcaccctcccaatccctgagtgtcacatgcacagtaagcggggtttccctccccgactacggtgtttcatggatcagacagcctccaaggaaaggacttgagtggctcggggtgatttggggtagcgaaaccacctactacaatagcgcgttgaagtccaggctcaccatcatcaaggataacagtaaatcccaggttttcctgaaaatgaatagcctgcagacagatgatactgccatatactactgcgccaaacactattactacggcggatcttatgcgatggactattggggtcaaggtacatctgtaaccgtgagttccatcgaagtgatgtaccctcctccttacctggacaacgagaagtccaacggcaccatcatccacgtgaagggcaagcacctgtgtccttctccactgttccccggacctagcaagcctttttgggtgctggtggtggttggtggagtcctggcttgctatagcttgctagtaacagtggcctttattattttctgggtgaggagtaagaggagcaggctcctgcacagtgactacatgaacatgactccccgccgccccgggcccacccgcaagcattaccagccctatgccccaccacgcgacttcgcagcctatcgctccctgagagtgaagttcagcaggagcgcagacgcccccgcgtaccagcagggccagaaccagctctataacgagctcaatctaggacgaagagaggagtacgatgttttggacaagagacgtggccgggaccctgagatggggggaaagccgcagagaaggaagaaccctcaggaaggcctgtacaatgaactgcagaaagataagatggcggaggcctacagtgagattgggatgaaaggcgagcgccggaggggcaaggggcacgatggcctttaccagggtctcagtacagccaccaaggacacctacgacgcccttcacatgcaggccctgccccctcgctaa

SEQ ID NO: 74 - protein, 482 aa, synthetic construct
MKHLWFFLLLVAAPRWVLSDIQMTQTTSSLSASLGDRVTISCRASQDISKYLNWYQQKPDGTVKLLIYHTSRLHSGVPRRFSGSGSGTDYSLRIRNLEQEDIATYFCQQGNTLPYTFGGGTKLEITGGGGSGGGGSGGGGSEVKLQESGPGLVAPSQSLSVTCTVSGVSLPDYGVSWIRQPPRKGLEWLGVIWGSETTYYNSALKSRLTIIKDNSKSQVFLKMNSLQTDDTAIYYCAKHYYYGGSYAMDYWGQGTSVTVSSIEVMYPPPYLDNEKSNGTIIHVKGKHLCPSPLFPGPSKPFWVLVVVGGVLACYSLLVTVAFIIFWVRSKRSRLLHSDYMNMTPRRPGPTRKHYQPYAPPRDFAAYRSLRVKFSRSADAPAYQQGQNQLYNELNLGRREEYDVLDKRRGRDPEMGGKPQRRKNPQEGLYNELQKDKMAEAYSEIGMKGERRRGKGHDGLYQGLSTATKDTYDALHMQALPPR

SEQ ID NO: 75 - DNA, 1449 bp, synthetic construct
  source 1..1449: mol_type = other DNA
atgaaacacctgtggttcttcctcctgctggtggcagctcccagatgggtcctgtccgacatccaaatgacgcagactacaagcagcttgtcagcctcactgggagatcgagtcaccattagctgcagagctagccaggatataagcaaatacctgaactggtatcagcagaaacccgatggcaccgtgaagctgctgatctatcacacatctcggctgcatagtggagttccttctcgattttcaggctctggctctgggacagattatagtctgacaatctccagattgagacagagagatatagccacctatttctgccagcaagggaataccctcccgtatacatttggaggcggcactaagctggagattacgggtggaggcggttcaggcggaggtggcagcggcggtggcgggagtgaagtgaaactgcaggagtcaggcccaggccttgtcgcaccctcccaatccctgagtgtcacatgcacagtaagcggggtttccctccccgactacggtgtttcatggatcagacagcctccaaggaaaggacttgagtggctcggggtgatttggggtagcgaaaccacctactacaatagcgcgttgaagtccaggctcaccatcatcaaggataacagtaaatcccaggttttcctgaaaatgaatagcctgcagacagatgatactgccatatactactgcgccaaacactattactacggcggatcttatgcgatggactattggggtcaaggtacatctgtaaccgtgagttccatcgaagtgatgtaccctcctccttacctggacaacgagaagtccaacggcaccatcatccacgtgaagggcaagcacctgtgtccttctccactgttccccggacctagcaagcctttttgggtgctggtggtggttggtggagtcctggcttgctatagcttgctagtaacagtggcctttattattttctgggtgaggagtaagaggagcaggctcctgcacagtgactacatgaacatgactccccgccgccccgggcccacccgcaagcattaccagccctatgccccaccacgcgacttcgcagcctatcgctccctgagagtgaagttcagcaggagcgcagacgcccccgcgtaccagcagggccagaaccagctctataacgagctcaatctaggacgaagagaggagtacgatgttttggacaagagacgtggccgggaccctgagatggggggaaagccgcagagaaggaagaaccctcaggaaggcctgtacaatgaactgcagaaagataagatggcggaggcctacagtgagattgggatgaaaggcgagcgccggaggggcaaggggcacgatggcctttaccagggtctcagtacagccaccaaggacacctacgacgcccttcacatgcaggccctgccccctcgctaa

SEQ ID NO: 76 - protein, 482 aa, synthetic construct
MKHLWFFLLLVAAPRWVLSDIQMTQTTSSLSASLGDRVTISCRASQDISKYLNWYQQKPDGTVKLLIYHTSRLHSGVPSRFSGSGSGTDYSLTISRLRQRDIATYFCQQGNTLPYTFGGGTKLEITGGGGSGGGGSGGGGSEVKLQESGPGLVAPSQSLSVTCTVSGVSLPDYGVSWIRQPPRKGLEWLGVIWGSETTYYNSALKSRLTIIKDNSKSQVFLKMNSLQTDDTAIYYCAKHYYYGGSYAMDYWGQGTSVTVSSIEVMYPPPYLDNEKSNGTIIHVKGKHLCPSPLFPGPSKPFWVLVVVGGVLACYSLLVTVAFIIFWVRSKRSRLLHSDYMNMTPRRPGPTRKHYQPYAPPRDFAAYRSLRVKFSRSADAPAYQQGQNQLYNELNLGRREEYDVLDKRRGRDPEMGGKPQRRKNPQEGLYNELQKDKMAEAYSEIGMKGERRRGKGHDGLYQGLSTATKDTYDALHMQALPPR

SEQ ID NO: 77 - DNA, 24 bp, synthetic construct
  source 1..24: mol_type = other DNA
aaatcgaattcccaaacttaagct

SEQ ID NO: 78 - DNA, 25 bp, synthetic construct
  source 1..25: mol_type = other DNA
ttcattcccccctttttctggagac

SEQ ID NO: 79 - DNA, 42 bp, synthetic construct
  source 1..42: mol_type = other DNA
cgattccgaggccgaaaccgagggaaccgagccactctgacc

SEQ ID NO: 80 - DNA, 42 bp, synthetic construct
  source 1..42: mol_type = other DNA
agtggctcggttccctcggtttcggcctcggaatcgctcagg

SEQ ID NO: 81 - DNA, 42 bp, synthetic construct
  source 1..42: mol_type = other DNA
cgattccgaggccgaaaccgagggaacacagcccgactgacc

SEQ ID NO: 82 - DNA, 42 bp, synthetic construct
  source 1..42: mol_type = other DNA
ggtcagtcgggctgtgttccctcggtttcggcctcggaatcg

SEQ ID NO: 83 - DNA, 31 bp, synthetic construct
  source 1..31: mol_type = other DNA
aacacagccaggctgaccatcagcgggaccc

SEQ ID NO: 84 - DNA, 31 bp, synthetic construct
  source 1..31: mol_type = other DNA
cccagagttcctgcctctgaatcgctcaggg

SEQ ID NO: 85 - DNA, 31 bp, synthetic construct
  source 1..31: mol_type = other DNA
aacaaagccactctgaccatcagcgggaccc

SEQ ID NO: 86 - DNA, 31 bp, synthetic construct
  source 1..31: mol_type = other DNA
ccccttgttggagcccttgaatcgctcaggg

SEQ ID NO: 87 - DNA, 31 bp, synthetic construct
  source 1..31: mol_type = other DNA
aacagagccaggctgaccatcagcgggaccc

SEQ ID NO: 88 - DNA, 31 bp, synthetic construct
  source 1..31: mol_type = other DNA
cccagagttggagcctctgaatcgctcaggg

SEQ ID NO: 89 - DNA, 31 bp, synthetic construct; identical to SEQ ID NO: 85
  source 1..31: mol_type = other DNA

SEQ ID NO: 90 - DNA, 31 bp, synthetic construct
  source 1..31: mol_type = other DNA
ccccttgttcttgccagagaatcgctcaggg

SEQ ID NO: 91 - DNA, 31 bp, synthetic construct; identical to SEQ ID NO: 87
  source 1..31: mol_type = other DNA

SEQ ID NO: 92 - DNA, 31 bp, synthetic construct
  source 1..31: mol_type = other DNA
cccagagttcctgccagagaatcgctcaggg

SEQ ID NO: 93 - DNA, 31 bp, synthetic construct; identical to SEQ ID NO: 87
  source 1..31: mol_type = other DNA

SEQ ID NO: 94 - DNA, 31 bp, synthetic construct
  source 1..31: mol_type = other DNA
ccctctgttggagccagagaatcgctcaggg

SEQ ID NO: 95 - DNA, 31 bp, synthetic construct
  source 1..31: mol_type = other DNA
aacaaagccaagctgaccatcagcgggaccc

SEQ ID NO: 96 - DNA, 31 bp, synthetic construct
  source 1..31: mol_type = other DNA
ccccttgttcttgcccttgaatcgctcaggg

SEQ ID NO: 97 - DNA, 19 bp, synthetic construct
  source 1..19: mol_type = other DNA
acccaggctatggatgagg

SEQ ID NO: 98 - DNA, 30 bp, synthetic construct
  source 1..30: mol_type = other DNA
ccccctgatcctcagagtggctgtgttccc

SEQ ID NO: 99 - DNA, 30 bp, synthetic construct
  source 1..30: mol_type = other DNA
tccctaggcgattctctggctccaactctg

SEQ ID NO: 100 - DNA, 22 bp, synthetic construct
  source 1..22: mol_type = other DNA
tccctgagggccggtcgctatc

SEQ ID NO: 101 - DNA, 49 bp, synthetic construct
  source 1..49: mol_type = other DNA
aataatgcggccgccctgcaggaccaccatgaaacacctgtggttcttc

SEQ ID NO: 102 - DNA, 43 bp, synthetic construct
  source 1..43: mol_type = other DNA
aaaaaagcggccgcaaatcgatttacacccacaggtctcccag

SEQ ID NO: 103 - DNA, 47 bp, synthetic construct
  source 1..47: mol_type = other DNA
cctgagcgattccgaggccgaaactcggggaacacggcccgactgac

SEQ ID NO: 104 - DNA, 46 bp, synthetic construct
  source 1..46: mol_type = other DNA
gatggtcagtcgggccgtgttccccgagtttcggcctcggaatcgc

SEQ ID NO: 105 - DNA, 46 bp, synthetic construct
  source 1..46: mol_type = other DNA
gcgattccgaggctccaactcggggaaccgagcccgactgaccatc

SEQ ID NO: 106 - DNA, 46 bp, synthetic construct
  source 1..46: mol_type = other DNA
gatggtcagtcgggctcggttccccgagttggagcctcggaatcgc

SEQ ID NO: 107 - DNA, 31 bp, synthetic construct
  source 1..31: mol_type = other DNA
gggaacaaggccaagctgaccatcagcagag

SEQ ID NO: 108 - DNA, 31 bp, synthetic construct
  source 1..31: mol_type = other DNA
cgagttcttgccagagaatcgctcagggatc

SEQ ID NO: 109 - DNA, 38 bp, synthetic construct
  source 1..38: mol_type = other DNA
agatgggtcctgtccgacatccaaatgacgcagactac

SEQ ID NO: 110 - DNA, 33 bp, synthetic construct
  source 1..33: mol_type = other DNA
acttcgatggaactcacggttacagatgtacct

SEQ ID NO: 111 - DNA, 321 bp, synthetic construct
  source 1..321: mol_type = other DNA
atcgaagtgatgtaccctcctccttacctggacaacgagaagtccaacggcaccatcatccacgtgaagggcaagcacctgtgtccttctccactgttccccggacctagcaagcctttctgggtgctcgttgttgttggcggcgtgctggcctgttacagcctgctggttaccgtggccttcatcatcttttgggtccgaagcaagcggagccggctgctgcacagcgactacatgaacatgacccctagacggcccggaccaaccagaaagcactaccagccttacgctcctcctagagacttcgccgcctacagatct

SEQ ID NO: 112 - DNA, 30 bp, synthetic construct
  source 1..30: mol_type = other DNA
gagttccatcgaagtgatgtaccctcctcc

SEQ ID NO: 113 - DNA, 39 bp, synthetic construct
  source 1..39: mol_type = other DNA
cttacgacctcttttgacccaaaagatgatgaaggccac

SEQ ID NO: 114 - DNA, 1704 bp, synthetic construct
  source 1..1704: mol_type = other DNA
gcggccgccaccatgaaacacctgtggttcttcctcctgctggtggcagctcccagatgggtcctgtcccaggtgcagctgcaggtccagctggtacagtctggggctgaggtgaagaagcctgggtcctcggtgaaggtctcctgcaaggcttctggaggcaccttcagcagctatgctatcagctgggtgcgacaggcccctggacaagggcttgagtggatgggagggatcatccctatctttggtacagcaaactacgcacagaagttccagggcagagtcacgattaccgcggacaaatccacgagcacagcctacatggagctgagcagcctgagatctgaggacacggccgtgtattactgtgcgagatccccccggcgggcatatcatgatgcttttgatatctggggccaagggacaatggtcaccgtctcttcaggtggaggcggttcaggcggaggtggcagcggcggtggcgggagttcctatgagctgactcagccaccctcgatgtcagtggccccaggaaagacggccagcattacctgtggcggagaccatattggaagtaaaagtgttcactggtaccagcagaagccaggccaggcccctgtactggtcgtctatgatgatagcgaccggccctcagggatccctgagcgattctctggctccaactctgggaacacagccactctgaccatcagcgggacccaggctatggatgaggctgactattactgtctggcgtgggacagcagcactgcgatcttcggcggaggcacccagctgaccgtcctcgtgggtcagcccaaggccaaccccactgtcactctgtttccgccctcctctgaggagctccaagccaacaaggccacactagtgtgtctgatcagtgacttctacccgggagctgtgacagtggcctggaaggcagatggcagccccgtcaaggcgggagtggagaccaccaaaccctccaaacagagcaacaacaagtacgcggccagcagctacctgagcctgacgcccgagcagtggaagtcccacagaagctacagctgccaggtcacgcatgaagggagcaccgtggagaagactgtggcccctacagaatgttcggcgcgccagactagattttgggtgctggtggtggttggtggagtcctggcttgctatagcttgctagtaacagtggcctttattattttctgggtgaggagtaagaggagcaggctcctgcacagtgactacatgaacatgactccccgccgccccgggcccacccgcaagcattaccagccctatgccccaccacgcgacttcgcagcctatcgctccctgagagtgaagttcagcaggagcgcagacgcccccgcgtaccagcagggccagaaccagctctataacgagctcaatctaggacgaagagaggagtacgatgttttggacaagagacgtggccgggaccctgagatggggggaaagccgcagagaaggaagaaccctcaggaaggcctgtacaatgaactgcagaaagataagatggcggaggcctacagtgagattgggatgaaaggcgagcgccggaggggcaaggggcacgatggcctttaccagggtctcagtacagccaccaaggacacctacgacgcccttcacatgcaggccctgccccctcgctaatcgattctcgag

SEQ ID NO: 115 - DNA, 22 bp, synthetic construct
  source 1..22: mol_type = other DNA
ttttgggtgctggtggtggttg

SEQ ID NO: 116 - DNA, 20 bp, synthetic construct
  source 1..20: mol_type = other DNA
ggacaggacccatctgggag

SEQ ID NO: 117 - DNA, 34 bp, synthetic construct
  source 1..34: mol_type = other DNA
gggacaagatataggctgacaatctccaacttgg

SEQ ID NO: 118 - DNA, 35 bp, synthetic construct
  source 1..35: mol_type = other DNA
agagcccctgcctctaaatcgagaaggaactccac

SEQ ID NO: 119 - DNA, 26 bp, synthetic construct
  source 1..26: mol_type = other DNA
ggcagaggctctgggacagattatag

SEQ ID NO: 120 - DNA, 31 bp, synthetic construct
  source 1..31: mol_type = other DNA
tctaaatcgtctaggaactccactatgcagc

SEQ ID NO: 121 - DNA, 34 bp, synthetic construct
  source 1..34: mol_type = other DNA
gggacaaaatatagtctgacaatctccaacttgg

SEQ ID NO: 122 - DNA, 35 bp, synthetic construct
  source 1..35: mol_type = other DNA
agagcccttgcccttaaatcgagaaggaactccac

SEQ ID NO: 123 - DNA, 34 bp, synthetic construct
  source 1..34: mol_type = other DNA
gggacagattataggctgacaatctccaacttgg

SEQ ID NO: 124 - DNA, 35 bp, synthetic construct; identical to SEQ ID NO: 118
  source 1..35: mol_type = other DNA

SEQ ID NO: 125 - DNA, 34 bp, synthetic construct
  source 1..34: mol_type = other DNA
gggacaagatatagtctgacaatctccaacttgg

SEQ ID NO: 126 - DNA, 35 bp, synthetic construct
  source 1..35: mol_type = other DNA
tctgccagagcctctaaatcgagaaggaactccac

SEQ ID NO: 127 - DNA, 34 bp, synthetic construct; identical to SEQ ID NO: 117
  source 1..34: mol_type = other DNA

SEQ ID NO: 128 - DNA, 35 bp, synthetic construct
  source 1..35: mol_type = other DNA
agagccagagcctctaaatcgagaaggaactccac

SEQ ID NO: 129 - DNA, 34 bp, synthetic construct; identical to SEQ ID NO: 125
  source 1..34: mol_type = other DNA

SEQ ID NO: 130 - DNA, 35 bp, synthetic construct
  source 1..35: mol_type = other DNA
tctgcccctgcctgaaaatcgagaaggaactccac

SEQ ID NO: 131 - DNA, 34 bp, synthetic construct; identical to SEQ ID NO: 123
  source 1..34: mol_type = other DNA

SEQ ID NO: 132 - DNA, 35 bp, synthetic construct; identical to SEQ ID NO: 130
  source 1..35: mol_type = other DNA

SEQ ID NO: 133 - DNA, 34 bp, synthetic construct
  source 1..34: mol_type = other DNA
gggacaaaatataagctgacaatctccaacttgg

SEQ ID NO: 134 - DNA, 35 bp, synthetic construct; identical to SEQ ID NO: 122
  source 1..35: mol_type = other DNA

SEQ ID NO: 135 - DNA, 34 bp, synthetic construct; identical to SEQ ID NO: 133
  source 1..34: mol_type = other DNA

SEQ ID NO: 136 - DNA, 35 bp, synthetic construct
  source 1..35: mol_type = other DNA
cttgcccttgcctgaaaatcgagaaggaactccac

SEQ ID NO: 137 - DNA, 34 bp, synthetic construct; identical to SEQ ID NO: 133
  source 1..34: mol_type = other DNA

SEQ ID NO: 138 - DNA, 35 bp, synthetic construct
  source 1..35: mol_type = other DNA
cttgcccttgcccttaaatcgagaaggaactccac

SEQ ID NO: 139 - DNA, 34 bp, synthetic construct; identical to SEQ ID NO: 117
  source 1..34: mol_type = other DNA

SEQ ID NO: 140 - DNA, 35 bp, synthetic construct
  source 1..35: mol_type = other DNA
tctgcccctgcctctaaatcgagaaggaactccac

SEQ ID NO: 141 - DNA, 24 bp, synthetic construct
  source 1..24: mol_type = other DNA
agaatctccaacttggaacaggag

SEQ ID NO: 142 - DNA, 29 bp, synthetic construct
  source 1..29: mol_type = other DNA
cagtctatatcttgtcccagagccagagc

SEQ ID NO: 143 - DNA, 17 bp, synthetic construct
  source 1..17: mol_type = other DNA
ggctctggctctgggac

SEQ ID NO: 144 - DNA, 31 bp, synthetic construct; identical to SEQ ID NO: 120
  source 1..31: mol_type = other DNA

SEQ ID NO: 145 - DNA, 32 bp, synthetic construct
  source 1..32: mol_type = other DNA
acaatcaggaacttggaacaggaggatatagc

SEQ ID NO: 146 - DNA, 29 bp, synthetic construct
  source 1..29: mol_type = other DNA
cagactataatctgtcccagagccagagc

SEQ ID NO: 147 - DNA, 31 bp, synthetic construct
  source 1..31: mol_type = other DNA
agaatcaggaacttggaacaggaggatatag

SEQ ID NO: 148 - DNA, 29 bp, synthetic construct
  source 1..29: mol_type = other DNA
cagactataatctgtcccagagccagagc

SEQ ID NO: 149 - DNA, 17 bp, synthetic construct
  source 1..17: mol_type = other DNA
ggctctggctctgggac

SEQ ID NO: 150 - DNA, 31 bp, synthetic construct
  source 1..31: mol_type = other DNA
tgaaaatcgtctaggaactccactatgcagc

SEQ ID NO: 151 - DNA, 34 bp, synthetic construct
  source 1..34: mol_type = other DNA
ttgagacagagagatatagccacctatttctgcc

SEQ ID NO: 152 - DNA, 29 bp, synthetic construct
  source 1..29: mol_type = other DNA
tctggagattgtcagactataatctgtcc

SEQ ID NO: 153 - DNA, 15 bp, synthetic construct
  source 1..15: mol_type = other DNA
agctatgctatcagc

SEQ ID NO: 154 - DNA, 51 bp, synthetic construct
  source 1..51: mol_type = other DNA
gggatcatccctatctttggtacagcaaactacgcacagaagttccagggc

SEQ ID NO: 155 - DNA, 36 bp, synthetic construct
  source 1..36: mol_type = other DNA
tccccccggcgggcatatcatgatgcttttgatatc

SEQ ID NO: 156 - DNA, 33 bp, synthetic construct
  source 1..33: mol_type = other DNA
ggcggagaccatattggaagtaaaagtgttcac

SEQ ID NO: 157 - DNA, 21 bp, synthetic construct
  source 1..21: mol_type = other DNA
gatgatagcgaccggccctca

SEQ ID NO: 158 - DNA, 27 bp, synthetic construct
  source 1..27: mol_type = other DNA
ctggcgtgggacagcagcactgcgatc

SEQ ID NO: 159 - DNA, 729 bp, synthetic construct
  source 1..729: mol_type = other DNA
caggtccagctggtacagtctggggctgaggtgaagaagcctgggtcctcggtgaaggtctcctgcaaggcttctggaggcaccttcagcagctatgctatcagctgggtgcgacaggcccctggacaagggcttgagtggatgggagggatcatccctatctttggtacagcaaactacgcacagaagttccagggcagagtcacgattaccgcggacaaatccacgagcacagcctacatggagctgagcagcctgagatctgaggacacggccgtgtattactgtgcgagatccccccggcgggcatatcatgatgcttttgatatctggggccaagggacaatggtcaccgtctcttcaggtggaggcggttcaggcggaggtggcagcggcggtggcgggagttcctatgagctgactcagccaccctcgatgtcagtggccccaggaaagacggccagcattacctgtggcggagaccatattggaagtaaaagtgttcactggtaccagcagaagccaggccaggcccctgtactggtcgtctatgatgatagcgaccggccctcagggatccctgagcgattctctggctccaactctgggaacacagccactctgaccatcagcgggacccaggctatggatgaggctgactattactgtctggcgtgggacagcagcactgcgatcttcggcggaggcacccagctgaccgtcctcgtg

SEQ ID NO: 160 - DNA, 729 bp, synthetic construct
  source 1..729: mol_type = other DNA
caggtccagctggtacagtctggggctgaggtgaagaagcctgggtcctcggtgaaggtctcctgcaaggcttctggaggcaccttcagcagctatgctatcagctgggtgcgacaggcccctggacaagggcttgagtggatgggagggatcatccctatctttggtacagcaaactacgcacagaagttccagggcagagtcacgattaccgcggacaaatccacgagcacagcctacatggagctgagcagcctgagatctgaggacacggccgtgtattactgtgcgagatccccccggcgggcatatcatgatgcttttgatatctggggccaagggacaatggtcaccgtctcttcaggtggaggcggttcaggcggaggtggcagcggcggtggcgggagttcctatgagctgactcagccaccctcgatgtcagtggccccaggaaagacggccagcattacctgtggcggagaccatattggaagtaaaagtgttcactggtaccagcagaagccaggccaggcccctgtactggtcgtctatgatgatagcgaccggccctcagggatccctgagcgattccgaggccgaaaccgagggaaccgagccactctgaccatcagcgggacccaggctatggatgaggctgactattactgtctggcgtgggacagcagcactgcgatcttcggcggaggcacccagctgaccgtcctcgtg

SEQ ID NO: 161 - DNA, 729 bp, synthetic construct
  source 1..729: mol_type = other DNA
caggtccagctggtacagtctggggctgaggtgaagaagcctgggtcctcggtgaaggtctcctgcaaggcttctggaggcaccttcagcagctatgctatcagctgggtgcgacaggcccctggacaagggcttgagtggatgggagggatcatccctatctttggtacagcaaactacgcacagaagttccagggcagagtcacgattaccgcggacaaatccacgagcacagcctacatggagctgagcagcctgagatctgaggacacggccgtgtattactgtgcgagatccccccggcgggcatatcatgatgcttttgatatctggggccaagggacaatggtcaccgtctcttcaggtggaggcggttcaggcggaggtggcagcggcggtggcgggagttcctatgagctgactcagccaccctcgatgtcagtggccccaggaaagacggccagcattacctgtggcggagaccatattggaagtaaaagtgttcactggtaccagcagaagccaggccaggcccctgtactggtcgtctatgatgatagcgaccggccctcagggatccctgagcgattccgaggccgaaaccgagggaacacagcccgactgaccatcagcgggacccaggctatggatgaggctgactattactgtctggcgtgggacagcagcactgcgatcttcggcggaggcacccagctgaccgtcctcgtg

SEQ ID NO: 162 - DNA, 729 bp, synthetic construct
  source 1..729: mol_type = other DNA
caggtccagctggtacagtctggggctgaggtgaagaagcctgggtcctcggtgaaggtctcctgcaaggcttctggaggcaccttcagcagctatgctatcagctgggtgcgacaggcccctggacaagggcttgagtggatgggagggatcatccctatctttggtacagcaaactacgcacagaagttccagggcagagtcacgattaccgcggacaaatccacgagcacagcctacatggagctgagcagcctgagatctgaggacacggccgtgtattactgtgcgagatccccccggcgggcatatcatgatgcttttgatatctggggccaagggacaatggtcaccgtctcttcaggtggaggcggttcaggcggaggtggcagcggcggtggcgggagttcctatgagctgactcagccaccctcgatgtcagtggccccaggaaagacggccagcattacctgtggcggagaccatattggaagtaaaagtgttcactggtaccagcagaagccaggccaggcccctgtactggtcgtctatgatgatagcgaccggccctcagggatccctgagcgattcagaggcaggaactctgggaacacagccaggctgaccatcagcgggacccaggctatggatgaggctgactattactgtctggcgtgggacagcagcactgcgatcttcggcggaggcacccagctgaccgtcctcgtg

SEQ ID NO: 163 - DNA, 729 bp, synthetic construct
  source 1..729: mol_type = other DNA
caggtccagctggtacagtctggggctgaggtgaagaagcctgggtcctcggtgaaggtctcctgcaaggcttctggaggcaccttcagcagctatgctatcagctgggtgcgacaggcccctggacaagggcttgagtggatgggagggatcatccctatctttggtacagcaaactacgcacagaagttccagggcagagtcacgattaccgcggacaaatccacgagcacagcctacatggagctgagcagcctgagatctgaggacacggccgtgtattactgtgcgagatccccccggcgggcatatcatgatgcttttgatatctggggccaagggacaatggtcaccgtctcttcaggtggaggcggttcaggcggaggtggcagcggcggtggcgggagttcctatgagctgactcagccaccctcgatgtcagtggccccaggaaagacggccagcattacctgtggcggagaccatattggaagtaaaagtgttcactggtaccagcagaagccaggccaggcccctgtactggtcgtctatgatgatagcgaccggccctcagggatccctgagcgattcaagggctccaacaaggggaacaaagccactctgaccatcagcgggacccaggctatggatgaggctgactattactgtctggcgtgggacagcagcactgcgatcttcggcggaggcacccagctgaccgtcctcgtg

SEQ ID NO: 164 - DNA, 729 bp, synthetic construct
  source 1..729: mol_type = other DNA
caggtccagctggtacagtctggggctgaggtgaagaagcctgggtcctcggtgaaggtctcctgcaaggcttctggaggcaccttcagcagctatgctatcagctgggtgcgacaggcccctggacaagggcttgagtggatgggagggatcatccctatctttggtacagcaaactacgcacagaagttccagggcagagtcacgattaccgcggacaaatccacgagcacagcctacatggagctgagcagcctgagatctgaggacacggccgtgtattactgtgcgagatccccccggcgggcatatcatgatgcttttgatatctggggccaagggacaatggtcaccgtctcttcaggtggaggcggttcaggcggaggtggcagcggcggtggcgggagttcctatgagctgactcagccaccctcgatgtcagtggccccaggaaagacggccagcattacctgtggcggagaccatattggaagtaaaagtgttcactggtaccagcagaagccaggccaggcccctgtactggtcgtctatgatgatagcgaccggccctcagggatccctgagcgattcagaggctccaactctgggaacagagccaggctgaccatcagcgggacccaggctatggatgaggctgactattactgtctggcgtgggacagcagcactgcgatcttcggcggaggcacccagctgaccgtcctcgtg

SEQ ID NO: 165 - DNA, 729 bp, synthetic construct
  source 1..729: mol_type = other DNA
caggtccagctggtacagtctggggctgaggtgaagaagcctgggtcctcggtgaaggtctcctgcaaggcttctggaggcaccttcagcagctatgctatcagctgggtgcgacaggcccctggacaagggcttgagtggatgggagggatcatccctatctttggtacagcaaactacgcacagaagttccagggcagagtcacgattaccgcggacaaatccacgagcacagcctacatggagctgagcagcctgagatctgaggacacggccgtgtattactgtgcgagatccccccggcgggcatatcatgatgcttttgatatctggggccaagggacaatggtcaccgtctcttcaggtggaggcggttcaggcggaggtggcagcggcggtggcgggagttcctatgagctgactcagccaccctcgatgtcagtggccccaggaaagacggccagcattacctgtggcggagaccatattggaagtaaaagtgttcactggtaccagcagaagccaggccaggcccctgtactggtcgtctatgatgatagcgaccggccctcagggatccctgagcgattctctggcaagaacaaggggaacaaagccactctgaccatcagcgggacccaggctatggatgaggctgactattactgtctggcgtgggacagcagcactgcgatcttcggcggaggcacccagctgaccgtcctcgtg

SEQ ID NO: 166 - DNA, 729 bp, synthetic construct
  source 1..729: mol_type = other DNA
caggtccagctggtacagtctggggctgaggtgaagaagcctgggtcctcggtgaaggtctcctgcaaggcttctggaggcaccttcagcagctatgctatcagctgggtgcgacaggcccctggacaagggcttgagtggatgggagggatcatccctatctttggtacagcaaactacgcacagaagttccagggcagagtcacgattaccgcggacaaatccacgagcacagcctacatggagctgagcagcctgagatctgaggacacggccgtgtattactgtgcgagatccccccggcgggcatatcatgatgcttttgatatctggggccaagggacaatggtcaccgtctcttcaggtggaggcggttcaggcggaggtggcagcggcggtggcgggagttcctatgagctgactcagccaccctcgatgtcagtggccccaggaaagacggccagcattacctgtggcggagaccatattggaagtaaaagtgttcactggtaccagcagaagccaggccaggcccctgtactggtcgtctatgatgatagcgaccggccctcagggatccctgagcgattctctggcaggaactctgggaacagagccaggctgaccatcagcgggacccaggctatggatgaggctgactattactgtctggcgtgggacagcagcactgcgatcttcggcggaggcacccagctgaccgtcctcgtg

SEQ ID NO: 167 - DNA, 729 bp, synthetic construct
  source 1..729: mol_type = other DNA
caggtccagctggtacagtctggggctgaggtgaagaagcctgggtcctcggtgaaggtctcctgcaaggcttctggaggcaccttcagcagctatgctatcagctgggtgcgacaggcccctggacaagggcttgagtggatgggagggatcatccctatctttggtacagcaaactacgcacagaagttccagggcagagtcacgattaccgcggacaaatccacgagcacagcctacatggagctgagcagcctgagatctgaggacacggccgtgtattactgtgcgagatccccccggcgggcatatcatgatgcttttgatatctggggccaagggacaatggtcaccgtctcttcaggtggaggcggttcaggcggaggtggcagcggcggtggcgggagttcctatgagctgactcagccaccctcgatgtcagtggccccaggaaagacggccagcattacctgtggcggagaccatattggaagtaaaagtgttcactggtaccagcagaagccaggccaggcccctgtactggtcgtctatgatgatagcgaccggccctcagggatccctgagcgattctctggctccaacagagggaacagagccaggctgaccatcagcgggacccaggctatggatgaggctgactattactgtctggcgtgggacagcagcactgcgatcttcggcggaggcacccagctgaccgtcctcgtg

SEQ ID NO: 168 - DNA, 729 bp, synthetic construct
  source 1..729: mol_type = other DNA
caggtccagctggtacagtctggggctgaggtgaagaagcctgggtcctcggtgaaggtctcctgcaaggcttctggaggcaccttcagcagctatgctatcagctgggtgcgacaggcccctggacaagggcttgagtggatgggagggatcatccctatctttggtacagcaaactacgcacagaagttccagggcagagtcacgattaccgcggacaaatccacgagcacagcctacatggagctgagcagcctgagatctgaggacacggccgtgtattactgtgcgagatccccccggcgggcatatcatgatgcttttgatatctggggccaagggacaatggtcaccgtctcttcaggtggaggcggttcaggcggaggtggcagcggcggtggcgggagttcctatgagctgactcagccaccctcgatgtcagtggccccaggaaagacggccagcattacctgtggcggagaccatattggaagtaaaagtgttcactggtaccagcagaagccaggccaggcccctgtactggtcgtctatgatgatagcgaccggccctcagggatccctgagcgattcaagggcaagaacaaggggaacaaagccaagctgaccatcagcgggacccaggctatggatgaggctgactattactgtctggcgtgggacagcagcactgcgatcttcggcggaggcacccagctgaccgtcctcgtg

SEQ ID NO: 169 - DNA, 729 bp, synthetic construct
  source 1..729: mol_type = other DNA
caggtccagctggtacagtctggggctgaggtgaagaagcctgggtcctcggtgaaggtctcctgcaaggcttctggaggcaccttcagcagctatgctatcagctgggtgcgacaggcccctggacaagggcttgagtggatgggagggatcatccctatctttggtacagcaaactacgcacagaagttccagggcagagtcacgattaccgcggacaaatccacgagcacagcctacatggagctgagcagcctgagatctgaggacacggccgtgtattactgtgcgagatccccccggcgggcatatcatgatgcttttgatatctggggccaagggacaatggtcaccgtctcttcaggtggaggcggttcaggcggaggtggcagcggcggtggcgggagttcctatgagctgactcagccaccctcgatgtcagtggccccaggaaagacggccagcattacctgtggcggagaccatattggaagtaaaagtgttcactggtaccagcagaagccaggccaggcccctgtactggtcgtctatgatgatagcgaccggccctcagggatccctaggcgattctctggctccaactctgggaacacagccactctgaggatcagggggacccaggctatggatgaggctgactattactgtctggcgtgggacagcagcactgcgatcttcggcggaggcacccagctgaccgtcctcgtg

SEQ ID NO: 170 - DNA, 15 bp, synthetic construct
  source 1..15: mol_type = other DNA
agctatgctatcagc

SEQ ID NO: 171 - DNA, 51 bp, synthetic construct; identical to SEQ ID NO: 154
  source 1..51: mol_type = other DNA

SEQ ID NO: 172 - DNA, 36 bp, synthetic construct
  source 1..36: mol_type = other DNA
caccacagtaactactactactacggtatggacgtc

SEQ ID NO: 173 - DNA, 33 bp, synthetic construct
  source 1..33: mol_type = other DNA
ggcggaaacaacattggaagtaaaaatgtgcac

SEQ ID NO: 174 - DNA, 21 bp, synthetic construct
  source 1..21: mol_type = other DNA
agggatagcaaccggccctct

SEQ ID NO: 175 - DNA, 24 bp, synthetic construct
  source 1..24: mol_type = other DNA
caggtgtgggacagcagccatgtc

SEQ ID NO: 176 - DNA, 729 bp, synthetic construct
  source 1..729: mol_type = other DNA
caggtgcagctggtgcagtctggggctgaggtgaagaagcctgggtcctcggtgaaggtctcctgcaaggcttctggaggcaccttcagcagctatgctatcagctgggtgcgacaggcccctggacaagggcttgagtggatgggagggatcatccctatctttggtacagcaaactacgcacagaagttccagggcagagtcacgattaccgcggacgaatccacgggcacagcctacatggagctgagcagcctgagatctgaggacacggccgtgtattactgtgcgagacaccacagtaactactactactacggtatggacgtctggggccaagggaccacggtcaccgtctcgagaggcggtggcggatcaggtggcggtggaagtggcggtggtgggtccatggcctcctatgagctgactcagccactctcagtgtcagtggccctgggacagacggccaggattacctgtggcggaaacaacattggaagtaaaaatgtgcactggtaccagcagaagccaggccaggcccctgtgctggtcatctatagggatagcaaccggccctctgggatccctgagcgattctctggctccaactcggggaacacggccaccctgaccatcagcagagcccaagccggggatgaggctgactattactgtcaggtgtgggacagcagccatgtcttcggaactgggaccaaggtcaccgtccta

SEQ ID NO: 177 - DNA, 729 bp, synthetic construct
  source 1..729: mol_type = other DNA
caggtgcagctggtgcagtctggggctgaggtgaagaagcctgggtcctcggtgaaggtctcctgcaaggcttctggaggcaccttcagcagctatgctatcagctgggtgcgacaggcccctggacaagggcttgagtggatgggagggatcatccctatctttggtacagcaaactacgcacagaagttccagggcagagtcacgattaccgcggacgaatccacgggcacagcctacatggagctgagcagcctgagatctgaggacacggccgtgtattactgtgcgagacaccacagtaactactactactacggtatggacgtctggggccaagggaccacggtcaccgtctcgagaggcggtggcggatcaggtggcggtggaagtggcggtggtgggtccatggcctcctatgagctgactcagccactctcagtgtcagtggccctgggacagacggccaggattacctgtggcggaaacaacattggaagtaaaaatgtgcactggtaccagcagaagccaggccaggcccctgtgctggtcatctatagggatagcaaccggccctctgggatccctgagcgattccgaggccgaaactcggggaacacggcccgactgaccatcagcagagcccaagccggggatgaggctgactattactgtcaggtgtgggacagcagccatgtcttcggaactgggaccaaggtcaccgtccta

SEQ ID NO: 178 - DNA, 729 bp, synthetic construct
  source 1..729: mol_type = other DNA
caggtgcagctggtgcagtctggggctgaggtgaagaagcctgggtcctcggtgaaggtctcctgcaaggcttctggaggcaccttcagcagctatgctatcagctgggtgcgacaggcccctggacaagggcttgagtggatgggagggatcatccctatctttggtacagcaaactacgcacagaagttccagggcagagtcacgattaccgcggacgaatccacgggcacagcctacatggagctgagcagcctgagatctgaggacacggccgtgtattactgtgcgagacaccacagtaactactactactacggtatggacgtctggggccaagggaccacggtcaccgtctcgagaggcggtggcggatcaggtggcggtggaagtggcggtggtgggtccatggcctcctatgagctgactcagccactctcagtgtcagtggccctgggacagacggccaggattacctgtggcggaaacaacattggaagtaaaaatgtgcactggtaccagcagaagccaggccaggcccctgtgctggtcatctatagggatagcaaccggccctctgggatccctgagcgattccgaggctccaactcggggaaccgagcccgactgaccatcagcagagcccaagccggggatgaggctgactattactgtcaggtgtgggacagcagccatgtcttcggaactgggaccaaggtcaccgtccta

SEQ ID NO: 179 - DNA, 729 bp, synthetic construct
  source 1..729: mol_type = other DNA
caggtgcagctggtgcagtctggggctgaggtgaagaagcctgggtcctcggtgaaggtctcctgcaaggcttctggaggcaccttcagcagctatgctatcagctgggtgcgacaggcccctggacaagggcttgagtggatgggagggatcatccctatctttggtacagcaaactacgcacagaagttccagggcagagtcacgattaccgcggacgaatccacgggcacagcctacatggagctgagcagcctgagatctgaggacacggccgtgtattactgtgcgagacaccacagtaactactactactacggtatggacgtctggggccaagggaccacggtcaccgtctcgagaggcggtggcggatcaggtggcggtggaagtggcggtggtgggtccatggcctcctatgagctgactcagccactctcagtgtcagtggccctgggacagacggccaggattacctgtggcggaaacaacattggaagtaaaaatgtgcactggtaccagcagaagccaggccaggcccctgtgctggtcatctatagggatagcaaccggccctctgggatccctgagcgattctctggcaagaactcggggaacaaggccaagctgaccatcagcagagcccaagccggggatgaggctgactattactgtcaggtgtgggacagcagccatgtcttcggaactgggaccaaggtcaccgtccta

SEQ ID NO: 180 - DNA, 15 bp, synthetic construct
  source 1..15: mol_type = other DNA
gactacggtgtttca

SEQ ID NO: 181 - DNA, 48 bp, synthetic construct
  source 1..48: mol_type = other DNA
gtgatttggggtagcgaaaccacctactacaatagcgcgttgaagtcc

SEQ ID NO: 182 - DNA, 36 bp, synthetic construct
  source 1..36: mol_type = other DNA
cactattactacggcggatcttatgcgatggactat

SEQ ID NO: 183 - DNA, 33 bp, synthetic construct
  source 1..33: mol_type = other DNA
agagctagccaggatataagcaaatacctgaac

SEQ ID NO: 184 - DNA, 21 bp, synthetic construct
  source 1..21: mol_type = other DNA
cacacatctcggctgcatagt

SEQ ID NO: 185 - DNA, 27 bp, synthetic construct
  source 1..27: mol_type = other DNA
cagcaagggaataccctcccgtataca

SEQ ID NO: 186 - DNA, 726 bp, synthetic construct
  source 1..726: mol_type = other DNA
gacatccaaatgacgcagactacaagcagcttgtcagcctcactgggagatcgagtcaccattagctgcagagctagccaggatataagcaaatacctgaactggtatcagcagaaacccgatggcaccgtgaagctgctgatctatcacacatctcggctgcatagtggagttccttctcgattttcaggctctggctctgggacagattatagtctgacaatctccaacttggaacaggaggatatagccacctatttctgccagcaagggaataccctcccgtatacatttggaggcggcactaagctggagattacgggtggaggcggttcaggcggaggtggcagcggcggtggcgggagtgaagtgaaactgcaggagtcaggcccaggccttgtcgcaccctcccaatccctgagtgtcacatgcacagtaagcggggtttccctccccgactacggtgtttcatggatcagacagcctccaaggaaaggacttgagtggctcggggtgatttggggtagcgaaaccacctactacaatagcgcgttgaagtccaggctcaccatcatcaaggataacagtaaatcccaggttttcctgaaaatgaatagcctgcagacagatgatactgccatatactactgcgccaaacactattactacggcggatcttatgcgatggactattggggtcaaggtacatctgtaaccgtgagttcc

SEQ ID NO: 187 - DNA, 726 bp, synthetic construct
  source 1..726: mol_type = other DNA
gacatccaaatgacgcagactacaagcagcttgtcagcctcactgggagatcgagtcaccattagctgcagagctagccaggatataagcaaatacctgaactggtatcagcagaaacccgatggcaccgtgaagctgctgatctatcacacatctcggctgcatagtggagttccttctcgatttcgaggccgaggccgagggacacgatatagtctgacaatctccaacttggaacaggaggatatagccacctatttctgccagcaagggaataccctcccgtatacatttggaggcggcactaagctggagattacgggtggaggcggttcaggcggaggtggcagcggcggtggcgggagtgaagtgaaactgcaggagtcaggcccaggccttgtcgcaccctcccaatccctgagtgtcacatgcacagtaagcggggtttccctccccgactacggtgtttcatggatcagacagcctccaaggaaaggacttgagtggctcggggtgatttggggtagcgaaaccacctactacaatagcgcgttgaagtccaggctcaccatcatcaaggataacagtaaatcccaggttttcctgaaaatgaatagcctgcagacagatgatactgccatatactactgcgccaaacactattactacggcggatcttatgcgatggactattggggtcaaggtacatctgtaaccgtgagttcc

SEQ ID NO: 188 - DNA, 726 bp, synthetic construct
  source 1..726: mol_type = other DNA
gacatccaaatgacgcagactacaagcagcttgtcagcctcactgggagatcgagtcaccattagctgcagagctagccaggatataagcaaatacctgaactggtatcagcagaaacccgatggcaccgtgaagctgctgatctatcacacatctcggctgcatagtggagttccttctcgatttcgaggccgaggccgagggacagattatcgactgacaatctccaacttggaacaggaggatatagccacctatttctgccagcaagggaataccctcccgtatacatttggaggcggcactaagctggagattacgggtggaggcggttcaggcggaggtggcagcggcggtggcgggagtgaagtgaaactgcaggagtcaggcccaggccttgtcgcaccctcccaatccctgagtgtcacatgcacagtaagcggggtttccctccccgactacggtgtttcatggatcagacagcctccaaggaaaggacttgagtggctcggggtgatttggggtagcgaaaccacctactacaatagcgcgttgaagtccaggctcaccatcatcaaggataacagtaaatcccaggttttcctgaaaatgaatagcctgcagacagatgatactgccatatactactgcgccaaacactattactacggcggatcttatgcgatggactattggggtcaaggtacatctgtaaccgtgagttcc

SEQ ID NO: 189 - DNA, 726 bp, synthetic construct
  source 1..726: mol_type = other DNA
gacatccaaatgacgcagactacaagcagcttgtcagcctcactgggagatcgagtcaccattagctgcagagctagccaggatataagcaaatacctgaactggtatcagcagaaacccgatggcaccgtgaagctgctgatctatcacacatctcggctgcatagtggagttccttctcgatttcgaggccgaggctctgggacacgatatcgactgacaatctccaacttggaacaggaggatatagccacctatttctgccagcaagggaataccctcccgtatacatttggaggcggcactaagctggagattacgggtggaggcggttcaggcggaggtggcagcggcggtggcgggagtgaagtgaaactgcaggagtcaggcccaggccttgtcgcaccctcccaatccctgagtgtcacatgcacagtaagcggggtttccctccccgactacggtgtttcatggatcagacagcctccaaggaaaggacttgagtggctcggggtgatttggggtagcgaaaccacctactacaatagcgcgttgaagtccaggctcaccatcatcaaggataacagtaaatcccaggttttcctgaaaatgaatagcctgcagacagatgatactgccatatactactgcgccaaacactattactacggcggatcttatgcgatggactattggggtcaaggtacatctgtaaccgtgagttcc

SEQ ID NO: 190 - DNA, 726 bp, synthetic construct
  source 1..726: mol_type = other DNA
gacatccaaatgacgcagactacaagcagcttgtcagcctcactgggagatcgagtcaccattagctgcagagctagccaggatataagcaaatacctgaactggtatcagcagaaacccgatggcaccgtgaagctgctgatctatcacacatctcggctgcatagtggagttccttctcgattttcaggcaggggcagagggacaagatataggctgacaatctccaacttggaacaggaggatatagccacctatttctgccagcaagggaataccctcccgtatacatttggaggcggcactaagctggagattacgggtggaggcggttcaggcggaggtggcagcggcggtggcgggagtgaagtgaaactgcaggagtcaggcccaggccttgtcgcaccctcccaatccctgagtgtcacatgcacagtaagcggggtttccctccccgactacggtgtttcatggatcagacagcctccaaggaaaggacttgagtggctcggggtgatttggggtagcgaaaccacctactacaatagcgcgttgaagtccaggctcaccatcatcaaggataacagtaaatcccaggttttcctgaaaatgaatagcctgcagacagatgatactgccatatactactgcgccaaacactattactacggcggatcttatgcgatggactattggggtcaaggtacatctgtaaccgtgagttcc

SEQ ID NO: 191 - DNA, 726 bp, synthetic construct
  source 1..726: mol_type = other DNA
gacatccaaatgacgcagactacaagcagcttgtcagcctcactgggagatcgagtcaccattagctgcagagctagccaggatataagcaaatacctgaactggtatcagcagaaacccgatggcaccgtgaagctgctgatctatcacacatctcggctgcatagtggagttcctagacgatttagaggcagaggctctgggacagattatagtctgacaatctccaacttggaacaggaggatatagccacctatttctgccagcaagggaataccctcccgtatacatttggaggcggcactaagctggagattacgggtggaggcggttcaggcggaggtggcagcggcggtggcgggagtgaagtgaaactgcaggagtcaggcccaggccttgtcgcaccctcccaatccctgagtgtcacatgcacagtaagcggggtttccctccccgactacggtgtttcatggatcagacagcctccaaggaaaggacttgagtggctcggggtgatttggggtagcgaaaccacctactacaatagcgcgttgaagtccaggctcaccatcatcaaggataacagtaaatcccaggttttcctgaaaatgaatagcctgcagacagatgatactgccatatactactgcgccaaacactattactacggcggatcttatgcgatggactattggggtcaaggtacatctgtaaccgtgagttcc

SEQ ID NO: 192 - DNA, 726 bp, synthetic construct
  source 1..726: mol_type = other DNA
gacatccaaatgacgcagactacaagcagcttgtcagcctcactgggagatcgagtcaccattagctgcagagctagccaggatataagcaaatacctgaactggtatcagcagaaacccgatggcaccgtgaagctgctgatctatcacacatctcggctgcatagtggagttccttctcgatttaagggcaagggctctgggacaaaatatagtctgacaatctccaacttggaacaggaggatatagccacctatttctgccagcaagggaataccctcccgtatacatttggaggcggcactaagctggagattacgggtggaggcggttcaggcggaggtggcagcggcggtggcgggagtgaagtgaaactgcaggagtcaggcccaggccttgtcgcaccctcccaatccctgagtgtcacatgcacagtaagcggggtttccctccccgactacggtgtttcatggatcagacagcctccaaggaaaggacttgagtggctcggggtgatttggggtagcgaaaccacctactacaatagcgcgttgaagtccaggctcaccatcatcaaggataacagtaaatcccaggttttcctgaaaatgaatagcctgcagacagatgatactgccatatactactgcgccaaacactattactacggcggatcttatgcgatggactattggggtcaaggtacatctgtaaccgtgagttcc

SEQ ID NO: 193 - DNA, 726 bp, synthetic construct
  source 1..726: mol_type = other DNA
gacatccaaatgacgcagactacaagcagcttgtcagcctcactgggagatcgagtcaccattagctgcagagctagccaggatataagcaaatacctgaactggtatcagcagaaacccgatggcaccgtgaagctgctgatctatcacacatctcggctgcatagtggagttccttctcgatttagaggcaggggctctgggacagattataggctgacaatctccaacttggaacaggaggatatagccacctatttctgccagcaagggaataccctcccgtatacatttggaggcggcactaagctggagattacgggtggaggcggttcaggcggaggtggcagcggcggtggcgggagtgaagtgaaactgcaggagtcaggcccaggccttgtcgcaccctcccaatccctgagtgtcacatgcacagtaagcggggtttccctccccgactacggtgtttcatggatcagacagcctccaaggaaaggacttgagtggctcggggtgatttggggtagcgaaaccacctactacaatagcgcgttgaagtccaggctcaccatcatcaaggataacagtaaatcccaggttttcctgaaaatgaatagcctgcagacagatgatactgccatatactactgcgccaaacactattactacggcggatcttatgcgatggactattggggtcaaggtacatctgtaaccgtgagttcc

SEQ ID NO: 194 - DNA, 726 bp, synthetic construct
  source 1..726: mol_type = other DNA
gacatccaaatgacgcagactacaagcagcttgtcagcctcactgggagatcgagtcaccattagctgcagagctagccaggatataagcaaatacctgaactggtatcagcagaaacccgatggcaccgtgaagctgctgatctatcacacatctcggctgcatagtggagttccttctcgatttagaggctctggcagagggacaagatatagtctgacaatctccaacttggaacaggaggatatagccacctatttctgccagcaagggaataccctcccgtatacatttggaggcggcactaagctggagattacgggtggaggcggttcaggcggaggtggcagcggcggtggcgggagtgaagtgaaactgcaggagtcaggcccaggccttgtcgcaccctcccaatccctgagtgtcacatgcacagtaagcggggtttccctccccgactacggtgtttcatggatcagacagcctccaaggaaaggacttgagtggctcggggtgatttggggtagcgaaaccacctactacaatagcgcgttgaagtccaggctcaccatcatcaaggataacagtaaatcccaggttttcctgaaaatgaatagcctgcagacagatgatactgccatatactactgcgccaaacactattactacggcggatcttatgcgatggactattggggtcaaggtacatctgtaaccgtgagttcc

SEQ ID NO: 195 - DNA, 726 bp, synthetic construct
  source 1..726: mol_type = other DNA
gacatccaaatgacgcagactacaagcagcttgtcagcctcactgggagatcgagtcaccattagctgcagagctagccaggatataagcaaatacctgaactggtatcagcagaaacccgatggcaccgtgaagctgctgatctatcacacatctcggctgcatagtggagttccttctcgatttagaggctctggctctgggacaagatataggctgacaatctccaacttggaacaggaggatatagccacctatttctgccagcaagggaataccctcccgtatacatttggaggcggcactaagctggagattacgggtggaggcggttcaggcggaggtggcagcggcggtggcgggagtgaagtgaaactgcaggagtcaggcccaggccttgtcgcaccctcccaatccctgagtgtcacatgcacagtaagcggggtttccctccccgactacggtgtttcatggatcagacagcctccaaggaaaggacttgagtggctcggggtgatttggggtagcgaaaccacctactacaatagcgcgttgaagtccaggctcaccatcatcaaggataacagtaaatcccaggttttcctgaaaatgaatagcctgcagacagatgatactgccatatactactgcgccaaacactattactacggcggatcttatgcgatggactattggggtcaaggtacatctgtaaccgtgagttcc

SEQ ID NO: 196 - DNA, 726 bp, synthetic construct
  source 1..726: mol_type = other DNA
gacatccaaatgacgcagactacaagcagcttgtcagcctcactgggagatcgagtcaccattagctgcagagctagccaggatataagcaaatacctgaactggtatcagcagaaacccgatggcaccgtgaagctgctgatctatcacacatctcggctgcatagtggagttccttctcgattttcaggcaggggcagagggacaagatatagtctgacaatctccaacttggaacaggaggatatagccacctatttctgccagcaagggaataccctcccgtatacatttggaggcggcactaagctggagattacgggtggaggcggttcaggcggaggtggcagcggcggtggcgggagtgaagtgaaactgcaggagtcaggcccaggccttgtcgcaccctcccaatccctgagtgtcacatgcacagtaagcggggtttccctccccgactacggtgtttcatggatcagacagcctccaaggaaaggacttgagtggctcggggtgatttggggtagcgaaaccacctactacaatagcgcgttgaagtccaggctcaccatcatcaaggataacagtaaatcccaggttttcctgaaaatgaatagcctgcagacagatgatactgccatatactactgcgccaaacactattactacggcggatcttatgcgatggactattggggtcaaggtacatctgtaaccgtgagttcc

SEQ ID NO: 197 - DNA, 726 bp, synthetic construct
  source 1..726: mol_type = other DNA
gacatccaaatgacgcagactacaagcagcttgtcagcctcactgggagatcgagtcaccattagctgcagagctagccaggatataagcaaatacctgaactggtatcagcagaaacccgatggcaccgtgaagctgctgatctatcacacatctcggctgcatagtggagttccttctcgattttcaggcaggggcagagggacagattataggctgacaatctccaacttggaacaggaggatatagccacctatttctgccagcaagggaataccctcccgtatacatttggaggcggcactaagctggagattacgggtggaggcggttcaggcggaggtggcagcggcggtggcgggagtgaagtgaaactgcaggagtcaggcccaggccttgtcgcaccctcccaatccctgagtgtcacatgcacagtaagcggggtttccctccccgactacggtgtttcatggatcagacagcctccaaggaaaggacttgagtggctcggggtgatttggggtagcgaaaccacctactacaatagcgcgttgaagtccaggctcaccatcatcaaggataacagtaaatcccaggttttcctgaaaatgaatagcctgcagacagatgatactgccatatactactgcgccaaacactattactacggcggatcttatgcgatggactattggggtcaaggtacatctgtaaccgtgagttcc

SEQ ID NO: 198 - DNA, 726 bp, synthetic construct
  source 1..726: mol_type = other DNA
gacatccaaatgacgcagactacaagcagcttgtcagcctcactgggagatcgagtcaccattagctgcagagctagccaggatataagcaaatacctgaactggtatcagcagaaacccgatggcaccgtgaagctgctgatctatcacacatctcggctgcatagtggagttccttctcgatttaagggcaagggctctgggacaaaatataagctgacaatctccaacttggaacaggaggatatagccacctatttctgccagcaagggaataccctcccgtatacatttggaggcggcactaagctggagattacgggtggaggcggttcaggcggaggtggcagcggcggtggcgggagtgaagtgaaactgcaggagtcaggcccaggccttgtcgcaccctcccaatccctgagtgtcacatgcacagtaagcggggtttccctccccgactacggtgtttcatggatcagacagcctccaaggaaaggacttgagtggctcggggtgatttggggtagcgaaaccacctactacaatagcgcgttgaagtccaggctcaccatcatcaaggataacagtaaatcccaggttttcctgaaaatgaatagcctgcagacagatgatactgccatatactactgcgccaaacactattactacggcggatcttatgcgatggactattggggtcaaggtacatctgtaaccgtgagttcc

SEQ ID NO: 199 - DNA, 726 bp, synthetic construct
  source 1..726: mol_type = other DNA
gacatccaaatgacgcagactacaagcagcttgtcagcctcactgggagatcgagtcaccattagctgcagagctagccaggatataagcaaatacctgaactggtatcagcagaaacccgatggcaccgtgaagctgctgatctatcacacatctcggctgcatagtggagttccttctcgattttcaggcaagggcaaggggacaaaatataagctgacaatctccaacttggaacaggaggatatagccacctatttctgccagcaagggaataccctcccgtatacatttggaggcggcactaagctggagattacgggtggaggcggttcaggcggaggtggcagcggcggtggcgggagtgaagtgaaactgcaggagtcaggcccaggccttgtcgcaccctcccaatccctgagtgtcacatgcacagtaagcggggtttccctccccgactacggtgtttcatggatcagacagcctccaaggaaaggacttgagtggctcggggtgatttggggtagcgaaaccacctactacaatagcgcgttgaagtccaggctcaccatcatcaaggataacagtaaatcccaggttttcctgaaaatgaatagcctgcagacagatgatactgccatatactactgcgccaaacactattactacggcggatcttatgcgatggactattggggtcaaggtacatctgtaaccgtgagttcc

SEQ ID NO: 200 - DNA, 726 bp, synthetic construct
  source 1..726: mol_type = other DNA
gacatccaaatgacgcagactacaagcagcttgtcagcctcactgggagatcgagtcaccattagctgcagagctagccaggatataagcaaatacctgaactggtatcagcagaaacccgatggcaccgtgaagctgctgatctatcacacatctcggctgcatagtggagttccttctcgatttaagggcaagggcaaggggacaaaatataagctgacaatctccaacttggaacaggaggatatagccacctatttctgccagcaagggaataccctcccgtatacatttggaggcggcactaagctggagattacgggtggaggcggttcaggcggaggtggcagcggcggtggcgggagtgaagtgaaactgcaggagtcaggcccaggccttgtcgcaccctcccaatccctgagtgtcacatgcacagtaagcggggtttccctccccgactacggtgtttcatggatcagacagcctccaaggaaaggacttgagtggctcggggtgatttggggtagcgaaaccacctactacaatagcgcgttgaagtccaggctcaccatcatcaaggataacagtaaatcccaggttttcctgaaaatgaatagcctgcagacagatgatactgccatatactactgcgccaaacactattactacggcggatcttatgcgatggactattggggtcaaggtacatctgtaaccgtgagttcc

SEQ ID NO: 201 - DNA, 726 bp, synthetic construct
  source 1..726: mol_type = other DNA
gacatccaaatgacgcagactacaagcagcttgtcagcctcactgggagatcgagtcaccattagctgcagagctagccaggatataagcaaatacctgaactggtatcagcagaaacccgatggcaccgtgaagctgctgatctatcacacatctcggctgcatagtggagttccttctcgatttagaggcaggggcagagggacaagatataggctgacaatctccaacttggaacaggaggatatagccacctatttctgccagcaagggaataccctcccgtatacatttggaggcggcactaagctggagattacgggtggaggcggttcaggcggaggtggcagcggcggtggcgggagtgaagtgaaactgcaggagtcaggcccaggccttgtcgcaccctcccaatccctgagtgtcacatgcacagtaagcggggtttccctccccgactacggtgtttcatggatcagacagcctccaaggaaaggacttgagtggctcggggtgatttggggtagcgaaaccacctactacaatagcgcgttgaagtccaggctcaccatcatcaaggataacagtaaatcccaggttttcctgaaaatgaatagcctgcagacagatgatactgccatatactactgcgccaaacactattactacggcggatcttatgcgatggactattggggtcaaggtacatctgtaaccgtgagttcc

SEQ ID NO: 202 - DNA, 726 bp, synthetic construct
  source 1..726: mol_type = other DNA
gacatccaaatgacgcagactacaagcagcttgtcagcctcactgggagatcgagtcaccattagctgcagagctagccaggatataagcaaatacctgaactggtatcagcagaaacccgatggcaccgtgaagctgctgatctatcacacatctcggctgcatagtggagttccttctcgattttcaggctctggctctgggacaagatatagactgagaatctccaacttggaacaggaggatatagccacctatttctgccagcaagggaataccctcccgtatacatttggaggcggcactaagctggagattacgggtggaggcggttcaggcggaggtggcagcggcggtggcgggagtgaagtgaaactgcaggagtcaggcccaggccttgtcgcaccctcccaatccctgagtgtcacatgcacagtaagcggggtttccctccccgactacggtgtttcatggatcagacagcctccaaggaaaggacttgagtggctcggggtgatttggggtagcgaaaccacctactacaatagcgcgttgaagtccaggctcaccatcatcaaggataacagtaaatcccaggttttcctgaaaatgaatagcctgcagacagatgatactgccatatactactgcgccaaacactattactacggcggatcttatgcgatggactattggggtcaaggtacatctgtaaccgtgagttcc

SEQ ID NO: 203 - DNA, 726 bp, synthetic construct
  source 1..726: mol_type = other DNA
gacatccaaatgacgcagactacaagcagcttgtcagcctcactgggagatcgagtcaccattagctgcagagctagccaggatataagcaaatacctgaactggtatcagcagaaacccgatggcaccgtgaagctgctgatctatcacacatctcggctgcatagtggagttcctagacgatttagaggctctggctctgggacagattatagtctgacaatcaggaacttggaacaggaggatatagccacctatttctgccagcaagggaataccctcccgtatacatttggaggcggcactaagctggagattacgggtggaggcggttcaggcggaggtggcagcggcggtggcgggagtgaagtgaaactgcaggagtcaggcccaggccttgtcgcaccctcccaatccctgagtgtcacatgcacagtaagcggggtttccctccccgactacggtgtttcatggatcagacagcctccaaggaaaggacttgagtggctcggggtgatttggggtagcgaaaccacctactacaatagcgcgttgaagtccaggctcaccatcatcaaggataacagtaaatcccaggttttcctgaaaatgaatagcctgcagacagatgatactgccatatactactgcgccaaacactattactacggcggatcttatgcgatggactattggggtcaaggtacatctgtaaccgtgagttcc

SEQ ID NO: 204 - DNA, 726 bp, synthetic construct
  source 1..726: mol_type = other DNA
gacatccaaatgacgcagactacaagcagcttgtcagcctcactgggagatcgagtcaccattagctgcagagctagccaggatataagcaaatacctgaactggtatcagcagaaacccgatggcaccgtgaagctgctgatctatcacacatctcggctgcatagtggagttcctagacgattttcaggctctggctctgggacagattatagtctgagaatcaggaacttggaacaggaggatatagccacctatttctgccagcaagggaataccctcccgtatacatttggaggcggcactaagctggagattacgggtggaggcggttcaggcggaggtggcagcggcggtggcgggagtgaagtgaaactgcaggagtcaggcccaggccttgtcgcaccctcccaatccctgagtgtcacatgcacagtaagcggggtttccctccccgactacggtgtttcatggatcagacagcctccaaggaaaggacttgagtggctcggggtgatttggggtagcgaaaccacctactacaatagcgcgttgaagtccaggctcaccatcatcaaggataacagtaaatcccaggttttcctgaaaatgaatagcctgcagacagatgatactgccatatactactgcgccaaacactattactacggcggatcttatgcgatggactattggggtcaaggtacatctgtaaccgtgagttcc

SEQ ID NO: 205 - DNA, 726 bp, synthetic construct
  source 1..726: mol_type = other DNA
gacatccaaatgacgcagactacaagcagcttgtcagcctcactgggagatcgagtcaccattagctgcagagctagccaggatataagcaaatacctgaactggtatcagcagaaacccgatggcaccgtgaagctgctgatctatcacacatctcggctgcatagtggagttccttctcgattttcaggctctggctctgggacagattatagtctgacaatctccagattgagacagagagatatagccacctatttctgccagcaagggaataccctcccgtatacatttggaggcggcactaagctggagattacgggtggaggcggttcaggcggaggtggcagcggcggtggcgggagtgaagtgaaactgcaggagtcaggcccaggccttgtcgcaccctcccaatccctgagtgtcacatgcacagtaagcggggtttccctccccgactacggtgtttcatggatcagacagcctccaaggaaaggacttgagtggctcggggtgatttggggtagcgaaaccacctactacaatagcgcgttgaagtccaggctcaccatcatcaaggataacagtaaatcccaggttttcctgaaaatgaatagcctgcagacagatgatactgccatatactactgcgccaaacactattactacggcggatcttatgcgatggactattggggtcaaggtacatctgtaaccgtgagttcc

SEQ ID NO: 206 - protein, 5 aa, synthetic construct
GGGGS

SEQ ID NO: 207 - DNA, 84 bp, synthetic construct
  source 1..84: mol_type = other DNA
ttttgggtgctggtggtggttggtggagtcctggcttgctatagcttgctagtaacagtggcctttattattttctgggtgagg

SEQ ID NO: 208 - DNA, 318 bp, synthetic construct
  source 1..318: mol_type = other DNA
ggtcagcccaaggccaaccccactgtcactctgtttccgccctcctctgaggagctccaagccaacaaggccacactagtgtgtctgatcagtgacttctacccgggagctgtgacagtggcctggaaggcagatggcagccccgtcaaggcgggagtggagaccaccaaaccctccaaacagagcaacaacaagtacgcggccagcagctacctgagcctgacgcccgagcagtggaagtcccacagaagctacagctgccaggtcacgcatgaagggagcaccgtggagaagactgtggcccctacagaatgttcg

SEQ ID NO: 209 - DNA, 117 bp, synthetic construct
  source 1..117: mol_type = other DNA
atcgaagtgatgtaccctcctccttacctggacaacgagaagtccaacggcaccatcatccacgtgaagggcaagcacctgtgtccttctccactgttccccggacctagcaagcct

SEQ ID NO: 210 - DNA, 342 bp, synthetic construct
  source 1..342: mol_type = other DNA
ctgagagtgaagttcagcaggagcgcagacgcccccgcgtaccagcagggccagaaccagctctataacgagctcaatctaggacgaagagaggagtacgatgttttggacaagagacgtggccgggaccctgagatggggggaaagccgcagagaaggaagaaccctcaggaaggcctgtacaatgaactgcagaaagataagatggcggaggcctacagtgagattgggatgaaaggcgagcgccggaggggcaaggggcacgatggcctttaccagggtctcagtacagccaccaaggacacctacgacgcccttcacatgcaggccctgccccctcgc

SEQ ID NO: 211 - DNA, 123 bp, synthetic construct
  source 1..123: mol_type = other DNA
aggagtaagaggagcaggctcctgcacagtgactacatgaacatgactccccgccgccccgggcccacccgcaagcattaccagccctatgccccaccacgcgacttcgcagcctatcgctcc

SEQ ID NO: 212 - DNA, 147 bp, synthetic construct
  source 1..147: mol_type = other DNA
aggagtcagtgcatgtggccccgagagacccagctgctgctggaggtgccgccgtcgaccgaagacgccagaagctgccagttccccgaggaagagcggggcgagcgatcggcagaggagaaggggcggctgggagacctgtgggtg

SEQ ID NO: 213 - protein, 5 aa, synthetic construct
SYAIS

SEQ ID NO: 214 - protein, 17 aa, synthetic construct
GIIPIFGTANYAQKFQG

SEQ ID NO: 215 - protein, 12 aa, synthetic construct
SPRRAYHDAFDI

SEQ ID NO: 216 - protein, 11 aa, synthetic construct
GGDHIGSKSVH

SEQ ID NO: 217 - protein, 7 aa, synthetic construct
DDSDRPS

SEQ ID NO: 218 - protein, 9 aa, synthetic construct
LAWDSSTAI

SEQ ID NO: 219 - protein, 241 aa, synthetic construct
QLVQSGAEVKKPGSSVKVSCKASGGTFSSYAISWVRQAPGQGLEWMGGIIPIFGTANYAQKFQGRVTITADKSTSTAYMELSSLRSEDTAVYYCARSPRRAYHDAFDIWGQGTMVTVSSGGGGSGGGGSGGGGSSYELTQPPSMSVAPGKTASITCGGDHIGSKSVHWYQQKPGQAPVLVVYDDSDRPSGIPERFSGSNSGNTATLTISGTQAMDEADYYCLAWDSSTAIFGGGTQLTVLV

SEQ ID NO: 220 - protein, 241 aa, synthetic construct
QLVQSGAEVKKPGSSVKVSCKASGGTFSSYAISWVRQAPGQGLEWMGGIIPIFGTANYAQKFQGRVTITADKSTSTAYMELSSLRSEDTAVYYCARSPRRAYHDAFDIWGQGTMVTVSSGGGGSGGGGSGGGGSSYELTQPPSMSVAPGKTASITCGGDHIGSKSVHWYQQKPGQAPVLVVYDDSDRPSGIPERFRGRNRGNRATLTISGTQAMDEADYYCLAWDSSTAIFGGGTQLTVLV

SEQ ID NO: 221 - protein, 241 aa, synthetic construct
QLVQSGAEVKKPGSSVKVSCKASGGTFSSYAISWVRQAPGQGLEWMGGIIPIFGTANYAQKFQGRVTITADKSTSTAYMELSSLRSEDTAVYYCARSPRRAYHDAFDIWGQGTMVTVSSGGGGSGGGGSGGGGSSYELTQPPSMSVAPGKTASITCGGDHIGSKSVHWYQQKPGQAPVLVVYDDSDRPSGIPERFRGRNRGNTARLTISGTQAMDEADYYCLAWDSSTAIFGGGTQLTVLV

SEQ ID NO: 222 - protein, 241 aa, synthetic construct
QLVQSGAEVKKPGSSVKVSCKASGGTFSSYAISWVRQAPGQGLEWMGGIIPIFGTANYAQKFQGRVTITADKSTSTAYMELSSLRSEDTAVYYCARSPRRAYHDAFDIWGQGTMVTVSSGGGGSGGGGSGGGGSSYELTQPPSMSVAPGKTASITCGGDHIGSKSVHWYQQKPGQAPVLVVYDDSDRPSGIPERFRGRNSGNTARLTISGTQAMDEADYYCLAWDSSTAIFGGGTQLTVLV

SEQ ID NO: 223 - protein, 241 aa, synthetic construct
QLVQSGAEVKKPGSSVKVSCKASGGTFSSYAISWVRQAPGQGLEWMGGIIPIFGTANYAQKFQGRVTITADKSTSTAYMELSSLRSEDTAVYYCARSPRRAYHDAFDIWGQGTMVTVSSGGGGSGGGGSGGGGSSYELTQPPSMSVAPGKTASITCGGDHIGSKSVHWYQQKPGQAPVLVVYDDSDRPSGIPERFKGSNKGNKATLTISGTQAMDEADYYCLAWDSSTAIFGGGTQLTVLV

SEQ ID NO: 224 - protein, 241 aa, synthetic construct
QLVQSGAEVKKPGSSVKVSCKASGGTFSSYAISWVRQAPGQGLEWMGGIIPIFGTANYAQKFQGRVTITADKSTSTAYMELSSLRSEDTAVYYCARSPRRAYHDAFDIWGQGTMVTVSSGGGGSGGGGSGGGGSSYELTQPPSMSVAPGKTASITCGGDHIGSKSVHWYQQKPGQAPVLVVYDDSDRPSGIPERFRGSNSGNRARLTISGTQAMDEADYYCLAWDSSTAIFGGGTQLTVLV

SEQ ID NO: 225 - protein, 241 aa, synthetic construct
QLVQSGAEVKKPGSSVKVSCKASGGTFSSYAISWVRQAPGQGLEWMGGIIPIFGTANYAQKFQGRVTITADKSTSTAYMELSSLRSEDTAVYYCARSPRRAYHDAFDIWGQGTMVTVSSGGGGSGGGGSGGGGSSYELTQPPSMSVAPGKTASITCGGDHIGSKSVHWYQQKPGQAPVLVVYDDSDRPSGIPERFSGKNKGNKATLTISGTQAMDEADYYCLAWDSSTAIFGGGTQLTVLV

SEQ ID NO: 226 - protein, 241 aa, synthetic construct
QLVQSGAEVKKPGSSVKVSCKASGGTFSSYAISWVRQAPGQGLEWMGGIIPIFGTANYAQKFQGRVTITADKSTSTAYMELSSLRSEDTAVYYCARSPRRAYHDAFDIWGQGTMVTVSSGGGGSGGGGSGGGGSSYELTQPPSMSVAPGKTASITCGGDHIGSKSVHWYQQKPGQAPVLVVYDDSDRPSGIPERFSGRNSGNRARLTISGTQAMDEADYYCLAWDSSTAIFGGGTQLTVLV

SEQ ID NO: 227 - protein, 241 aa, synthetic construct
QLVQSGAEVKKPGSSVKVSCKASGGTFSSYAISWVRQAPGQGLEWMGGIIPIFGTANYAQKFQGRVTITADKSTSTAYMELSSLRSEDTAVYYCARSPRRAYHDAFDIWGQGTMVTVSSGGGGSGGGGSGGGGSSYELTQPPSMSVAPGKTASITCGGDHIGSKSVHWYQQKPGQAPVLVVYDDSDRPSGIPERFSGSNRGNRARLTISGTQAMDEADYYCLAWDSSTAIFGGGTQLTVLV

SEQ ID NO: 228 - protein, 241 aa, synthetic construct
QLVQSGAEVKKPGSSVKVSCKASGGTFSSYAISWVRQAPGQGLEWMGGIIPIFGTANYAQKFQGRVTITADKSTSTAYMELSSLRSEDTAVYYCARSPRRAYHDAFDIWGQGTMVTVSSGGGGSGGGGSGGGGSSYELTQPPSMSVAPGKTASITCGGDHIGSKSVHWYQQKPGQAPVLVVYDDSDRPSGIPERFKGKNKGNKAKLTISGTQAMDEADYYCLAWDSSTAIFGGGTQLTVLV

SEQ ID NO: 229 - protein, 241 aa, synthetic construct
QLVQSGAEVKKPGSSVKVSCKASGGTFSSYAISWVRQAPGQGLEWMGGIIPIFGTANYAQKFQGRVTITADKSTSTAYMELSSLRSEDTAVYYCARSPRRAYHDAFDIWGQGTMVTVSSGGGGSGGGGSGGGGSSYELTQPPSMSVAPGKTASITCGGDHIGSKSVHWYQQKPGQAPVLVVYDDSDRPSGIPRRFSGSNSGNTATLRIRGTQAMDEADYYCLAWDSSTAIFGGGTQLTVLV

SEQ ID NO: 230 - protein, 5 aa, synthetic construct
SYAIS

SEQ ID NO: 231 - protein, 17 aa, synthetic construct
GIIPIFGTANYAQKFQG

SEQ ID NO: 232 - protein, 12 aa, synthetic construct
HHSNYYYYGMDV

SEQ ID NO: 233 - protein, 11 aa, synthetic construct
GGNNIGSKNVH

SEQ ID NO: 234 - protein, 7 aa, synthetic construct
RDSNRPS

SEQ ID NO: 235 - protein, 8 aa, synthetic construct
QVWDSSHV

SEQ ID NO: 236 - protein, 243 aa, synthetic construct
QVQLVQSGAEVKKPGSSVKVSCKASGGTFSSYAISWVRQAPGQGLEWMGGIIPIFGTANYAQKFQGRVTITADESTGTAYMELSSLRSEDTAVYYCARHHSNYYYYGMDVWGQGTTVTVSRGGGGSGGGGSGGGGSMASYELTQPLSVSVALGQTARITCGGNNIGSKNVHWYQQKPGQAPVLVIYRDSNRPSGIPERFSGSNSGNTATLTISRAQAGDEADYYCQVWDSSHVFGTGTKVTVL

SEQ ID NO: 237 - protein, 243 aa, synthetic construct
QVQLVQSGAEVKKPGSSVKVSCKASGGTFSSYAISWVRQAPGQGLEWMGGIIPIFGTANYAQKFQGRVTITADESTGTAYMELSSLRSEDTAVYYCARHHSNYYYYGMDVWGQGTTVTVSRGGGGSGGGGSGGGGSMASYELTQPLSVSVALGQTARITCGGNNIGSKNVHWYQQKPGQAPVLVIYRDSNRPSGIPERFRGRNSGNTARLTISRAQAGDEADYYCQVWDSSHVFGTGTKVTVL

SEQ ID NO: 238 - protein, 243 aa, synthetic construct
QVQLVQSGAEVKKPGSSVKVSCKASGGTFSSYAISWVRQAPGQGLEWMGGIIPIFGTANYAQKFQGRVTITADESTGTAYMELSSLRSEDTAVYYCARHHSNYYYYGMDVWGQGTTVTVSRGGGGSGGGGSGGGGSMASYELTQPLSVSVALGQTARITCGGNNIGSKNVHWYQQKPGQAPVLVIYRDSNRPSGIPERFRGSNSGNRARLTISRAQAGDEADYYCQVWDSSHVFGTGTKVTVL

SEQ ID NO: 239 - protein, 243 aa, synthetic construct
QVQLVQSGAEVKKPGSSVKVSCKASGGTFSSYAISWVRQAPGQGLEWMGGIIPIFGTANYAQKFQGRVTITADESTGTAYMELSSLRSEDTAVYYCARHHSNYYYYGMDVWGQGTTVTVSRGGGGSGGGGSGGGGSMASYELTQPLSVSVALGQTARITCGGNNIGSKNVHWYQQKPGQAPVLVIYRDSNRPSGIPERFSGKNSGNKAKLTISRAQAGDEADYYCQVWDSSHVFGTGTKVTVL

SEQ ID NO: 240 - protein, 5 aa, synthetic construct
DYGVS

SEQ ID NO: 241 - protein, 16 aa, synthetic construct
VIWGSETTYYNSALKS

SEQ ID NO: 242 - protein, 12 aa, synthetic construct
HYYYGGSYAMDY

SEQ ID NO: 243 - protein, 11 aa, synthetic construct
RASQDISKYLN

SEQ ID NO: 244 - protein, 7 aa, synthetic construct
HTSRLHS

SEQ ID NO: 245 - protein, 9 aa, synthetic construct
QQGNTLPYT

SEQ ID NO: 246 - protein, 242 aa, synthetic construct
DIQMTQTTSSLSASLGDRVTISCRASQDISKYLNWYQQKPDGTVKLLIYHTSRLHSGVPSRFSGSGSGTDYSLTISNLEQEDIATYFCQQGNTLPYTFGGGTKLEITGGGGSGGGGSGGGGSEVKLQESGPGLVAPSQSLSVTCTVSGVSLPDYGVSWIRQPPRKGLEWLGVIWGSETTYYNSALKSRLTIIKDNSKSQVFLKMNSLQTDDTAIYYCAKHYYYGGSYAMDYWGQGTSVTVSS

SEQ ID NO: 247 - protein, 242 aa, synthetic construct
DIQMTQTTSSLSASLGDRVTISCRASQDISKYLNWYQQKPDGTVKLLIYHTSRLHSGVPSRFRGRGRGTRYSLTISNLEQEDIATYFCQQGNTLPYTFGGGTKLEITGGGGSGGGGSGGGGSEVKLQESGPGLVAPSQSLSVTCTVSGVSLPDYGVSWIRQPPRKGLEWLGVIWGSETTYYNSALKSRLTIIKDNSKSQVFLKMNSLQTDDTAIYYCAKHYYYGGSYAMDYWGQGTSVTVSS

SEQ ID NO: 248 - protein, 242 aa, synthetic construct
DIQMTQTTSSLSASLGDRVTISCRASQDISKYLNWYQQKPDGTVKLLIYHTSRLHSGVPSRFRGRGRGTDYRLTISNLEQEDIATYFCQQGNTLPYTFGGGTKLEITGGGGSGGGGSGGGGSEVKLQESGPGLVAPSQSLSVTCTVSGVSLPDYGVSWIRQPPRKGLEWLGVIWGSETTYYNSALKSRLTIIKDNSKSQVFLKMNSLQTDDTAIYYCAKHYYYGGSYAMDYWGQGTSVTVSS

SEQ ID NO: 249 - protein, 242 aa, synthetic construct
DIQMTQTTSSLSASLGDRVTISCRASQDISKYLNWYQQKPDGTVKLLIYHTSRLHSGVPSRFRGRGSGTRYRLTISNLEQEDIATYFCQQGNTLPYTFGGGTKLEITGGGGSGGGGSGGGGSEVKLQESGPGLVAPSQSLSVTCTVSGVSLPDYGVSWIRQPPRKGLEWLGVIWGSETTYYNSALKSRLTIIKDNSKSQVFLKMNSLQTDDTAIYYCAKHYYYGGSYAMDYWGQGTSVTVSS

SEQ ID NO: 250 - protein, 242 aa, synthetic construct
DIQMTQTTSSLSASLGDRVTISCRASQDISKYLNWYQQKPDGTVKLLIYHTSRLHSGVPSRFSGRGRGTRYRLTISNLEQEDIATYFCQQGNTLPYTFGGGTKLEITGGGGSGGGGSGGGGSEVKLQESGPGLVAPSQSLSVTCTVSGVSLPDYGVSWIRQPPRKGLEWLGVIWGSETTYYNSALKSRLTIIKDNSKSQVFLKMNSLQTDDTAIYYCAKHYYYGGSYAMDYWGQGTSVTVSS

SEQ ID NO: 251 - protein, 242 aa, synthetic construct
DIQMTQTTSSLSASLGDRVTISCRASQDISKYLNWYQQKPDGTVKLLIYHTSRLHSGVPRRFRGRGSGTDYSLTISNLEQEDIATYFCQQGNTLPYTFGGGTKLEITGGGGSGGGGSGGGGSEVKLQESGPGLVAPSQSLSVTCTVSGVSLPDYGVSWIRQPPRKGLEWLGVIWGSETTYYNSALKSRLTIIKDNSKSQVFLKMNSLQTDDTAIYYCAKHYYYGGSYAMDYWGQGTSVTVSS

SEQ ID NO: 252 - protein, 242 aa, synthetic construct
DIQMTQTTSSLSASLGDRVTISCRASQDISKYLNWYQQKPDGTVKLLIYHTSRLHSGVPSRFKGKGSGTKYSLTISNLEQEDIATYFCQQGNTLPYTFGGGTKLEITGGGGSGGGGSGGGGSEVKLQESGPGLVAPSQSLSVTCTVSGVSLPDYGVSWIRQPPRKGLEWLGVIWGSETTYYNSALKSRLTIIKDNSKSQVFLKMNSLQTDDTAIYYCAKHYYYGGSYAMDYWGQGTSVTVSS

SEQ ID NO: 253 - protein, 242 aa, synthetic construct
DIQMTQTTSSLSASLGDRVTISCRASQDISKYLNWYQQKPDGTVKLLIYHTSRLHSGVPSRFRGRGSGTDYRLTISNLEQEDIATYFCQQGNTLPYTFGGGTKLEITGGGGSGGGGSGGGGSEVKLQESGPGLVAPSQSLSVTCTVSGVSLPDYGVSWIRQPPRKGLEWLGVIWGSETTYYNSALKSRLTIIKDNSKSQVFLKMNSLQTDDTAIYYCAKHYYYGGSYAMDYWGQGTSVTVSS

SEQ ID NO: 254 - protein, 242 aa, synthetic construct
DIQMTQTTSSLSASLGDRVTISCRASQDISKYLNWYQQKPDGTVKLLIYHTSRLHSGVPSRFRGSGRGTRYSLTISNLEQEDIATYFCQQGNTLPYTFGGGTKLEITGGGGSGGGGSGGGGSEVKLQESGPGLVAPSQSLSVTCTVSGVSLPDYGVSWIRQPPRKGLEWLGVIWGSETTYYNSALKSRLTIIKDNSKSQVFLKMNSLQTDDTAIYYCAKHYYYGGSYAMDYWGQGTSVTVSS

SEQ ID NO: 255 - protein, 242 aa, synthetic construct
DIQMTQTTSSLSASLGDRVTISCRASQDISKYLNWYQQKPDGTVKLLIYHTSRLHSGVPSRFRGSGSGTRYRLTISNLEQEDIATYFCQQGNTLPYTFGGGTKLEITGGGGSGGGGSGGGGSEVKLQESGPGLVAPSQSLSVTCTVSGVSLPDYGVSWIRQPPRKGLEWLGVIWGSETTYYNSALKSRLTIIKDNSKSQVFLKMNSLQTDDTAIYYCAKHYYYGGSYAMDYWGQGTSVTVSS

SEQ ID NO: 256 - protein, 242 aa, synthetic construct
DIQMTQTTSSLSASLGDRVTISCRASQDISKYLNWYQQKPDGTVKLLIYHTSRLHSGVPSRFSGRGRGTRYSLTISNLEQEDIATYFCQQGNTLPYTFGGGTKLEITGGGGSGGGGSGGGGSEVKLQESGPGLVAPSQSLSVTCTVSGVSLPDYGVSWIRQPPRKGLEWLGVIWGSETTYYNSALKSRLTIIKDNSKSQVFLKMNSLQTDDTAIYYCAKHYYYGGSYAMDYWGQGTSVTVSS

SEQ ID NO: 257 - protein, 242 aa, synthetic construct
DIQMTQTTSSLSASLGDRVTISCRASQDISKYLNWYQQKPDGTVKLLIYHTSRLHSGVPSRFSGRGRGTDYRLTISNLEQEDIATYFCQQGNTLPYTFGGGTKLEITGGGGSGGGGSGGGGSEVKLQESGPGLVAPSQSLSVTCTVSGVSLPDYGVSWIRQPPRKGLEWLGVIWGSETTYYNSALKSRLTIIKDNSKSQVFLKMNSLQTDDTAIYYCAKHYYYGGSYAMDYWGQGTSVTVSS

SEQ ID NO: 258 - protein, 242 aa, synthetic construct
DIQMTQTTSSLSASLGDRVTISCRASQDISKYLNWYQQKPDGTVKLLIYHTSRLHSGVPSRFKGKGSGTKYKLTISNLEQEDIATYFCQQGNTLPYTFGGGTKLEITGGGGSGGGGSGGGGSEVKLQESGPGLVAPSQSLSVTCTVSGVSLPDYGVSWIRQPPRKGLEWLGVIWGSETTYYNSALKSRLTIIKDNSKSQVFLKMNSLQTDDTAIYYCAKHYYYGGSYAMDYWGQGTSVTVSS

SEQ ID NO: 259 - protein, 242 aa, synthetic construct
DIQMTQTTSSLSASLGDRVTISCRASQDISKYLNWYQQKPDGTVKLLIYHTSRLHSGVPSRFSGKGKGTKYKLTISNLEQEDIATYFCQQGNTLPYTFGGGTKLEITGGGGSGGGGSGGGGSEVKLQESGPGLVAPSQSLSVTCTVSGVSLPDYGVSWIRQPPRKGLEWLGVIWGSETTYYNSALKSRLTIIKDNSKSQVFLKMNSLQTDDTAIYYCAKHYYYGGSYAMDYWGQGTSVTVSS

SEQ ID NO: 260 - protein, 242 aa, synthetic construct
DIQMTQTTSSLSASLGDRVTISCRASQDISKYLNWYQQKPDGTVKLLIYHTSRLHSGVPSRFKGKGKGTKYKLTISNLEQEDIATYFCQQGNTLPYTFGGGTKLEITGGGGSGGGGSGGGGSEVKLQESGPGLVAPSQSLSVTCTVSGVSLPDYGVSWIRQPPRKGLEWLGVIWGSETTYYNSALKSRLTIIKDNSKSQVFLKMNSLQTDDTAIYYCAKHYYYGGSYAMDYWGQGTSVTVSS

SEQ ID NO: 261 - protein, 242 aa, synthetic construct
DIQMTQTTSSLSASLGDRVTISCRASQDISKYLNWYQQKPDGTVKLLIYHTSRLHSGVPSRFRGRGRGTRYRLTISNLEQEDIATYFCQQGNTLPYTFGGGTKLEITGGGGSGGGGSGGGGSEVKLQESGPGLVAPSQSLSVTCTVSGVSLPDYGVSWIRQPPRKGLEWLGVIWGSETTYYNSALKSRLTIIKDNSKSQVFLKMNSLQTDDTAIYYCAKHYYYGGSYAMDYWGQGTSVTVSS

SEQ ID NO: 262 - protein, 242 aa, synthetic construct
DIQMTQTTSSLSASLGDRVTISCRASQDISKYLNWYQQKPDGTVKLLIYHTSRLHSGVPSRFSGSGSGTRYRLRISNLEQEDIATYFCQQGNTLPYTFGGGTKLEITGGGGSGGGGSGGGGSEVKLQESGPGLVAPSQSLSVTCTVSGVSLPDYGVSWIRQPPRKGLEWLGVIWGSETTYYNSALKSRLTIIKDNSKSQVFLKMNSLQTDDTAIYYCAKHYYYGGSYAMDYWGQGTSVTVSS

SEQ ID NO: 263 - protein, 242 aa, synthetic construct
DIQMTQTTSSLSASLGDRVTISCRASQDISKYLNWYQQKPDGTVKLLIYHTSRLHSGVPRRFRGSGSGTDYSLTIRNLEQEDIATYFCQQGNTLPYTFGGGTKLEITGGGGSGGGGSGGGGSEVKLQESGPGLVAPSQSLSVTCTVSGVSLPDYGVSWIRQPPRKGLEWLGVIWGSETTYYNSALKSRLTIIKDNSKSQVFLKMNSLQTDDTAIYYCAKHYYYGGSYAMDYWGQGTSVTVSS

SEQ ID NO: 264 - protein, 242 aa, synthetic construct
DIQMTQTTSSLSASLGDRVTISCRASQDISKYLNWYQQKPDGTVKLLIYHTSRLHSGVPRRFSGSGSGTDYSLRIRNLEQEDIATYFCQQGNTLPYTFGGGTKLEITGGGGSGGGGSGGGGSEVKLQESGPGLVAPSQSLSVTCTVSGVSLPDYGVSWIRQPPRKGLEWLGVIWGSETTYYNSALKSRLTIIKDNSKSQVFLKMNSLQTDDTAIYYCAKHYYYGGSYAMDYWGQGTSVTVSS

SEQ ID NO: 265 - protein, 242 aa, synthetic construct
DIQMTQTTSSLSASLGDRVTISCRASQDISKYLNWYQQKPDGTVKLLIYHTSRLHSGVPSRFSGSGSGTDYSLTISRLRQRDIATYFCQQGNTLPYTFGGGTKLEITGGGGSGGGGSGGGGSEVKLQESGPGLVAPSQSLSVTCTVSGVSLPDYGVSWIRQPPRKGLEWLGVIWGSETTYYNSALKSRLTIIKDNSKSQVFLKMNSLQTDDTAIYYCAKHYYYGGSYAMDYWGQGTSVTVSS

SEQ ID NO: 266 - protein, 28 aa, synthetic construct
FWVLVVVGGVLACYSLLVTVAFIIFWVR

SEQ ID NO: 267 - protein, 106 aa, synthetic construct
GQPKANPTVTLFPPSSEELQANKATLVCLISDFYPGAVTVAWKADGSPVKAGVETTKPSKQSNNKYAASSYLSLTPEQWKSHRSYSCQVTHEGSTVEKTVAPTECS

SEQ ID NO: 268 - protein, 39 aa, synthetic construct
IEVMYPPPYLDNEKSNGTIIHVKGKHLCPSPLFPGPSKP

SEQ ID NO: 269 - protein, 114 aa, synthetic construct
LRVKFSRSADAPAYQQGQNQLYNELNLGRREEYDVLDKRRGRDPEMGGKPQRRKNPQEGLYNELQKDKMAEAYSEIGMKGERRRGKGHDGLYQGLSTATKDTYDALHMQALPPR

SEQ ID NO: 270 - protein, 41 aa, synthetic construct
RSKRSRLLHSDYMNMTPRRPGPTRKHYQPYAPPRDFAAYRS

SEQ ID NO: 271 - protein, 49 aa, synthetic construct
RSQCMWPRETQLLLEVPPSTEDARSCQFPEEERGERSAEEKGRLGDLWV